European Patent Application EP 4 339 202 A1 - sequence listing, part 2

SEQ ID NO: 48523 - protein, 9 aa, synthetic construct
GGNGNDRIH

SEQ ID NO: 48524 - protein, 9 aa, synthetic construct
GGNGNDNLM

SEQ ID NO: 48525 - protein, 9 aa, synthetic construct
GGNGNDLVH

SEQ ID NO: 48526 - protein, 9 aa, synthetic construct
GGNGNDLVL

SEQ ID NO: 48527 - protein, 9 aa, synthetic construct
GGNGNDLVR

SEQ ID NO: 48528 - protein, 9 aa, synthetic construct
GGNGNDLVY

SEQ ID NO: 48529 - protein, 9 aa, synthetic construct
GGNGNDLYV

SEQ ID NO: 48530 - protein, 9 aa, synthetic construct
GGNGNDMIS

SEQ ID NO: 48531 - protein, 9 aa, synthetic construct
GGNGNDMLL

SEQ ID NO: 48532 - protein, 9 aa, synthetic construct
GGNGNDMLM

SEQ ID NO: 48533 - protein, 9 aa, synthetic construct
GGNGNDMLS

SEQ ID NO: 48534 - protein, 9 aa, synthetic construct
GGNGNDMLV

SEQ ID NO: 48535 - protein, 9 aa, synthetic construct
GGNGNDNAF

SEQ ID NO: 48536 - protein, 9 aa, synthetic construct
GGNGNDNIG

SEQ ID NO: 48537 - protein, 9 aa, synthetic construct
GGNGNDNLL

SEQ ID NO: 48538 - protein, 9 aa, synthetic construct
GGNGNDNLR

SEQ ID NO: 48539 - protein, 9 aa, synthetic construct
GGNGNDRFV

SEQ ID NO: 48540 - protein, 9 aa, synthetic construct
GGNGNDNLV

SEQ ID NO: 48541 - protein, 9 aa, synthetic construct
GGNGNDQIH

SEQ ID NO: 48542 - protein, 9 aa, synthetic construct
GGNGNDQIT

SEQ ID NO: 48543 - protein, 9 aa, synthetic construct
GGNGNDQIV

SEQ ID NO: 48544 - protein, 9 aa, synthetic construct
GGNGNDQLG

SEQ ID NO: 48545 - protein, 9 aa, synthetic construct
GGNGNDQLI

SEQ ID NO: 48546 - protein, 9 aa, synthetic construct
GGNGNDQLN

SEQ ID NO: 48547 - protein, 9 aa, synthetic construct
GGNGNDQMC

SEQ ID NO: 48548 - protein, 9 aa, synthetic construct
GGNGNDQMF

SEQ ID NO: 48549 - protein, 9 aa, synthetic construct
GGNGNDQVE

SEQ ID NO: 48550 - protein, 9 aa, synthetic construct
GGNGNDRAL

SEQ ID NO: 48551 - protein, 9 aa, synthetic construct
GGNGNDRAY

SEQ ID NO: 48552 - protein, 9 aa, synthetic construct
GGNGNDRFE

SEQ ID NO: 48553 - protein, 9 aa, synthetic construct
GGNGNDTAN

SEQ ID NO: 48554 - protein, 9 aa, synthetic construct
GGNGNDTAQ

SEQ ID NO: 48555 - protein, 9 aa, synthetic construct
GGNGNDTFA

SEQ ID NO: 48556 - protein, 9 aa, synthetic construct
GGNGNDYIH

SEQ ID NO: 48557 - protein, 9 aa, synthetic construct
GGNGNDWIV

SEQ ID NO: 48558 - protein, 9 aa, synthetic construct
GGNGNDWIY

SEQ ID NO: 48559 - protein, 9 aa, synthetic construct
GGNGNDWLE

SEQ ID NO: 48560 - protein, 9 aa, synthetic construct
GGNGNDWLG

SEQ ID NO: 48561 - protein, 9 aa, synthetic construct
GGNGNDWLH

SEQ ID NO: 48562 - protein, 9 aa, synthetic construct
GGNGNDWLQ

SEQ ID NO: 48563 - protein, 9 aa, synthetic construct
GGNGNDWLW

SEQ ID NO: 48564 - protein, 9 aa, synthetic construct
GGNGNDWMD

SEQ ID NO: 48565 - protein, 9 aa, synthetic construct
GGNGNDWYS

SEQ ID NO: 48566 - protein, 9 aa, synthetic construct
GGNGNDWYV

SEQ ID NO: 48567 - protein, 9 aa, synthetic construct
GGNGNDYAW

SEQ ID NO: 48568 - protein, 9 aa, synthetic construct
GGNGNDYFV

SEQ ID NO: 48569 - protein, 9 aa, synthetic construct
GGNGNDYIE

SEQ ID NO: 48570 - protein, 9 aa, synthetic construct
GGNGNDYIT

SEQ ID NO: 48571 - protein, 9 aa, synthetic construct
GGNGNDWFT

SEQ ID NO: 48572 - protein, 9 aa, synthetic construct
GGNGNDYIV

SEQ ID NO: 48573 - protein, 9 aa, synthetic construct
GGNGNDYLG

SEQ ID NO: 48574 - protein, 9 aa, synthetic construct
GGNGNDYLH

SEQ ID NO: 48575 - protein, 9 aa, synthetic construct
GGNGNDYLI

SEQ ID NO: 48576 - protein, 9 aa, synthetic construct
GGNGNDYLT

SEQ ID NO: 48577 - protein, 9 aa, synthetic construct
GGNGNDYLW

SEQ ID NO: 48578 - protein, 9 aa, synthetic construct
GGNGNDYMD

SEQ ID NO: 48579 - protein, 9 aa, synthetic construct
GGNGNDYMK

SEQ ID NO: 48580 - protein, 9 aa, synthetic construct
GGNGNDYVY

SEQ ID NO: 48581 - protein, 9 aa, synthetic construct
GGNGPDALY

SEQ ID NO: 48582 - protein, 9 aa, synthetic construct
GGNGPDLIL

SEQ ID NO: 48583 - protein, 9 aa, synthetic construct
GGNGPDLLD

SEQ ID NO: 48584 - protein, 9 aa, synthetic construct
GGNGPDLVV

SEQ ID NO: 48585 - protein, 9 aa, synthetic construct
GGNGNDWID

SEQ ID NO: 48586 - protein, 9 aa, synthetic construct
GGNGNDVYR

SEQ ID NO: 48587 - protein, 9 aa, synthetic construct
GGNGNDTFE

SEQ ID NO: 48588 - protein, 9 aa, synthetic construct
GGNGNDTYK

SEQ ID NO: 48589 - protein, 9 aa, synthetic construct
GGNGNDTFI

SEQ ID NO: 48590 - protein, 9 aa, synthetic construct
GGNGNDTFM

SEQ ID NO: 48591 - protein, 9 aa, synthetic construct
GGNGNDTFQ

SEQ ID NO: 48592 - protein, 9 aa, synthetic construct
GGNGNDTFR

SEQ ID NO: 48593 - protein, 9 aa, synthetic construct
GGNGNDTIC

SEQ ID NO: 48594 - protein, 9 aa, synthetic construct
GGNGNDTIH

SEQ ID NO: 48595 - protein, 9 aa, synthetic construct
GGNGNDTIM

SEQ ID NO: 48596 - protein, 9 aa, synthetic construct
GGNGNDTIR

SEQ ID NO: 48597 - protein, 9 aa, synthetic construct
GGNGNDTMF

SEQ ID NO: 48598 - protein, 9 aa, synthetic construct
GGNGNDTMH

SEQ ID NO: 48599 - protein, 9 aa, synthetic construct
GGNGNDTVD

SEQ ID NO: 48600 - protein, 9 aa, synthetic construct
GGNGNDTVH

SEQ ID NO: 48601 - protein, 9 aa, synthetic construct
GGNGNDTVK

SEQ ID NO: 48602 - protein, 9 aa, synthetic construct
GGNGNDTYS

SEQ ID NO: 48603 - protein, 9 aa, synthetic construct
GGNGNDVYL

SEQ ID NO: 48604 - protein, 9 aa, synthetic construct
GGNGNDTYT

SEQ ID NO: 48605 - protein, 9 aa, synthetic construct
GGNGNDVFI

SEQ ID NO: 48606 - protein, 9 aa, synthetic construct
GGNGNDVFL

SEQ ID NO: 48607 - protein, 9 aa, synthetic construct
GGNGNDVFR

SEQ ID NO: 48608 - protein, 9 aa, synthetic construct
GGNGNDVII

SEQ ID NO: 48609 - protein, 9 aa, synthetic construct
GGNGNDVMN

SEQ ID NO: 48610 - protein, 9 aa, synthetic construct
GGNGNDVVE

SEQ ID NO: 48611 - protein, 9 aa, synthetic construct
GGNGNDVVH

SEQ ID NO: 48612 - protein, 9 aa, synthetic construct
GGNGNDVVI

SEQ ID NO: 48613 - protein, 9 aa, synthetic construct
GGNGNDVVN

SEQ ID NO: 48614 - protein, 9 aa, synthetic construct
GGNGNDVVR

SEQ ID NO: 48615 - protein, 9 aa, synthetic construct
GGNGNDVVV

SEQ ID NO: 48616 - protein, 9 aa, synthetic construct
GGNGNDVYI

SEQ ID NO: 48617 - protein, 9 aa, synthetic construct
GGLGTDFLI

SEQ ID NO: 48618 - protein, 9 aa, synthetic construct
GGLGTDFLD

SEQ ID NO: 48619 - protein, 9 aa, synthetic construct
GGLGTDELF

SEQ ID NO: 48620 - protein, 9 aa, synthetic construct
GGKGYDLLL

SEQ ID NO: 48621 - protein, 9 aa, synthetic construct
GGKGTDTLY

SEQ ID NO: 48622 - protein, 9 aa, synthetic construct
GGKGTDTMD

SEQ ID NO: 48623 - protein, 9 aa, synthetic construct
GGKGTDVIF

SEQ ID NO: 48624 - protein, 9 aa, synthetic construct
GGKGTDYLD

SEQ ID NO: 48625 - protein, 9 aa, synthetic construct
GGKGVDALN

SEQ ID NO: 48626 - protein, 9 aa, synthetic construct
GGKGVDFLR

SEQ ID NO: 48627 - protein, 9 aa, synthetic construct
GGKGVDHLF

SEQ ID NO: 48628 - protein, 9 aa, synthetic construct
GGKGVDIIK

SEQ ID NO: 48629 - protein, 9 aa, synthetic construct
GGKGVDILR

SEQ ID NO: 48630 - protein, 9 aa, synthetic construct
GGKGVDIMV

SEQ ID NO: 48631 - protein, 9 aa, synthetic construct
GGKGVDIVT

SEQ ID NO: 48632 - protein, 9 aa, synthetic construct
GGKGVDLLD

SEQ ID NO: 48633 - protein, 9 aa, synthetic construct
GGKGVDNLD

SEQ ID NO: 48634 - protein, 9 aa, synthetic construct
GGKGVDQMS

SEQ ID NO: 48635 - protein, 9 aa, synthetic construct
GGKGVDRFY

SEQ ID NO: 48636 - protein, 9 aa, synthetic construct
GGKGVDSLK

SEQ ID NO: 48637 - protein, 9 aa, synthetic construct
GGKGVDTIS

SEQ ID NO: 48638 - protein, 9 aa, synthetic construct
GGKGVDTMV

SEQ ID NO: 48639 - protein, 9 aa, synthetic construct
GGKGVDTVS

SEQ ID NO: 48640 - protein, 9 aa, synthetic construct
GGKGVDVAS

SEQ ID NO: 48641 - protein, 9 aa, synthetic construct
GGKGVDVLM

SEQ ID NO: 48642 - protein, 9 aa, synthetic construct
GGKGVDVLT

SEQ ID NO: 48643 - protein, 9 aa, synthetic construct
GGKGVDVVS

SEQ ID NO: 48644 - protein, 9 aa, synthetic construct
GGKGVDWLW

SEQ ID NO: 48645 - protein, 9 aa, synthetic construct
GGKGWDKLF

SEQ ID NO: 48646 - protein, 9 aa, synthetic construct
GGKGWDKLY

SEQ ID NO: 48647 - protein, 9 aa, synthetic construct
GGKGWDNLS

SEQ ID NO: 48648 - protein, 9 aa, synthetic construct
GGKGWDTYS

SEQ ID NO: 48649 - protein, 9 aa, synthetic construct
GGKGWDVLV

SEQ ID NO: 48650 - protein, 9 aa, synthetic construct
GGKGTDTLS

SEQ ID NO: 48651 - protein, 9 aa, synthetic construct
GGKGTDTLI

SEQ ID NO: 48652 - protein, 9 aa, synthetic construct
GGKGTDTLH

SEQ ID NO: 48653 - protein, 9 aa, synthetic construct
GGKGTDKLT

SEQ ID NO: 48654 - protein, 9 aa, synthetic construct
GGKGSDVIN

SEQ ID NO: 48655 - protein, 9 aa, synthetic construct
GGKGSDVIY

SEQ ID NO: 48656 - protein, 9 aa, synthetic construct
GGKGSDVLF

SEQ ID NO: 48657 - protein, 9 aa, synthetic construct
GGKGSDVLL

SEQ ID NO: 48658 - protein, 9 aa, synthetic construct
GGKGSDVLS

SEQ ID NO: 48659 - protein, 9 aa, synthetic construct
GGKGSDVLV

SEQ ID NO: 48660 - protein, 9 aa, synthetic construct
GGKGSDVYH

SEQ ID NO: 48661 - protein, 9 aa, synthetic construct
GGKGSDVYL

SEQ ID NO: 48662 - protein, 9 aa, synthetic construct
GGKGSDYIE

SEQ ID NO: 48663 - protein, 9 aa, synthetic construct
GGKGTDFLW

SEQ ID NO: 48664 - protein, 9 aa, synthetic construct
GGKGTDHLE

SEQ ID NO: 48665 - protein, 9 aa, synthetic construct
GGKGTDILA

SEQ ID NO: 48666 - protein, 9 aa, synthetic construct
GGKGTDILY

SEQ ID NO: 48667 - protein, 9 aa, synthetic construct
GGKGTDLAV

SEQ ID NO: 48668 - protein, 9 aa, synthetic construct
GGKGTDTLF

SEQ ID NO: 48669 - protein, 9 aa, synthetic construct
GGKGTDLLD

SEQ ID NO: 48670 - protein, 9 aa, synthetic construct
GGKGTDLMY

SEQ ID NO: 48671 - protein, 9 aa, synthetic construct
GGKGTDMLY

SEQ ID NO: 48672 - protein, 9 aa, synthetic construct
GGKGTDNLR

SEQ ID NO: 48673 - protein, 9 aa, synthetic construct
GGKGTDRID

SEQ ID NO: 48674 - protein, 9 aa, synthetic construct
GGKGTDRIE

SEQ ID NO: 48675 - protein, 9 aa, synthetic construct
GGKGTDRLT

SEQ ID NO: 48676 - protein, 9 aa, synthetic construct
GGKGTDRMN

SEQ ID NO: 48677 - protein, 9 aa, synthetic construct
GGKGTDRVY

SEQ ID NO: 48678 - protein, 9 aa, synthetic construct
GGKGTDSIS

SEQ ID NO: 48679 - protein, 9 aa, synthetic construct
GGKGTDSIT

SEQ ID NO: 48680 - protein, 9 aa, synthetic construct
GGKGTDSLV

SEQ ID NO: 48681 - protein, 9 aa, synthetic construct
GGKGTDTLA

SEQ ID NO: 48682 - protein, 9 aa, synthetic construct
GGKGWDWAY

SEQ ID NO: 48683 - protein, 9 aa, synthetic construct
GGKGYDLLV

SEQ ID NO: 48684 - protein, 9 aa, synthetic construct
GGLGADKFR

SEQ ID NO: 48685 - protein, 9 aa, synthetic construct
GGKGYDSMA

SEQ ID NO: 48686 - protein, 9 aa, synthetic construct
GGLGADELA

SEQ ID NO: 48687 - protein, 9 aa, synthetic construct
GGLGADELD

SEQ ID NO: 48688 - protein, 9 aa, synthetic construct
GGLGADELF

SEQ ID NO: 48689 - protein, 9 aa, synthetic construct
GGLGADEMF

SEQ ID NO: 48690 - protein, 9 aa, synthetic construct
GGLGADEMW

SEQ ID NO: 48691 - protein, 9 aa, synthetic construct
GGLGADEVY

SEQ ID NO: 48692 - protein, 9 aa, synthetic construct
GGLGADFFV

SEQ ID NO: 48693 - protein, 9 aa, synthetic construct
GGLGADFIT

SEQ ID NO: 48694 - protein, 9 aa, synthetic construct
GGLGADFLD

SEQ ID NO: 48695 - protein, 9 aa, synthetic construct
GGLGADFML

SEQ ID NO: 48696 - protein, 9 aa, synthetic construct
GGLGADFVD

SEQ ID NO: 48697 - protein, 9 aa, synthetic construct
GGLGADGID

SEQ ID NO: 48698 - protein, 9 aa, synthetic construct
GGLGADGLH

SEQ ID NO: 48699 - protein, 9 aa, synthetic construct
GGLGADGLT

SEQ ID NO: 48700 - protein, 9 aa, synthetic construct
GGLGADGLY

SEQ ID NO: 48701 - protein, 9 aa, synthetic construct
GGLGADHIM

SEQ ID NO: 48702 - protein, 9 aa, synthetic construct
GGLGADHLD

SEQ ID NO: 48703 - protein, 9 aa, synthetic construct
GGLGADHLS

SEQ ID NO: 48704 - protein, 9 aa, synthetic construct
GGLGADIFA

SEQ ID NO: 48705 - protein, 9 aa, synthetic construct
GGLGADIFD

SEQ ID NO: 48706 - protein, 9 aa, synthetic construct
GGLGADIFV

SEQ ID NO: 48707 - protein, 9 aa, synthetic construct
GGLGADIIK

SEQ ID NO: 48708 - protein, 9 aa, synthetic construct
GGLGADILE

SEQ ID NO: 48709 - protein, 9 aa, synthetic construct
GGLGADILF

SEQ ID NO: 48710 - protein, 9 aa, synthetic construct
GGLGADILG

SEQ ID NO: 48711 - protein, 9 aa, synthetic construct
GGLGADILH

SEQ ID NO: 48712 - protein, 9 aa, synthetic construct
GGLGADIVT

SEQ ID NO: 48713 - protein, 9 aa, synthetic construct
GGLGADIYV

SEQ ID NO: 48714 - protein, 9 aa, synthetic construct
GGLGADKFI

SEQ ID NO: 48715 - protein, 9 aa, synthetic construct
GGLGADEIY

SEQ ID NO: 48716 - protein, 9 aa, synthetic construct
GGLGADEIK

SEQ ID NO: 48717 - protein, 9 aa, synthetic construct
GGLGADDMW

SEQ ID NO: 48718 - protein, 9 aa, synthetic construct
GGLGADAII

SEQ ID NO: 48719 - protein, 9 aa, synthetic construct
GGKGYDSMD

SEQ ID NO: 48720 - protein, 9 aa, synthetic construct
GGKGYDSYQ

SEQ ID NO: 48721 - protein, 9 aa, synthetic construct
GGKGYDTLK

SEQ ID NO: 48722 - protein, 9 aa, synthetic construct
GGKGYDVLI

SEQ ID NO: 48723 - protein, 9 aa, synthetic construct
GGKGYDVLR

SEQ ID NO: 48724 - protein, 9 aa, synthetic construct
GGKGYDVMY

SEQ ID NO: 48725 - protein, 9 aa, synthetic construct
GGLGADAAS

SEQ ID NO: 48726 - protein, 9 aa, synthetic construct
GGLGADAFA

SEQ ID NO: 48727 - protein, 9 aa, synthetic construct
GGLGADAFF

SEQ ID NO: 48728 - protein, 9 aa, synthetic construct
GGLGADAFI

SEQ ID NO: 48729 - protein, 9 aa, synthetic construct
GGLGADAFT

SEQ ID NO: 48730 - protein, 9 aa, synthetic construct
GGLGADAID

SEQ ID NO: 48731 - protein, 9 aa, synthetic construct
GGLGADAIH

SEQ ID NO: 48732 - protein, 9 aa, synthetic construct
GGLGADAIN

SEQ ID NO: 48733 - protein, 9 aa, synthetic construct
GGLGADDMR

SEQ ID NO: 48734 - protein, 9 aa, synthetic construct
GGLGADALH

SEQ ID NO: 48735 - protein, 9 aa, synthetic construct
GGLGADALL

SEQ ID NO: 48736 - protein, 9 aa, synthetic construct
GGLGADALN

SEQ ID NO: 48737 - protein, 9 aa, synthetic construct
GGLGADALR

SEQ ID NO: 48738 - protein, 9 aa, synthetic construct
GGLGADALW

SEQ ID NO: 48739 - protein, 9 aa, synthetic construct
GGLGADAMS

SEQ ID NO: 48740 - protein, 9 aa, synthetic construct
GGLGADCLV

SEQ ID NO: 48741 - protein, 9 aa, synthetic construct
GGLGADDFI

SEQ ID NO: 48742 - protein, 9 aa, synthetic construct
GGLGADDFS

SEQ ID NO: 48743 - protein, 9 aa, synthetic construct
GGLGADDIR

SEQ ID NO: 48744 - protein, 9 aa, synthetic construct
GGLGADDLG

SEQ ID NO: 48745 - protein, 9 aa, synthetic construct
GGLGADDLW

SEQ ID NO: 48746 - protein, 9 aa, synthetic construct
GGLGADDMA

SEQ ID NO: 48747 - protein, 9 aa, synthetic construct
GGKGSDVIL

SEQ ID NO: 48748 - protein, 9 aa, synthetic construct
GGKGSDVID

SEQ ID NO: 48749 - protein, 9 aa, synthetic construct
GGKGSDVFL

SEQ ID NO: 48750 - protein, 9 aa, synthetic construct
GGKGSDVAT

SEQ ID NO: 48751 - protein, 9 aa, synthetic construct
GGKGRDRMD

SEQ ID NO: 48752 - protein, 9 aa, synthetic construct
GGKGRDSFS

SEQ ID NO: 48753 - protein, 9 aa, synthetic construct
GGKGRDSFV

SEQ ID NO: 48754 - protein, 9 aa, synthetic construct
GGKGRDSII

SEQ ID NO: 48755 - protein, 9 aa, synthetic construct
GGKGRDSIL

SEQ ID NO: 48756 - protein, 9 aa, synthetic construct
GGKGRDSLF

SEQ ID NO: 48757 - protein, 9 aa, synthetic construct
GGKGRDSLS

SEQ ID NO: 48758 - protein, 9 aa, synthetic construct
GGKGRDTLE

SEQ ID NO: 48759 - protein, 9 aa, synthetic construct
GGKGRDTLT

SEQ ID NO: 48760 - protein, 9 aa, synthetic construct
GGKGRDTLV

SEQ ID NO: 48761 - protein, 9 aa, synthetic construct
GGKGRDTMH

SEQ ID NO: 48762 - protein, 9 aa, synthetic construct
GGKGRDTML

SEQ ID NO: 48763 - protein, 9 aa, synthetic construct
GGKGRDTMT

SEQ ID NO: 48764 - protein, 9 aa, synthetic construct
GGKGRDTMV

SEQ ID NO: 48765 - protein, 9 aa, synthetic construct
GGKGRDVFA

SEQ ID NO: 48766 - protein, 9 aa, synthetic construct
GGKGRDVLD

SEQ ID NO: 48767 - protein, 9 aa, synthetic construct
GGKGRDVLK

SEQ ID NO: 48768 - protein, 9 aa, synthetic construct
GGKGRDVLR

SEQ ID NO: 48769 - protein, 9 aa, synthetic construct
GGKGRDVMF

SEQ ID NO: 48770 - protein, 9 aa, synthetic construct
GGKGRDVVA

SEQ ID NO: 48771 - protein, 9 aa, synthetic construct
GGKGRDVYF

SEQ ID NO: 48772 - protein, 9 aa, synthetic construct
GGKGRDWLN

SEQ ID NO: 48773 - protein, 9 aa, synthetic construct
GGKGRDYLY

SEQ ID NO: 48774 - protein, 9 aa, synthetic construct
GGKGSDAFV

SEQ ID NO: 48775 - protein, 9 aa, synthetic construct
GGKGSDALD

SEQ ID NO: 48776 - protein, 9 aa, synthetic construct
GGKGSDALV

SEQ ID NO: 48777 - protein, 9 aa, synthetic construct
GGKGSDAMA

SEQ ID NO: 48778 - protein, 9 aa, synthetic construct
GGKGSDAYL

SEQ ID NO: 48779 - protein, 9 aa, synthetic construct
GGKGSDDLD

SEQ ID NO: 48780 - protein, 9 aa, synthetic construct
GGKGRDRLT

SEQ ID NO: 48781 - protein, 9 aa, synthetic construct
GGKGRDRLD

SEQ ID NO: 48782 - protein, 9 aa, synthetic construct
GGKGRDRIE

SEQ ID NO: 48783 - protein, 9 aa, synthetic construct
GGKGRDKLT

SEQ ID NO: 48784 - protein, 9 aa, synthetic construct
GGKGRDAFV

SEQ ID NO: 48785 - protein, 9 aa, synthetic construct
GGKGRDALT

SEQ ID NO: 48786 - protein, 9 aa, synthetic construct
GGKGRDDIE

SEQ ID NO: 48787 - protein, 9 aa, synthetic construct
GGKGRDEIE

SEQ ID NO: 48788 - protein, 9 aa, synthetic construct
GGKGRDELN

SEQ ID NO: 48789 - protein, 9 aa, synthetic construct
GGKGRDFLV

SEQ ID NO: 48790 - protein, 9 aa, synthetic construct
GGKGRDHLD

SEQ ID NO: 48791 - protein, 9 aa, synthetic construct
GGKGRDIFR

SEQ ID NO: 48792 - protein, 9 aa, synthetic construct
GGKGRDIFS

SEQ ID NO: 48793 - protein, 9 aa, synthetic construct
GGKGRDIIN

SEQ ID NO: 48794 - protein, 9 aa, synthetic construct
GGKGRDKLE

SEQ ID NO: 48795 - protein, 9 aa, synthetic construct
GGKGRDKLI

SEQ ID NO: 48796 - protein, 9 aa, synthetic construct
GGKGRDKLL

SEQ ID NO: 48797 - protein, 9 aa, synthetic construct
GGKGRDLID

SEQ ID NO: 48798 - protein, 9 aa, synthetic construct
GGKGRDRFN

SEQ ID NO: 48799 - protein, 9 aa, synthetic construct
GGKGRDLIE

SEQ ID NO: 48800 - protein, 9 aa, synthetic construct
GGKGRDLIF

SEQ ID NO: 48801 - protein, 9 aa, synthetic construct
GGKGRDLIT

SEQ ID NO: 48802 - protein, 9 aa, synthetic construct
GGKGRDLLY

SEQ ID NO: 48803 - protein, 9 aa, synthetic construct
GGKGRDLML

SEQ ID NO: 48804 - protein, 9 aa, synthetic construct
GGKGRDMLM

SEQ ID NO: 48805 - protein, 9 aa, synthetic construct
GGKGRDMLV

SEQ ID NO: 48806 - protein, 9 aa, synthetic construct
GGKGRDNLF

SEQ ID NO: 48807 - protein, 9 aa, synthetic construct
GGKGRDNMH

SEQ ID NO: 48808 - protein, 9 aa, synthetic construct
GGKGRDQFV

SEQ ID NO: 48809 - protein, 9 aa, synthetic construct
GGKGRDQLD

SEQ ID NO: 48810 - protein, 9 aa, synthetic construct
GGKGRDQLT

SEQ ID NO: 48811 - protein, 9 aa, synthetic construct
GGKGRDQVW

SEQ ID NO: 48812 - protein, 9 aa, synthetic construct
GGKGSDEIW

SEQ ID NO: 48813 - protein, 9 aa, synthetic construct
GGKGSDELT

SEQ ID NO: 48814 - protein, 9 aa, synthetic construct
GGKGSDFIE

SEQ ID NO: 48815 - protein, 9 aa, synthetic construct
GGKGSDTLH

SEQ ID NO: 48816 - protein, 9 aa, synthetic construct
GGKGSDSLI

SEQ ID NO: 48817 - protein, 9 aa, synthetic construct
GGKGSDSLS

SEQ ID NO: 48818 - protein, 9 aa, synthetic construct
GGKGSDSLY

SEQ ID NO: 48819 - protein, 9 aa, synthetic construct
GGKGSDSVL

SEQ ID NO: 48820 - protein, 9 aa, synthetic construct
GGKGSDSYW

SEQ ID NO: 48821 - protein, 9 aa, synthetic construct
GGKGSDTAD

SEQ ID NO: 48822 - protein, 9 aa, synthetic construct
GGKGSDTAT

SEQ ID NO: 48823 - protein, 9 aa, synthetic construct
GGKGSDTAV

SEQ ID NO: 48824 - protein, 9 aa, synthetic construct
GGKGSDTFL

SEQ ID NO: 48825 - protein, 9 aa, synthetic construct
GGKGSDTID

SEQ ID NO: 48826 - protein, 9 aa, synthetic construct
GGKGSDTIR

SEQ ID NO: 48827 - protein, 9 aa, synthetic construct
GGKGSDTLA

SEQ ID NO: 48828 - protein, 9 aa, synthetic construct
GGKGSDTLF

SEQ ID NO: 48829 - protein, 9 aa, synthetic construct
GGKGSDTLQ

SEQ ID NO: 48830 - protein, 9 aa, synthetic construct
GGKGSDSIR

SEQ ID NO: 48831 - protein, 9 aa, synthetic construct
GGKGSDTLS

SEQ ID NO: 48832 - protein, 9 aa, synthetic construct
GGKGSDTMA

SEQ ID NO: 48833 - protein, 9 aa, synthetic construct
GGKGSDTMR

SEQ ID NO: 48834 - protein, 9 aa, synthetic construct
GGKGSDTMT

SEQ ID NO: 48835 - protein, 9 aa, synthetic construct
GGKGSDTMV

SEQ ID NO: 48836 - protein, 9 aa, synthetic construct
GGKGSDTMX

SEQ ID NO: 48837 - protein, 9 aa, synthetic construct
GGKGSDTVF

SEQ ID NO: 48838 - protein, 9 aa, synthetic construct
GGKGSDTVS

SEQ ID NO: 48839 - protein, 9 aa, synthetic construct
GGKGSDTYA

SEQ ID NO: 48840 - protein, 9 aa, synthetic construct
GGKGSDTYF

SEQ ID NO: 48841 - protein, 9 aa, synthetic construct
GGKGSDTYL

SEQ ID NO: 48842 - protein, 9 aa, synthetic construct
GGKGSDTYR

SEQ ID NO: 48843 - protein, 9 aa, synthetic construct
GGKGSDTYS

SEQ ID NO: 48844 - protein, 9 aa, synthetic construct
GGKGSDSIS

SEQ ID NO: 48845 - protein, 9 aa, synthetic construct
GGKGSDSIK

SEQ ID NO: 48846 - protein, 9 aa, synthetic construct
GGKGSDGLK

SEQ ID NO: 48847 - protein, 9 aa, synthetic construct
GGKGSDKLG

SEQ ID NO: 48848 - protein, 9 aa, synthetic construct
GGKGSDGMT

SEQ ID NO: 48849 - protein, 9 aa, synthetic construct
GGKGSDHLE

SEQ ID NO: 48850 - protein, 9 aa, synthetic construct
GGKGSDHLI

SEQ ID NO: 48851 - protein, 9 aa, synthetic construct
GGKGSDILF

SEQ ID NO: 48852 - protein, 9 aa, synthetic construct
GGKGSDILS

SEQ ID NO: 48853 - protein, 9 aa, synthetic construct
GGKGSDILT

SEQ ID NO: 48854 - protein, 9 aa, synthetic construct
GGKGSDIMD

SEQ ID NO: 48855 - protein, 9 aa, synthetic construct
GGKGSDIVK

SEQ ID NO: 48856 - protein, 9 aa, synthetic construct
GGKGSDIVR

SEQ ID NO: 48857 - protein, 9 aa, synthetic construct
GGKGSDIYR

SEQ ID NO: 48858 - protein, 9 aa, synthetic construct
GGKGSDIYY

SEQ ID NO: 48859 - protein, 9 aa, synthetic construct
GGKGSDKFT

SEQ ID NO: 48860 - protein, 9 aa, synthetic construct
GGKGSDKLD

SEQ ID NO: 48861 - protein, 9 aa, synthetic construct
GGKGSDKLI

SEQ ID NO: 48862 - protein, 9 aa, synthetic construct
GGKGSDRVF

SEQ ID NO: 48863 - protein, 9 aa, synthetic construct
GGKGSDKLV

SEQ ID NO: 48864 - protein, 9 aa, synthetic construct
GGKGSDKYE

SEQ ID NO: 48865 - protein, 9 aa, synthetic construct
GGKGSDLIL

SEQ ID NO: 48866 - protein, 9 aa, synthetic construct
GGKGSDLVN

SEQ ID NO: 48867 - protein, 9 aa, synthetic construct
GGKGSDNLN

SEQ ID NO: 48868 - protein, 9 aa, synthetic construct
GGKGSDQID

SEQ ID NO: 48869 - protein, 9 aa, synthetic construct
GGKGSDRFD

SEQ ID NO: 48870 - protein, 9 aa, synthetic construct
GGKGSDRFE

SEQ ID NO: 48871 - protein, 9 aa, synthetic construct
GGKGSDRIF

SEQ ID NO: 48872 - protein, 9 aa, synthetic construct
GGKGSDRIY

SEQ ID NO: 48873 - protein, 9 aa, synthetic construct
GGKGSDRLI

SEQ ID NO: 48874 - protein, 9 aa, synthetic construct
GGKGSDRLY

SEQ ID NO: 48875 - protein, 9 aa, synthetic construct
GGKGSDRMF

SEQ ID NO: 48876 - protein, 9 aa, synthetic construct
GGLGADKFQ

SEQ ID NO: 48877 - protein, 9 aa, synthetic construct
GGLGADKLF

SEQ ID NO: 48878 - protein, 9 aa, synthetic construct
GGLGDDQMT

SEQ ID NO: 48879 - protein, 9 aa, synthetic construct
GGLGDDIMA

SEQ ID NO: 48880 - protein, 9 aa, synthetic construct
GGLGDDELS

SEQ ID NO: 48881 - protein, 9 aa, synthetic construct
GGLGDDELT

SEQ ID NO: 48882 - protein, 9 aa, synthetic construct
GGLGDDELV

SEQ ID NO: 48883 - protein, 9 aa, synthetic construct
GGLGDDELW

SEQ ID NO: 48884 - protein, 9 aa, synthetic construct
GGLGDDEMT

SEQ ID NO: 48885 - protein, 9 aa, synthetic construct
GGLGDDEYC

SEQ ID NO: 48886 - protein, 9 aa, synthetic construct
GGLGDDFIL

SEQ ID NO: 48887 - protein, 9 aa, synthetic construct
GGLGDDFIV

SEQ ID NO: 48888 - protein, 9 aa, synthetic construct
GGLGDDFIY

SEQ ID NO: 48889 - protein, 9 aa, synthetic construct
GGLGDDFLE

SEQ ID NO: 48890 - protein, 9 aa, synthetic construct
GGLGDDFLM

SEQ ID NO: 48891 - protein, 9 aa, synthetic construct
GGLGDDFME

SEQ ID NO: 48892 - protein, 9 aa, synthetic construct
GGLGDDFVD

SEQ ID NO: 48893 - protein, 9 aa, synthetic construct
GGLGDDFVS

SEQ ID NO: 48894 - protein, 9 aa, synthetic construct
GGLGDDFYV

SEQ ID NO: 48895 - protein, 9 aa, synthetic construct
GGLGDDGAS

SEQ ID NO: 48896 - protein, 9 aa, synthetic construct
GGLGDDGFS

SEQ ID NO: 48897 - protein, 9 aa, synthetic construct
GGLGDDGIW

SEQ ID NO: 48898 - protein, 9 aa, synthetic construct
GGLGDDGLV

SEQ ID NO: 48899 - protein, 9 aa, synthetic construct
GGLGDDGLW

SEQ ID NO: 48900 - protein, 9 aa, synthetic construct
GGLGDDGMA

SEQ ID NO: 48901 - protein, 9 aa, synthetic construct
GGLGDDHID

SEQ ID NO: 48902 - protein, 9 aa, synthetic construct
GGLGDDHIM

SEQ ID NO: 48903 - protein, 9 aa, synthetic construct
GGLGDDHIN

SEQ ID NO: 48904 - protein, 9 aa, synthetic construct
GGLGDDHLL

SEQ ID NO: 48905 - protein, 9 aa, synthetic construct
GGLGDDHVW

SEQ ID NO: 48906 - protein, 9 aa, synthetic construct
GGLGDDIAY

SEQ ID NO: 48907 - protein, 9 aa, synthetic construct
GGLGDDIFV

SEQ ID NO: 48908 - protein, 9 aa, synthetic construct
GGLGDDIIL

SEQ ID NO: 48909 - protein, 9 aa, synthetic construct
GGLGDDELN

SEQ ID NO: 48910 - protein, 9 aa, synthetic construct
GGLGDDELL

SEQ ID NO: 48911 - protein, 9 aa, synthetic construct
GGLGDDELH

SEQ ID NO: 48912 - protein, 9 aa, synthetic construct
GGLGDDCIK

SEQ ID NO: 48913 - protein, 9 aa, synthetic construct
GGLGDDAIN

SEQ ID NO: 48914 - protein, 9 aa, synthetic construct
GGLGDDAIT

SEQ ID NO: 48915 - protein, 9 aa, synthetic construct
GGLGDDAIY

SEQ ID NO: 48916 - protein, 9 aa, synthetic construct
GGLGDDALA

SEQ ID NO: 48917 - protein, 9 aa, synthetic construct
GGLGDDALL

SEQ ID NO: 48918 - protein, 9 aa, synthetic construct
GGLGDDALM

SEQ ID NO: 48919 - protein, 9 aa, synthetic construct
GGLGDDALN

SEQ ID NO: 48920 - protein, 9 aa, synthetic construct
GGLGDDALQ

SEQ ID NO: 48921 - protein, 9 aa, synthetic construct
GGLGDDALV

SEQ ID NO: 48922 - protein, 9 aa, synthetic construct
GGLGDDAMD

SEQ ID NO: 48923 - protein, 9 aa, synthetic construct
GGLGDDAMQ

SEQ ID NO: 48924 - protein, 9 aa, synthetic construct
GGLGDDAMS

SEQ ID NO: 48925 - protein, 9 aa, synthetic construct
GGLGDDAVR

SEQ ID NO: 48926 - protein, 9 aa, synthetic construct
GGLGDDCYV

SEQ ID NO: 48927 - protein, 9 aa, synthetic construct
GGLGDDELG

SEQ ID NO: 48928 - protein, 9 aa, synthetic construct
GGLGDDDIN

SEQ ID NO: 48929 - protein, 9 aa, synthetic construct
GGLGDDDIS

SEQ ID NO: 48930 - protein, 9 aa, synthetic construct
GGLGDDDLF

SEQ ID NO: 48931 - protein, 9 aa, synthetic construct
GGLGDDDLI

SEQ ID NO: 48932 - protein, 9 aa, synthetic construct
GGLGDDDLY

SEQ ID NO: 48933 - protein, 9 aa, synthetic construct
GGLGDDDVD

SEQ ID NO: 48934 - protein, 9 aa, synthetic construct
GGLGDDDVR

SEQ ID NO: 48935 - protein, 9 aa, synthetic construct
GGLGDDDYF

SEQ ID NO: 48936 - protein, 9 aa, synthetic construct
GGLGDDDYT

SEQ ID NO: 48937 - protein, 9 aa, synthetic construct
GGLGDDDYY

SEQ ID NO: 48938 - protein, 9 aa, synthetic construct
GGLGDDEAF

SEQ ID NO: 48939 - protein, 9 aa, synthetic construct
GGLGDDEIA

SEQ ID NO: 48940 - protein, 9 aa, synthetic construct
GGLGDDEIH

SEQ ID NO: 48941 - protein, 9 aa, synthetic construct
GGLGDDIIR

SEQ ID NO: 48942 - protein, 9 aa, synthetic construct
GGLGDDIVD

SEQ ID NO: 48943 - protein, 9 aa, synthetic construct
GGLGADKLN

SEQ ID NO: 48944 - protein, 9 aa, synthetic construct
GGLGDDIVL

SEQ ID NO: 48945 - protein, 9 aa, synthetic construct
GGLGDDLVM

SEQ ID NO: 48946 - protein, 9 aa, synthetic construct
GGLGDDLVY

SEQ ID NO: 48947 - protein, 9 aa, synthetic construct
GGLGDDLYA

SEQ ID NO: 48948 - protein, 9 aa, synthetic construct
GGLGDDLYE

SEQ ID NO: 48949 - protein, 9 aa, synthetic construct
GGLGDDLYT

SEQ ID NO: 48950 - protein, 9 aa, synthetic construct
GGLGDDMIR

SEQ ID NO: 48951 - protein, 9 aa, synthetic construct
GGLGDDMIT

SEQ ID NO: 48952 - protein, 9 aa, synthetic construct
GGLGDDMLI

SEQ ID NO: 48953 - protein, 9 aa, synthetic construct
GGLGDDMLK

SEQ ID NO: 48954 - protein, 9 aa, synthetic construct
GGLGDDMLL

SEQ ID NO: 48955 - protein, 9 aa, synthetic construct
GGLGDDMLT

SEQ ID NO: 48956 - protein, 9 aa, synthetic construct
GGLGDDMLY

SEQ ID NO: 48957 - protein, 9 aa, synthetic construct
GGLGDDMMD

SEQ ID NO: 48958 - protein, 9 aa, synthetic construct
GGLGDDNAR

SEQ ID NO: 48959 - protein, 9 aa, synthetic construct
GGLGDDNID

SEQ ID NO: 48960 - protein, 9 aa, synthetic construct
GGLGDDNIS

SEQ ID NO: 48961 - protein, 9 aa, synthetic construct
GGLGDDNIW

SEQ ID NO: 48962 - protein, 9 aa, synthetic construct
GGLGDDNLA

SEQ ID NO: 48963 - protein, 9 aa, synthetic construct
GGLGDDNLN

SEQ ID NO: 48964 - protein, 9 aa, synthetic construct
GGLGDDNYV

SEQ ID NO: 48965 - protein, 9 aa, synthetic construct
GGLGDDNYY

SEQ ID NO: 48966 - protein, 9 aa, synthetic construct
GGLGDDQFR

SEQ ID NO: 48967 - protein, 9 aa, synthetic construct
GGLGDDQIE

SEQ ID NO: 48968 - protein, 9 aa, synthetic construct
GGLGDDQIQ

SEQ ID NO: 48969 - protein, 9 aa, synthetic construct
GGLGDDQLA

SEQ ID NO: 48970 - protein, 9 aa, synthetic construct
GGLGDDQLQ

SEQ ID NO: 48971 - protein, 9 aa, synthetic construct
GGLGDDQLS

SEQ ID NO: 48972 - protein, 9 aa, synthetic construct
GGLGDDQLW

SEQ ID NO: 48973 - protein, 9 aa, synthetic construct
GGLGDDQMI

SEQ ID NO: 48974 - protein, 9 aa, synthetic construct
GGLGDDLVK

SEQ ID NO: 48975 - protein, 9 aa, synthetic construct
GGLGDDLMT

SEQ ID NO: 48976 - protein, 9 aa, synthetic construct
GGLGDDLMS

SEQ ID NO: 48977 - protein, 9 aa, synthetic construct
GGLGDDKLT

SEQ ID NO: 48978 - protein, 9 aa, synthetic construct
GGLGDDIVS

SEQ ID NO: 48979 - protein, 9 aa, synthetic construct
GGLGDDIVY

SEQ ID NO: 48980 - protein, 9 aa, synthetic construct
GGLGDDIYH

SEQ ID NO: 48981 - protein, 9 aa, synthetic construct
GGLGDDIYR

SEQ ID NO: 48982 - protein, 9 aa, synthetic construct
GGLGDDIYW

SEQ ID NO: 48983 - protein, 9 aa, synthetic construct
GGLGDDKFV

SEQ ID NO: 48984 - protein, 9 aa, synthetic construct
GGLGDDKID

SEQ ID NO: 48985 - protein, 9 aa, synthetic construct
GGLGDDKIK

SEQ ID NO: 48986 - protein, 9 aa, synthetic construct
GGLGDDKIL

SEQ ID NO: 48987 - protein, 9 aa, synthetic construct
GGLGDDKLK

SEQ ID NO: 48988 - protein, 9 aa, synthetic construct
GGLGDDKLL

SEQ ID NO: 48989 - protein, 9 aa, synthetic construct
GGLGDDKLN

SEQ ID NO: 48990 - protein, 9 aa, synthetic construct
GGLGDDKLR

SEQ ID NO: 48991 - protein, 9 aa, synthetic construct
GGLGDDKLV

SEQ ID NO: 48992 - protein, 9 aa, synthetic construct
GGLGDDLMR

SEQ ID NO: 48993 - protein, 9 aa, synthetic construct
GGLGDDKMD

SEQ ID NO: 48994 - protein, 9 aa, synthetic construct
GGLGDDLFG

SEQ ID NO: 48995 - protein, 9 aa, synthetic construct
GGLGDDLFK

SEQ ID NO: 48996 - protein, 9 aa, synthetic construct
GGLGDDLFM

SEQ ID NO: 48997 - protein, 9 aa, synthetic construct
GGLGDDLFR

SEQ ID NO: 48998 - protein, 9 aa, synthetic construct
GGLGDDLIA

SEQ ID NO: 48999 - protein, 9 aa, synthetic construct
GGLGDDLIH

SEQ ID NO: 49000 - protein, 9 aa, synthetic construct
GGLGDDLMD

SEQ ID NO: 49001 - protein, 9 aa, synthetic construct
GGLGDDLME

SEQ ID NO: 49002 - protein, 9 aa, synthetic construct
GGLGDDLMF

SEQ ID NO: 49003 - protein, 9 aa, synthetic construct
GGLGDDLMI

SEQ ID NO: 49004 - protein, 9 aa, synthetic construct
GGLGDDLMN

SEQ ID NO: 49005 - protein, 9 aa, synthetic construct
GGLGDDLMQ

SEQ ID NO: 49006 - protein, 9 aa, synthetic construct
GGLGDDAIK

SEQ ID NO: 49007 - protein, 9 aa, synthetic construct
GGLGDDAAY

SEQ ID NO: 49008 - protein, 9 aa, synthetic construct
GGLGCDRMV

SEQ ID NO: 49009 - protein, 9 aa, synthetic construct
GGLGCDRLS

SEQ ID NO: 49010 - protein, 9 aa, synthetic construct
GGLGADQIR

SEQ ID NO: 49011 - protein, 9 aa, synthetic construct
GGLGADQLA

SEQ ID NO: 49012 - protein, 9 aa, synthetic construct
GGLGADQLD

SEQ ID NO: 49013 - protein, 9 aa, synthetic construct
GGLGADQLH

SEQ ID NO: 49014 - protein, 9 aa, synthetic construct
GGLGADQLL

SEQ ID NO: 49015 - protein, 9 aa, synthetic construct
GGLGADQLR

SEQ ID NO: 49016 - protein, 9 aa, synthetic construct
GGLGADQLS

SEQ ID NO: 49017 - protein, 9 aa, synthetic construct
GGLGADQLY

SEQ ID NO: 49018 - protein, 9 aa, synthetic construct
GGLGADQMA

SEQ ID NO: 49019 - protein, 9 aa, synthetic construct
GGLGADQMS

SEQ ID NO: 49020 - protein, 9 aa, synthetic construct
GGLGADQVF

SEQ ID NO: 49021 - protein, 9 aa, synthetic construct
GGLGADQVS

SEQ ID NO: 49022 - protein, 9 aa, synthetic construct
GGLGADQVW

SEQ ID NO: 49023 - protein, 9 aa, synthetic construct
GGLGADQYS

SEQ ID NO: 49024 - protein, 9 aa, synthetic construct
GGLGADRAE

SEQ ID NO: 49025 - protein, 9 aa, synthetic construct
GGLGADRFA

SEQ ID NO: 49026 - protein, 9 aa, synthetic construct
GGLGADRFM

SEQ ID NO: 49027 - protein, 9 aa, synthetic construct
GGLGADRID

SEQ ID NO: 49028 - protein, 9 aa, synthetic construct
GGLGADRLG

SEQ ID NO: 49029 - protein, 9 aa, synthetic construct
GGLGADRLH

SEQ ID NO: 49030 - protein, 9 aa, synthetic construct
GGLGADRLK

SEQ ID NO: 49031 - protein, 9 aa, synthetic construct
GGLGADRLQ

SEQ ID NO: 49032 - protein, 9 aa, synthetic construct
GGLGADRVR

SEQ ID NO: 49033 - protein, 9 aa, synthetic construct
GGLGADRYE

SEQ ID NO: 49034 - protein, 9 aa, synthetic construct
GGLGADSFD

SEQ ID NO: 49035 - protein, 9 aa, synthetic construct
GGLGADSFS

SEQ ID NO: 49036 - protein, 9 aa, synthetic construct
GGLGADSIG

SEQ ID NO: 49037 - protein, 9 aa, synthetic construct
GGLGADSIK

SEQ ID NO: 49038 - protein, 9 aa, synthetic construct
GGLGADSIN

SEQ ID NO: 49039 - protein, 9 aa, synthetic construct
GGLGADQID

SEQ ID NO: 49040 - protein, 9 aa, synthetic construct
GGLGADPLW

SEQ ID NO: 49041 - protein, 9 aa, synthetic construct
GGLGADPAL

SEQ ID NO: 49042 - protein, 9 aa, synthetic construct
GGLGADLYH

SEQ ID NO: 49043 - protein, 9 aa, synthetic construct
GGLGADKMA

SEQ ID NO: 49044 - protein, 9 aa, synthetic construct
GGLGADKMS

SEQ ID NO: 49045 - protein, 9 aa, synthetic construct
GGLGADKMW

SEQ ID NO: 49046 - protein, 9 aa, synthetic construct
GGLGADLFL

SEQ ID NO: 49047 - protein, 9 aa, synthetic construct
GGLGADLFR

SEQ ID NO: 49048 - protein, 9 aa, synthetic construct
GGLGADLIG

SEQ ID NO: 49049 - protein, 9 aa, synthetic construct
GGLGADLIN

SEQ ID NO: 49050 - protein, 9 aa, synthetic construct
GGLGADLIV

SEQ ID NO: 49051 - protein, 9 aa, synthetic construct
GGLGADLMA

SEQ ID NO: 49052 - protein, 9 aa, synthetic construct
GGLGADLMH

SEQ ID NO: 49053 - protein, 9 aa, synthetic construct
GGLGADLMK

SEQ ID NO: 49054 - protein, 9 aa, synthetic construct
GGLGADLMT

SEQ ID NO: 49055 - protein, 9 aa, synthetic construct
GGLGADLVQ

SEQ ID NO: 49056 - protein, 9 aa, synthetic construct
GGLGADLYR

SEQ ID NO: 49057 - protein, 9 aa, synthetic construct
GGLGADNMQ

SEQ ID NO: 49058 - protein, 9 aa, synthetic construct
GGLGADMFI

SEQ ID NO: 49059 - protein, 9 aa, synthetic construct
GGLGADMIF

SEQ ID NO: 49060 - protein, 9 aa, synthetic construct
GGLGADMLE

SEQ ID NO: 49061 - protein, 9 aa, synthetic construct
GGLGADMLH

SEQ ID NO: 49062 - protein, 9 aa, synthetic construct
GGLGADMLI

SEQ ID NO: 49063 - protein, 9 aa, synthetic construct
GGLGADMMI

SEQ ID NO: 49064 - protein, 9 aa, synthetic construct
GGLGADMMS

SEQ ID NO: 49065 - protein, 9 aa, synthetic construct
GGLGADMVY

SEQ ID NO: 49066 - protein, 9 aa, synthetic construct
GGLGADNLE

SEQ ID NO: 49067 - protein, 9 aa, synthetic construct
GGLGADNLH

SEQ ID NO: 49068 - protein, 9 aa, synthetic construct
GGLGADNLV

SEQ ID NO: 49069 - protein, 9 aa, synthetic construct
GGLGADNMA

SEQ ID NO: 49070 - protein, 9 aa, synthetic construct
GGLGADNMF

SEQ ID NO: 49071 - protein, 9 aa, synthetic construct
GGLGADSIS

SEQ ID NO: 49072 - protein, 9 aa, synthetic construct
GGLGADSLE

SEQ ID NO: 49073 - protein, 9 aa, synthetic construct
GGLGADSLF

SEQ ID NO: 49074 - protein, 9 aa, synthetic construct
GGLGADWIE

SEQ ID NO: 49075 - protein, 9 aa, synthetic construct
GGLGADVIQ

SEQ ID NO: 49076 - protein, 9 aa, synthetic construct
GGLGADVIT

SEQ ID NO: 49077 - protein, 9 aa, synthetic construct
GGLGADVMA

SEQ ID NO: 49078 - protein, 9 aa, synthetic construct
GGLGADVME

SEQ ID NO: 49079 - protein, 9 aa, synthetic construct
GGLGADVMF

SEQ ID NO: 49080 - protein, 9 aa, synthetic construct
GGLGADVMG

SEQ ID NO: 49081 - protein, 9 aa, synthetic construct
GGLGADVMH

SEQ ID NO: 49082 - protein, 9 aa, synthetic construct
GGLGADVMM

SEQ ID NO: 49083 - protein, 9 aa, synthetic construct
GGLGADVVD

SEQ ID NO: 49084 - protein, 9 aa, synthetic construct
GGLGADVVI

SEQ ID NO: 49085 - protein, 9 aa, synthetic construct
GGLGADVYI

SEQ ID NO: 49086 - protein, 9 aa, synthetic construct
GGLGADVYR

SEQ ID NO: 49087 - protein, 9 aa, synthetic construct
GGLGADVYV

SEQ ID NO: 49088 - protein, 9 aa, synthetic construct
GGLGADWIH

SEQ ID NO: 49089 - protein, 9 aa, synthetic construct
GGLGADVIH

SEQ ID NO: 49090 - protein, 9 aa, synthetic construct
GGLGADWIT

SEQ ID NO: 49091 - protein, 9 aa, synthetic construct
GGLGADWLS

SEQ ID NO: 49092 - protein, 9 aa, synthetic construct
GGLGADWLT

SEQ ID NO: 49093 - protein, 9 aa, synthetic construct
GGLGADWLV

SEQ ID NO: 49094 - protein, 9 aa, synthetic construct
GGLGADWLY

SEQ ID NO: 49095 - protein, 9 aa, synthetic construct
GGLGADWML

SEQ ID NO: 49096 - protein, 9 aa, synthetic construct
GGLGADWMT

SEQ ID NO: 49097 - protein, 9 aa, synthetic construct
GGLGADWVR

SEQ ID NO: 49098 - protein, 9 aa, synthetic construct
GGLGADYFQ

SEQ ID NO: 49099 - protein, 9 aa, synthetic construct
GGLGADYIE

SEQ ID NO: 49100 - protein, 9 aa, synthetic construct
GGLGADYLV

SEQ ID NO: 49101 - protein, 9 aa, synthetic construct
GGLGADYMD

SEQ ID NO: 49102 - protein, 9 aa, synthetic construct
GGLGADYYD

SEQ ID NO: 49103 - protein, 9 aa, synthetic construct
GGLGADVIL

SEQ ID NO: 49104 - protein, 9 aa, synthetic construct
GGLGADVIE

SEQ ID NO: 49105 - protein, 9 aa, synthetic construct
GGLGADSLG

SEQ ID NO: 49106 - protein, 9 aa, synthetic construct
GGLGADTFT

SEQ ID NO: 49107 - protein, 9 aa, synthetic construct
GGLGADSLK

SEQ ID NO: 49108 - protein, 9 aa, synthetic construct
GGLGADSMY

SEQ ID NO: 49109 - protein, 9 aa, synthetic construct
GGLGADSVE

SEQ ID NO: 49110 - protein, 9 aa, synthetic construct
GGLGADSVL

SEQ ID NO: 49111 - protein, 9 aa, synthetic construct
GGLGADSVN

SEQ ID NO: 49112 - protein, 9 aa, synthetic construct
GGLGADSVS

SEQ ID NO: 49113 - protein, 9 aa, synthetic construct
GGLGADSVY

SEQ ID NO: 49114 - protein, 9 aa, synthetic construct
GGLGADSYG

SEQ ID NO: 49115 - protein, 9 aa, synthetic construct
GGLGADSYW

SEQ ID NO: 49116 - protein, 9 aa, synthetic construct
GGLGADTAE

SEQ ID NO: 49117 - protein, 9 aa, synthetic construct
GGLGADTAT

SEQ ID NO: 49118 - protein, 9 aa, synthetic construct
GGLGADTFN

SEQ ID NO: 49119 - protein, 9 aa, synthetic construct
GGLGADTFQ

SEQ ID NO: 49120 - protein, 9 aa, synthetic construct
GGLGADTIH

SEQ ID NO: 49121 - protein, 9 aa, synthetic construct
GGLGADVIA

SEQ ID NO: 49122 - protein, 9 aa, synthetic construct
GGLGADTIW

SEQ ID NO: 49123 - protein, 9 aa, synthetic construct
GGLGADTLW

SEQ ID NO: 49124 - protein, 9 aa, synthetic construct
GGLGADTMG

SEQ ID NO: 49125 - protein, 9 aa, synthetic construct
GGLGADTMH

SEQ ID NO: 49126 - protein, 9 aa, synthetic construct
GGLGADTVA

SEQ ID NO: 49127 - protein, 9 aa, synthetic construct
GGLGADTVI

SEQ ID NO: 49128 - protein, 9 aa, synthetic construct
GGLGADTVL

SEQ ID NO: 49129 - protein, 9 aa, synthetic construct
GGLGADTVN

SEQ ID NO: 49130 - protein, 9 aa, synthetic construct
GGLGADTVS

SEQ ID NO: 49131 - protein, 9 aa, synthetic construct
GGLGADTYL

SEQ ID NO: 49132 - protein, 9 aa, synthetic construct
GGLGADVFD

SEQ ID NO: 49133 - protein, 9 aa, synthetic construct
GGLGADVFF

SEQ ID NO: 49134 - protein, 9 aa, synthetic construct
GGLGADVFI

SEQ ID NO: 49135 - protein, 9 aa, synthetic construct
GGKGQDWLY

SEQ ID NO: 49136 - protein, 9 aa, synthetic construct
GGKGQDWLS

SEQ ID NO: 49137 - protein, 9 aa, synthetic construct
GGKGQDWIH

SEQ ID NO: 49138 - protein, 9 aa, synthetic construct
GGKGGDKLN

SEQ ID NO: 49139 - protein, 9 aa, synthetic construct
GGKGEDTLD

SEQ ID NO: 49140 - protein, 9 aa, synthetic construct
GGKGEDTLL

SEQ ID NO: 49141 - protein, 9 aa, synthetic construct
GGKGEDTLV

SEQ ID NO: 49142 - protein, 9 aa, synthetic construct
GGYGYDVMI

SEQ ID NO: 49143 - protein, 9 aa, synthetic construct
GGKGEDTVD

SEQ ID NO: 49144 - protein, 9 aa, synthetic construct
GGKGEDVLH

SEQ ID NO: 49145 - protein, 9 aa, synthetic construct
GGKGEDVLQ

SEQ ID NO: 49146 - protein, 9 aa, synthetic construct
GGKGEDVLR

SEQ ID NO: 49147 - protein, 9 aa, synthetic construct
GGKGEDVVS

SEQ ID NO: 49148 - protein, 9 aa, synthetic construct
GGKGEDYID

SEQ ID NO: 49149 - protein, 9 aa, synthetic construct
GGKGFDEIK

SEQ ID NO: 49150 - protein, 9 aa, synthetic construct
GGKGFDFVV

SEQ ID NO: 49151 - protein, 9 aa, synthetic construct
GGKGFDLLI

SEQ ID NO: 49152 - protein, 9 aa, synthetic construct
GGKGFDRAY

SEQ ID NO: 49153 - protein, 9 aa, synthetic construct
GGKGFDSIV

SEQ ID NO: 49154 - protein, 9 aa, synthetic construct
GGKGFDSLI

SEQ ID NO: 49155 - protein, 9 aa, synthetic construct
GGKGFDSYI

SEQ ID NO: 49156 - protein, 9 aa, synthetic construct
GGKGFDTAE

SEQ ID NO: 49157 - protein, 9 aa, synthetic construct
GGKGFDTLR

SEQ ID NO: 49158 - protein, 9 aa, synthetic construct
GGKGFDTVV

SEQ ID NO: 49159 - protein, 9 aa, synthetic construct
GGKGFDVAS

SEQ ID NO: 49160 - protein, 9 aa, synthetic construct
GGKGGDAFA

SEQ ID NO: 49161 - protein, 9 aa, synthetic construct
GGKGGDALN

SEQ ID NO: 49162 - protein, 9 aa, synthetic construct
GGKGGDALV

SEQ ID NO: 49163 - protein, 9 aa, synthetic construct
GGKGGDFLD

SEQ ID NO: 49164 - protein, 9 aa, synthetic construct
GGKGGDFLL

SEQ ID NO: 49165 - protein, 9 aa, synthetic construct
GGKGGDIIQ

SEQ ID NO: 49166 - protein, 9 aa, synthetic construct
GGKGGDILI

SEQ ID NO: 49167 - protein, 9 aa, synthetic construct
GGKGGDKLH

SEQ ID NO: 49168 - protein, 9 aa, synthetic construct
GGKGEDTIN

SEQ ID NO: 49169 - protein, 9 aa, synthetic construct
GGKGEDTIK

SEQ ID NO: 49170 - protein, 9 aa, synthetic construct
GGKGEDTFV

SEQ ID NO: 49171 - protein, 9 aa, synthetic construct
GGKGEDDLN

SEQ ID NO: 49172 - protein, 9 aa, synthetic construct
GGKGDDVYN

SEQ ID NO: 49173 - protein, 9 aa, synthetic construct
GGKGDDVYQ

SEQ ID NO: 49174 - protein, 9 aa, synthetic construct
GGKGDDVYR

SEQ ID NO: 49175 - protein, 9 aa, synthetic construct
GGKGDDVYY

SEQ ID NO: 49176 - protein, 9 aa, synthetic construct
GGKGDDWLE

SEQ ID NO: 49177 - protein, 9 aa, synthetic construct
GGKGDDWLL

SEQ ID NO: 49178 - protein, 9 aa, synthetic construct
GGKGDDWLV

SEQ ID NO: 49179 - protein, 9 aa, synthetic construct
GGKGDDWVV

SEQ ID NO: 49180 - protein, 9 aa, synthetic construct
GGKGDDYIL

SEQ ID NO: 49181 - protein, 9 aa, synthetic construct
GGKGDDYLA

SEQ ID NO: 49182 - protein, 9 aa, synthetic construct
GGKGDDYMV

SEQ ID NO: 49183 - protein, 9 aa, synthetic construct
GGKGDDYYV

SEQ ID NO: 49184 - protein, 9 aa, synthetic construct
GGKGEDALE

SEQ ID NO: 49185 - protein, 9 aa, synthetic construct
GGKGEDDLY

SEQ ID NO: 49186 - protein, 9 aa, synthetic construct
GGKGEDTAE

SEQ ID NO: 49187 - protein, 9 aa, synthetic construct
GGKGEDELY

SEQ ID NO: 49188 - protein, 9 aa, synthetic construct
GGKGEDFLS

SEQ ID NO: 49189 - protein, 9 aa, synthetic construct
GGKGEDFVS

SEQ ID NO: 49190 - protein, 9 aa, synthetic construct
GGKGEDHIH

SEQ ID NO: 49191 - protein, 9 aa, synthetic construct
GGKGEDHLD

SEQ ID NO: 49192 - protein, 9 aa, synthetic construct
GGKGEDHLI

SEQ ID NO: 49193 - protein, 9 aa, synthetic construct
GGKGEDIFR

SEQ ID NO: 49194 - protein, 9 aa, synthetic construct
GGKGEDILF

SEQ ID NO: 49195 - protein, 9 aa, synthetic construct
GGKGEDILR

SEQ ID NO: 49196 - protein, 9 aa, synthetic construct
GGKGEDKLY

SEQ ID NO: 49197 - protein, 9 aa, synthetic construct
GGKGEDLIL

SEQ ID NO: 49198 - protein, 9 aa, synthetic construct
GGKGEDLLD

SEQ ID NO: 49199 - protein, 9 aa, synthetic construct
GGKGEDRLS

SEQ ID NO: 49200 - protein, 9 aa, synthetic construct
GGKGGDKLK

SEQ ID NO: 49201 - protein, 9 aa, synthetic construct
GGKGGDKLY

SEQ ID NO: 49202 - protein, 9 aa, synthetic construct
GGKGQDVLQ

SEQ ID NO: 49203 - protein, 9 aa, synthetic construct
GGKGGDLAV

SEQ ID NO: 49204 - protein, 9 aa, synthetic construct
GGKGHDIMT

SEQ ID NO: 49205 - protein, 9 aa, synthetic construct
GGKGHDIVN

SEQ ID NO: 49206 - protein, 9 aa, synthetic construct
GGKGHDKLY

SEQ ID NO: 49207 - protein, 9 aa, synthetic construct
GGKGHDKVD

SEQ ID NO: 49208 - protein, 9 aa, synthetic construct
GGKGHDLLA

SEQ ID NO: 49209 - protein, 9 aa, synthetic construct
GGKGHDLYI

SEQ ID NO: 49210 - protein, 9 aa, synthetic construct
GGKGHDNFV

SEQ ID NO: 49211 - protein, 9 aa, synthetic construct
GGKGHDRLE

SEQ ID NO: 49212 - protein, 9 aa, synthetic construct
GGKGHDRLF

SEQ ID NO: 49213 - protein, 9 aa, synthetic construct
GGKGHDRLI

SEQ ID NO: 49214 - protein, 9 aa, synthetic construct
GGKGHDSIA

SEQ ID NO: 49215 - protein, 9 aa, synthetic construct
GGKGHDSIS

SEQ ID NO: 49216 - protein, 9 aa, synthetic construct
GGKGHDSLL

SEQ ID NO: 49217 - protein, 9 aa, synthetic construct
GGKGHDSLN

SEQ ID NO: 49218 - protein, 9 aa, synthetic construct
GGKGHDTIL

SEQ ID NO: 49219 - protein, 9 aa, synthetic construct
GGKGHDTIR

SEQ ID NO: 49220 - protein, 9 aa, synthetic construct
GGKGHDTIY

SEQ ID NO: 49221 - protein, 9 aa, synthetic construct
GGKGHDTLK

SEQ ID NO: 49222 - protein, 9 aa, synthetic construct
GGKGHDTLM

SEQ ID NO: 49223 - protein, 9 aa, synthetic construct
GGKGHDTLS

SEQ ID NO: 49224 - protein, 9 aa, synthetic construct
GGKGHDTLT

SEQ ID NO: 49225 - protein, 9 aa, synthetic construct
GGKGHDTLY

SEQ ID NO: 49226 - protein, 9 aa, synthetic construct
GGKGHDVLD

SEQ ID NO: 49227 - protein, 9 aa, synthetic construct
GGKGHDVLI

SEQ ID NO: 49228 - protein, 9 aa, synthetic construct
GGKGHDVLK

SEQ ID NO: 49229 - protein, 9 aa, synthetic construct
GGKGHDVVN

SEQ ID NO: 49230 - protein, 9 aa, synthetic construct
GGKGHDVYV

SEQ ID NO: 49231 - protein, 9 aa, synthetic construct
GGKGHDWLF

SEQ ID NO: 49232 - protein, 9 aa, synthetic construct
GGKGHDWVS

SEQ ID NO: 49233 - protein, 9 aa, synthetic construct
GGKGHDILK

SEQ ID NO: 49234 - protein, 9 aa, synthetic construct
GGKGHDIIA

SEQ ID NO: 49235 - protein, 9 aa, synthetic construct
GGKGHDIAR

SEQ ID NO: 49236 - protein, 9 aa, synthetic construct
GGKGGDTLT

SEQ ID NO: 49237 - protein, 9 aa, synthetic construct
GGKGGDLIE

SEQ ID NO: 49238 - protein, 9 aa, synthetic construct
GGKGGDLLC

SEQ ID NO: 49239 - protein, 9 aa, synthetic construct
GGKGGDLLL

SEQ ID NO: 49240 - protein, 9 aa, synthetic construct
GGKGGDLLS

SEQ ID NO: 49241 - protein, 9 aa, synthetic construct
GGKGGDLLY

SEQ ID NO: 49242 - protein, 9 aa, synthetic construct
GGKGGDLMQ

SEQ ID NO: 49243 - protein, 9 aa, synthetic construct
GGKGGDMIA

SEQ ID NO: 49244 - protein, 9 aa, synthetic construct
GGKGGDRLE

SEQ ID NO: 49245 - protein, 9 aa, synthetic construct
GGKGGDRLF

SEQ ID NO: 49246 - protein, 9 aa, synthetic construct
GGKGGDRVH

SEQ ID NO: 49247 - protein, 9 aa, synthetic construct
GGKGGDSLR

SEQ ID NO: 49248 - protein, 9 aa, synthetic construct
GGKGGDTLF

SEQ ID NO: 49249 - protein, 9 aa, synthetic construct
GGKGGDTLN

SEQ ID NO: 49250 - protein, 9 aa, synthetic construct
GGKGGDTLY

SEQ ID NO: 49251 - protein, 9 aa, synthetic construct
GGKGHDHLD

SEQ ID NO: 49252 - protein, 9 aa, synthetic construct
GGKGGDTMV

SEQ ID NO: 49253 - protein, 9 aa, synthetic construct
GGKGGDTYI

SEQ ID NO: 49254 - protein, 9 aa, synthetic construct
GGKGGDTYL

SEQ ID NO: 49255 - protein, 9 aa, synthetic construct
GGKGGDTYV

SEQ ID NO: 49256 - protein, 9 aa, synthetic construct
GGKGGDVLE

SEQ ID NO: 49257 - protein, 9 aa, synthetic construct
GGKGGDVLM

SEQ ID NO: 49258 - protein, 9 aa, synthetic construct
GGKGGDVLW

SEQ ID NO: 49259 - protein, 9 aa, synthetic construct
GGKGHDAFD

SEQ ID NO: 49260 - protein, 9 aa, synthetic construct
GGKGHDALN

SEQ ID NO: 49261 - protein, 9 aa, synthetic construct
GGKGHDELF

SEQ ID NO: 49262 - protein, 9 aa, synthetic construct
GGKGHDFVS

SEQ ID NO: 49263 - protein, 9 aa, synthetic construct
GGKGHDFYI

SEQ ID NO: 49264 - protein, 9 aa, synthetic construct
GGKGHDHIQ

SEQ ID NO: 49265 - protein, 9 aa, synthetic construct
GGKGDDVYL

SEQ ID NO: 49266 - protein, 9 aa, synthetic construct
GGKGDDVMV

SEQ ID NO: 49267 - protein, 9 aa, synthetic construct
GGKGDDVMI

SEQ ID NO: 49268 - protein, 9 aa, synthetic construct
GGKGDDVMF

SEQ ID NO: 49269 - protein, 9 aa, synthetic construct
GGKGDDIIE

SEQ ID NO: 49270 - protein, 9 aa, synthetic construct
GGKGDDIIV

SEQ ID NO: 49271 - protein, 9 aa, synthetic construct
GGKGDDIIW

SEQ ID NO: 49272 - protein, 9 aa, synthetic construct
GGKGDDILG

SEQ ID NO: 49273 - protein, 9 aa, synthetic construct
GGKGDDILW

SEQ ID NO: 49274 - protein, 9 aa, synthetic construct
GGKGDDIMS

SEQ ID NO: 49275 - protein, 9 aa, synthetic construct
GGKGDDIMW

SEQ ID NO: 49276 - protein, 9 aa, synthetic construct
GGKGDDIVE

SEQ ID NO: 49277 - protein, 9 aa, synthetic construct
GGKGDDIVK

SEQ ID NO: 49278 - protein, 9 aa, synthetic construct
GGKGDDIVL

SEQ ID NO: 49279 - protein, 9 aa, synthetic construct
GGKGDDIVN

SEQ ID NO: 49280 - protein, 9 aa, synthetic construct
GGKGDDIYE

SEQ ID NO: 49281 - protein, 9 aa, synthetic construct
GGKGDDKIN

SEQ ID NO: 49282 - protein, 9 aa, synthetic construct
GGKGDDKIY

SEQ ID NO: 49283 - protein, 9 aa, synthetic construct
GGKGDDKLA

SEQ ID NO: 49284 - protein, 9 aa, synthetic construct
GGKGDDKLE

SEQ ID NO: 49285 - protein, 9 aa, synthetic construct
GGKGDDKLH

SEQ ID NO: 49286 - protein, 9 aa, synthetic construct
GGKGDDKLS

SEQ ID NO: 49287 - protein, 9 aa, synthetic construct
GGKGDDKLV

SEQ ID NO: 49288 - protein, 9 aa, synthetic construct
GGKGDDKMD

SEQ ID NO: 49289 - protein, 9 aa, synthetic construct
GGKGDDLFV

SEQ ID NO: 49290 - protein, 9 aa, synthetic construct
GGKGDDLID

SEQ ID NO: 49291 - protein, 9 aa, synthetic construct
GGKGDDLIK

SEQ ID NO: 49292 - protein, 9 aa, synthetic construct
GGKGDDLLQ

SEQ ID NO: 49293 - protein, 9 aa, synthetic construct
GGKGDDLML

SEQ ID NO: 49294 - protein, 9 aa, synthetic construct
GGKGDDLMM

SEQ ID NO: 49295 - protein, 9 aa, synthetic construct
GGKGDDLMS

SEQ ID NO: 49296 - protein, 9 aa, synthetic construct
GGKGDDLVF

SEQ ID NO: 49297 - protein, 9 aa, synthetic construct
GGKGDDLVH

SEQ ID NO: 49298 - protein, 9 aa, synthetic construct
GGKGDDIIA

SEQ ID NO: 49299 - protein, 9 aa, synthetic construct
GGKGDDHYY

SEQ ID NO: 49300 - protein, 9 aa, synthetic construct
GGKGDDHYI

SEQ ID NO: 49301 - protein, 9 aa, synthetic construct
GGKGDDFIS

SEQ ID NO: 49302 - protein, 9 aa, synthetic construct
GGKGDDDLI

SEQ ID NO: 49303 - protein, 9 aa, synthetic construct
GGKGDDDLN

SEQ ID NO: 49304 - protein, 9 aa, synthetic construct
GGKGDDDMR

SEQ ID NO: 49305 - protein, 9 aa, synthetic construct
GGKGDDELC

SEQ ID NO: 49306 - protein, 9 aa, synthetic construct
GGKGDDELD

SEQ ID NO: 49307 - protein, 9 aa, synthetic construct
GGKGDDELK

SEQ ID NO: 49308 - protein, 9 aa, synthetic construct
GGKGDDELN

SEQ ID NO: 49309 - protein, 9 aa, synthetic construct
GGKGDDEVH

SEQ ID NO: 49310 - protein, 9 aa, synthetic construct
GGKGDDEVR

SEQ ID NO: 49311 - protein, 9 aa, synthetic construct
GGKGDDFAD

SEQ ID NO: 49312 - protein, 9 aa, synthetic construct
GGKGDDFFD

SEQ ID NO: 49313 - protein, 9 aa, synthetic construct
GGKGDDFIF

SEQ ID NO: 49314 - protein, 9 aa, synthetic construct
GGKGDDFII

SEQ ID NO: 49315 - protein, 9 aa, synthetic construct
GGKGDDFIY

SEQ ID NO: 49316 - protein, 9 aa, synthetic construct
GGKGDDHVV

SEQ ID NO: 49317 - protein, 9 aa, synthetic construct
GGKGDDFLL

SEQ ID NO: 49318 - protein, 9 aa, synthetic construct
GGKGDDFVH

SEQ ID NO: 49319 - protein, 9 aa, synthetic construct
GGKGDDFVS

SEQ ID NO: 49320 - protein, 9 aa, synthetic construct
GGKGDDGFD

SEQ ID NO: 49321 - protein, 9 aa, synthetic construct
GGKGDDGIH

SEQ ID NO: 49322 - protein, 9 aa, synthetic construct
GGKGDDGLH

SEQ ID NO: 49323 - protein, 9 aa, synthetic construct
GGKGDDGYI

SEQ ID NO: 49324 - protein, 9 aa, synthetic construct
GGKGDDHIE

SEQ ID NO: 49325 - protein, 9 aa, synthetic construct
GGKGDDHLK

SEQ ID NO: 49326 - protein, 9 aa, synthetic construct
GGKGDDHLM

SEQ ID NO: 49327 - protein, 9 aa, synthetic construct
GGKGDDHLS

SEQ ID NO: 49328 - protein, 9 aa, synthetic construct
GGKGDDHLT

SEQ ID NO: 49329 - protein, 9 aa, synthetic construct
GGKGDDHME

SEQ ID NO: 49330 - protein, 9 aa, synthetic construct
GGKGDDLVV

SEQ ID NO: 49331 - protein, 9 aa, synthetic construct
GGKGDDLYI

SEQ ID NO: 49332 - protein, 9 aa, synthetic construct
GGKGDDLYV

SEQ ID NO: 49333 - protein, 9 aa, synthetic construct
GGKGDDTYQ

SEQ ID NO: 49334 - protein, 9 aa, synthetic construct
GGKGDDTFI

SEQ ID NO: 49335 - protein, 9 aa, synthetic construct
GGKGDDTIE

SEQ ID NO: 49336 - protein, 9 aa, synthetic construct
GGKGDDTIH

SEQ ID NO: 49337 - protein, 9 aa, synthetic construct
GGKGDDTIW

SEQ ID NO: 49338 - protein, 9 aa, synthetic construct
GGKGDDTLN

SEQ ID NO: 49339 - protein, 9 aa, synthetic construct
GGKGDDTLQ

SEQ ID NO: 49340 - protein, 9 aa, synthetic construct
GGKGDDTMN

SEQ ID NO: 49341 - protein, 9 aa, synthetic construct
GGKGDDTMR

SEQ ID NO: 49342 - protein, 9 aa, synthetic construct
GGKGDDTYA

SEQ ID NO: 49343 - protein, 9 aa, synthetic construct
GGKGDDTYD

SEQ ID NO: 49344 - protein, 9 aa, synthetic construct
GGKGDDTYG

SEQ ID NO: 49345 - protein, 9 aa, synthetic construct
GGKGDDTYH

SEQ ID NO: 49346 - protein, 9 aa, synthetic construct
GGKGDDTYM

SEQ ID NO: 49347 - protein, 9 aa, synthetic construct
GGKGDDTYR

SEQ ID NO: 49348 - protein, 9 aa, synthetic construct
GGKGDDSYI

SEQ ID NO: 49349 - protein, 9 aa, synthetic construct
GGKGDDVAD

SEQ ID NO: 49350 - protein, 9 aa, synthetic construct
GGKGDDVAN

SEQ ID NO: 49351 - protein, 9 aa, synthetic construct
GGKGDDVAS

SEQ ID NO: 49352 - protein, 9 aa, synthetic construct
GGKGDDVFK

SEQ ID NO: 49353 - protein, 9 aa, synthetic construct
GGKGDDVFM

SEQ ID NO: 49354 - protein, 9 aa, synthetic construct
GGKGDDVFR

SEQ ID NO: 49355 - protein, 9 aa, synthetic construct
GGKGDDVIG

SEQ ID NO: 49356 - protein, 9 aa, synthetic construct
GGKGDDVIH

SEQ ID NO: 49357 - protein, 9 aa, synthetic construct
GGKGDDVIL

SEQ ID NO: 49358 - protein, 9 aa, synthetic construct
GGKGDDVIN

SEQ ID NO: 49359 - protein, 9 aa, synthetic construct
GGKGDDVIS

SEQ ID NO: 49360 - protein, 9 aa, synthetic construct
GGKGDDVIT

SEQ ID NO: 49361 - protein, 9 aa, synthetic construct
GGKGDDVIY

SEQ ID NO: 49362 - protein, 9 aa, synthetic construct
GGKGDDTAI

SEQ ID NO: 49363 - protein, 9 aa, synthetic construct
GGKGDDSVY

SEQ ID NO: 49364 - protein, 9 aa, synthetic construct
GGKGDDLYY

SEQ ID NO: 49365 - protein, 9 aa, synthetic construct
GGKGDDRII

SEQ ID NO: 49366 - protein, 9 aa, synthetic construct
GGKGDDMLT

SEQ ID NO: 49367 - protein, 9 aa, synthetic construct
GGKGDDMVW

SEQ ID NO: 49368 - protein, 9 aa, synthetic construct
GGKGDDNII

SEQ ID NO: 49369 - protein, 9 aa, synthetic construct
GGKGDDNIK

SEQ ID NO: 49370 - protein, 9 aa, synthetic construct
GGKGDDNIQ

SEQ ID NO: 49371 - protein, 9 aa, synthetic construct
GGKGDDNLI

SEQ ID NO: 49372 - protein, 9 aa, synthetic construct
GGKGDDQID

SEQ ID NO: 49373 - protein, 9 aa, synthetic construct
GGKGDDQLS

SEQ ID NO: 49374 - protein, 9 aa, synthetic construct
GGKGDDQLW

SEQ ID NO: 49375 - protein, 9 aa, synthetic construct
GGKGDDRAK

SEQ ID NO: 49376 - protein, 9 aa, synthetic construct
GGKGDDRFH

SEQ ID NO: 49377 - protein, 9 aa, synthetic construct
GGKGDDRIE

SEQ ID NO: 49378 - protein, 9 aa, synthetic construct
GGKGDDRIG

SEQ ID NO: 49379 - protein, 9 aa, synthetic construct
GGKGDDRIQ

SEQ ID NO: 49380 - protein, 9 aa, synthetic construct
GGKGDDSVN

SEQ ID NO: 49381 - protein, 9 aa, synthetic construct
GGKGDDRIV

SEQ ID NO: 49382 - protein, 9 aa, synthetic construct
GGKGDDRLL

SEQ ID NO: 49383 - protein, 9 aa, synthetic construct
GGKGDDRLW

SEQ ID NO: 49384 - protein, 9 aa, synthetic construct
GGKGDDRYE

SEQ ID NO: 49385 - protein, 9 aa, synthetic construct
GGKGDDSFE

SEQ ID NO: 49386 - protein, 9 aa, synthetic construct
GGKGDDSIN

SEQ ID NO: 49387 - protein, 9 aa, synthetic construct
GGKGDDSIR

SEQ ID NO: 49388 - protein, 9 aa, synthetic construct
GGKGDDSLI

SEQ ID NO: 49389 - protein, 9 aa, synthetic construct
GGKGDDSLR

SEQ ID NO: 49390 - protein, 9 aa, synthetic construct
GGKGDDSLT

SEQ ID NO: 49391 - protein, 9 aa, synthetic construct
GGKGDDSVE

SEQ ID NO: 49392 - protein, 9 aa, synthetic construct
GGKGDDSVI

SEQ ID NO: 49393 - protein, 9 aa, synthetic construct
GGKGDDSVL

SEQ ID NO: 49394 - protein, 9 aa, synthetic construct
GGKGIDELS

SEQ ID NO: 49395 - protein, 9 aa, synthetic construct
GGKGIDFLF

SEQ ID NO: 49396 - protein, 9 aa, synthetic construct
GGKGIDILF

SEQ ID NO: 49397 - protein, 9 aa, synthetic construct
GGKGNDGVN

SEQ ID NO: 49398 - protein, 9 aa, synthetic construct
GGKGNDQLL

SEQ ID NO: 49399 - protein, 9 aa, synthetic construct
GGKGNDQLN

SEQ ID NO: 49400 - protein, 9 aa, synthetic construct
GGKGNDQLW

SEQ ID NO: 49401 - protein, 9 aa, synthetic construct
GGKGNDQMH

SEQ ID NO: 49402 - protein, 9 aa, synthetic construct
GGKGNDQMT

SEQ ID NO: 49403 - protein, 9 aa, synthetic construct
GGKGNDQVF

SEQ ID NO: 49404 - protein, 9 aa, synthetic construct
GGKGNDQVH

SEQ ID NO: 49405 - protein, 9 aa, synthetic construct
GGKGNDQYQ

SEQ ID NO: 49406 - protein, 9 aa, synthetic construct
GGKGNDRFF

SEQ ID NO: 49407 - protein, 9 aa, synthetic construct
GGKGNDRFW

SEQ ID NO: 49408 - protein, 9 aa, synthetic construct
GGKGNDRIE

SEQ ID NO: 49409 - protein, 9 aa, synthetic construct
GGKGNDRIN

SEQ ID NO: 49410 - protein, 9 aa, synthetic construct
GGKGNDRLF

SEQ ID NO: 49411 - protein, 9 aa, synthetic construct
GGKGNDRLR

SEQ ID NO: 49412 - protein, 9 aa, synthetic construct
GGKGNDRMM

SEQ ID NO: 49413 - protein, 9 aa, synthetic construct
GGKGNDRMV

SEQ ID NO: 49414 - protein, 9 aa, synthetic construct
GGKGNDRVF

SEQ ID NO: 49415 - protein, 9 aa, synthetic construct
GGKGNDRYI

SEQ ID NO: 49416 - protein, 9 aa, synthetic construct
GGKGNDRYV

SEQ ID NO: 49417 - protein, 9 aa, synthetic construct
GGKGNDSAL

SEQ ID NO: 49418 - protein, 9 aa, synthetic construct
GGKGNDSIV

SEQ ID NO: 49419 - protein, 9 aa, synthetic construct
GGKGNDSLA

SEQ ID NO: 49420 - protein, 9 aa, synthetic construct
GGKGNDSLR

SEQ ID NO: 49421 - protein, 9 aa, synthetic construct
GGKGNDSLW

SEQ ID NO: 49422 - protein, 9 aa, synthetic construct
GGKGNDSVV

SEQ ID NO: 49423 - protein, 9 aa, synthetic construct
GGKGNDSYR

SEQ ID NO: 49424 - protein, 9 aa, synthetic construct
GGKGNDSYW

SEQ ID NO: 49425 - protein, 9 aa, synthetic construct
GGKGNDTAL

SEQ ID NO: 49426 - protein, 9 aa, synthetic construct
GGKGNDTAS

SEQ ID NO: 49427 - protein, 9 aa, synthetic construct
GGKGNDQLH

SEQ ID NO: 49428 - protein, 9 aa, synthetic construct
GGKGNDQIY

SEQ ID NO: 49429 - protein, 9 aa, synthetic construct
GGKGNDNLN

SEQ ID NO: 49430 - protein, 9 aa, synthetic construct
GGKGNDKMD

SEQ ID NO: 49431 - protein, 9 aa, synthetic construct
GGKGNDHLL

SEQ ID NO: 49432 - protein, 9 aa, synthetic construct
GGKGNDIFS

SEQ ID NO: 49433 - protein, 9 aa, synthetic construct
GGKGNDIID

SEQ ID NO: 49434 - protein, 9 aa, synthetic construct
GGKGNDIIN

SEQ ID NO: 49435 - protein, 9 aa, synthetic construct
GGKGNDIIR

SEQ ID NO: 49436 - protein, 9 aa, synthetic construct
GGKGNDILW

SEQ ID NO: 49437 - protein, 9 aa, synthetic construct
GGKGNDIVR

SEQ ID NO: 49438 - protein, 9 aa, synthetic construct
GGKGNDIVY

SEQ ID NO: 49439 - protein, 9 aa, synthetic construct
GGKGNDIYG

SEQ ID NO: 49440 - protein, 9 aa, synthetic construct
GGKGNDIYK

SEQ ID NO: 49441 - protein, 9 aa, synthetic construct
GGKGNDKIF

SEQ ID NO: 49442 - protein, 9 aa, synthetic construct
GGKGNDKLL

SEQ ID NO: 49443 - protein, 9 aa, synthetic construct
GGKGNDKLW

SEQ ID NO: 49444 - protein, 9 aa, synthetic construct
GGKGNDKMV

SEQ ID NO: 49445 - protein, 9 aa, synthetic construct
GGKGNDNLM

SEQ ID NO: 49446 - protein, 9 aa, synthetic construct
GGKGNDKYV

SEQ ID NO: 49447 - protein, 9 aa, synthetic construct
GGKGNDLIY

SEQ ID NO: 49448 - protein, 9 aa, synthetic construct
GGKGNDLLE

SEQ ID NO: 49449 - protein, 9 aa, synthetic construct
GGKGNDLLM

SEQ ID NO: 49450 - protein, 9 aa, synthetic construct
GGKGNDLMI

SEQ ID NO: 49451 - protein, 9 aa, synthetic construct
GGKGNDLMS

SEQ ID NO: 49452 - protein, 9 aa, synthetic construct
GGKGNDLVH

SEQ ID NO: 49453 - protein, 9 aa, synthetic construct
GGKGNDLYF

SEQ ID NO: 49454 - protein, 9 aa, synthetic construct
GGKGNDMLI

SEQ ID NO: 49455 - protein, 9 aa, synthetic construct
GGKGNDMLY

SEQ ID NO: 49456 - protein, 9 aa, synthetic construct
GGKGNDNIQ

SEQ ID NO: 49457 - protein, 9 aa, synthetic construct
GGKGNDNIR

SEQ ID NO: 49458 - protein, 9 aa, synthetic construct
GGKGNDNIS

SEQ ID NO: 49459 - protein, 9 aa, synthetic construct
GGKGNDTAT

SEQ ID NO: 49460 - protein, 9 aa, synthetic construct
GGKGNDTAV

SEQ ID NO: 49461 - protein, 9 aa, synthetic construct
GGKGNDTFD

SEQ ID NO: 49462 - protein, 9 aa, synthetic construct
GGKGQDLMS

SEQ ID NO: 49463 - protein, 9 aa, synthetic construct
GGKGNDYLL

SEQ ID NO: 49464 - protein, 9 aa, synthetic construct
GGKGNDYLT

SEQ ID NO: 49465 - protein, 9 aa, synthetic construct
GGKGNDYMS

SEQ ID NO: 49466 - protein, 9 aa, synthetic construct
GGKGPDILS

SEQ ID NO: 49467 - protein, 9 aa, synthetic construct
GGKGPDLIE

SEQ ID NO: 49468 - protein, 9 aa, synthetic construct
GGKGPDTIF

SEQ ID NO: 49469 - protein, 9 aa, synthetic construct
GGKGPDVLD

SEQ ID NO: 49470 - protein, 9 aa, synthetic construct
GGKGQDAFV

SEQ ID NO: 49471 - protein, 9 aa, synthetic construct
GGKGQDELT

SEQ ID NO: 49472 - protein, 9 aa, synthetic construct
GGKGQDFIV

SEQ ID NO: 49473 - protein, 9 aa, synthetic construct
GGKGQDGLY

SEQ ID NO: 49474 - protein, 9 aa, synthetic construct
GGKGQDLLD

SEQ ID NO: 49475 - protein, 9 aa, synthetic construct
GGKGQDLLH

SEQ ID NO: 49476 - protein, 9 aa, synthetic construct
GGKGQDQLF

SEQ ID NO: 49477 - protein, 9 aa, synthetic construct
GGKGNDYIW

SEQ ID NO: 49478 - protein, 9 aa, synthetic construct
GGKGQDRIA

SEQ ID NO: 49479 - protein, 9 aa, synthetic construct
GGKGQDSIN

SEQ ID NO: 49480 - protein, 9 aa, synthetic construct
GGKGQDTAH

SEQ ID NO: 49481 - protein, 9 aa, synthetic construct
GGKGQDTFF

SEQ ID NO: 49482 - protein, 9 aa, synthetic construct
GGKGQDTLE

SEQ ID NO: 49483 - protein, 9 aa, synthetic construct
GGKGQDTLF

SEQ ID NO: 49484 - protein, 9 aa, synthetic construct
GGKGQDTLH

SEQ ID NO: 49485 - protein, 9 aa, synthetic construct
GGKGQDTLL

SEQ ID NO: 49486 - protein, 9 aa, synthetic construct
GGKGQDTLY

SEQ ID NO: 49487 - protein, 9 aa, synthetic construct
GGKGQDTMD

SEQ ID NO: 49488 - protein, 9 aa, synthetic construct
GGKGQDTVT

SEQ ID NO: 49489 - protein, 9 aa, synthetic construct
GGKGQDVFV

SEQ ID NO: 49490 - protein, 9 aa, synthetic construct
GGKGQDVLI

SEQ ID NO: 49491 - protein, 9 aa, synthetic construct
GGKGNDYLF

SEQ ID NO: 49492 - protein, 9 aa, synthetic construct
GGKGNDYIE

SEQ ID NO: 49493 - protein, 9 aa, synthetic construct
GGKGNDTFI

SEQ ID NO: 49494 - protein, 9 aa, synthetic construct
GGKGNDVFD

SEQ ID NO: 49495 - protein, 9 aa, synthetic construct
GGKGNDTFK

SEQ ID NO: 49496 - protein, 9 aa, synthetic construct
GGKGNDTFL

SEQ ID NO: 49497 - protein, 9 aa, synthetic construct
GGKGNDTIA

SEQ ID NO: 49498 - protein, 9 aa, synthetic construct
GGKGNDTIS

SEQ ID NO: 49499 - protein, 9 aa, synthetic construct
GGKGNDTLG

SEQ ID NO: 49500 - protein, 9 aa, synthetic construct
GGKGNDTLQ

SEQ ID NO: 49501 - protein, 9 aa, synthetic construct
GGKGNDTMN

SEQ ID NO: 49502 - protein, 9 aa, synthetic construct
GGKGNDTMQ

SEQ ID NO: 49503 - protein, 9 aa, synthetic construct
GGKGNDTVF

SEQ ID NO: 49504 - protein, 9 aa, synthetic construct
GGKGNDTVK

SEQ ID NO: 49505 - protein, 9 aa, synthetic construct
GGKGNDTVW

SEQ ID NO: 49506 - protein, 9 aa, synthetic construct
GGKGNDVAD

SEQ ID NO: 49507 - protein, 9 aa, synthetic construct
GGKGNDVAS

SEQ ID NO: 49508 - protein, 9 aa, synthetic construct
GGKGNDVFE

SEQ ID NO: 49509 - protein, 9 aa, synthetic construct
GGKGNDWVQ

SEQ ID NO: 49510 - protein, 9 aa, synthetic construct
GGKGNDVIE

SEQ ID NO: 49511 - protein, 9 aa, synthetic construct
GGKGNDVIV

SEQ ID NO: 49512 - protein, 9 aa, synthetic construct
GGKGNDVLF

SEQ ID NO: 49513 - protein, 9 aa, synthetic construct
GGKGNDVLG

SEQ ID NO: 49514 - protein, 9 aa, synthetic construct
GGKGNDVMA

SEQ ID NO: 49515 - protein, 9 aa, synthetic construct
GGKGNDVML

SEQ ID NO: 49516 - protein, 9 aa, synthetic construct
GGKGNDVMN

SEQ ID NO: 49517 - protein, 9 aa, synthetic construct
GGKGNDWIS

SEQ ID NO: 49518 - protein, 9 aa, synthetic construct
GGKGNDWLH

SEQ ID NO: 49519 - protein, 9 aa, synthetic construct
GGKGNDWLI

SEQ ID NO: 49520 - protein, 9 aa, synthetic construct
GGKGNDWLL

SEQ ID NO: 49521 - protein, 9 aa, synthetic construct
GGKGNDWLQ

SEQ ID NO: 49522 - protein, 9 aa, synthetic construct
GGKGNDWLS

SEQ ID NO: 49523 - protein, 9 aa, synthetic construct
GGKGNDHIF

SEQ ID NO: 49524 - protein, 9 aa, synthetic construct
GGKGNDGLD

SEQ ID NO: 49525 - protein, 9 aa, synthetic construct
GGKGIDLAV

SEQ ID NO: 49526 - protein, 9 aa, synthetic construct
GGKGNDGIN

SEQ ID NO: 49527 - protein, 9 aa, synthetic construct
GGKGKDKLY

SEQ ID NO: 49528 - protein, 9 aa, synthetic construct
GGKGKDKMS

SEQ ID NO: 49529 - protein, 9 aa, synthetic construct
GGKGKDLLF

SEQ ID NO: 49530 - protein, 9 aa, synthetic construct
GGKGKDLLK

SEQ ID NO: 49531 - protein, 9 aa, synthetic construct
GGKGKDLLL

SEQ ID NO: 49532 - protein, 9 aa, synthetic construct
GGKGKDLLQ

SEQ ID NO: 49533 - protein, 9 aa, synthetic construct
GGKGKDLLT

SEQ ID NO: 49534 - protein, 9 aa, synthetic construct
GGKGKDMLT

SEQ ID NO: 49535 - protein, 9 aa, synthetic construct
GGKGKDNIN

SEQ ID NO: 49536 - protein, 9 aa, synthetic construct
GGKGKDNLT

SEQ ID NO: 49537 - protein, 9 aa, synthetic construct
GGKGKDNMH

SEQ ID NO: 49538 - protein, 9 aa, synthetic construct
GGKGKDQLD

SEQ ID NO: 49539 - protein, 9 aa, synthetic construct
GGKGKDQLR

SEQ ID NO: 49540 - protein, 9 aa, synthetic construct
GGKGKDQLT

SEQ ID NO: 49541 - protein, 9 aa, synthetic construct
GGKGKDQYY

SEQ ID NO: 49542 - protein, 9 aa, synthetic construct
GGKGKDRIE

SEQ ID NO: 49543 - protein, 9 aa, synthetic construct
GGKGKDRLA

SEQ ID NO: 49544 - protein, 9 aa, synthetic construct
GGKGKDRLD

SEQ ID NO: 49545 - protein, 9 aa, synthetic construct
GGKGKDRLI

SEQ ID NO: 49546 - protein, 9 aa, synthetic construct
GGKGKDRLY

SEQ ID NO: 49547 - protein, 9 aa, synthetic construct
GGKGKDSIL

SEQ ID NO: 49548 - protein, 9 aa, synthetic construct
GGKGKDSLF

SEQ ID NO: 49549 - protein, 9 aa, synthetic construct
GGKGKDSLT

SEQ ID NO: 49550 - protein, 9 aa, synthetic construct
GGKGKDTAI

SEQ ID NO: 49551 - protein, 9 aa, synthetic construct
GGKGKDTFN

SEQ ID NO: 49552 - protein, 9 aa, synthetic construct
GGKGKDTFT

SEQ ID NO: 49553 - protein, 9 aa, synthetic construct
GGKGKDTLD

SEQ ID NO: 49554 - protein, 9 aa, synthetic construct
GGKGKDTLI

SEQ ID NO: 49555 - protein, 9 aa, synthetic construct
GGKGKDTLV

SEQ ID NO: 49556 - protein, 9 aa, synthetic construct
GGKGKDKLW

SEQ ID NO: 49557 - protein, 9 aa, synthetic construct
GGKGKDKLF

SEQ ID NO: 49558 - protein, 9 aa, synthetic construct
GGKGKDKLD

SEQ ID NO: 49559 - protein, 9 aa, synthetic construct
GGKGKDDIS

SEQ ID NO: 49560 - protein, 9 aa, synthetic construct
GGKGIDRLD

SEQ ID NO: 49561 - protein, 9 aa, synthetic construct
GGKGIDRLN

SEQ ID NO: 49562 - protein, 9 aa, synthetic construct
GGKGIDSII

SEQ ID NO: 49563 - protein, 9 aa, synthetic construct
GGKGIDSLE

SEQ ID NO: 49564 - protein, 9 aa, synthetic construct
GGKGIDSLF

SEQ ID NO: 49565 - protein, 9 aa, synthetic construct
GGKGIDTAD

SEQ ID NO: 49566 - protein, 9 aa, synthetic construct
GGKGIDTAV

SEQ ID NO: 49567 - protein, 9 aa, synthetic construct
GGKGIDTFV

SEQ ID NO: 49568 - protein, 9 aa, synthetic construct
GGKGIDTLS

SEQ ID NO: 49569 - protein, 9 aa, synthetic construct
GGKGIDTLV

SEQ ID NO: 49570 - protein, 9 aa, synthetic construct
GGKGIDVLK

SEQ ID NO: 49571 - protein, 9 aa, synthetic construct
GGKGKDAFI

SEQ ID NO: 49572 - protein, 9 aa, synthetic construct
GGKGKDAID

SEQ ID NO: 49573 - protein, 9 aa, synthetic construct
GGKGKDDLK

SEQ ID NO: 49574 - protein, 9 aa, synthetic construct
GGKGKDKIE

SEQ ID NO: 49575 - protein, 9 aa, synthetic construct
GGKGKDEID

SEQ ID NO: 49576 - protein, 9 aa, synthetic construct
GGKGKDELI

SEQ ID NO: 49577 - protein, 9 aa, synthetic construct
GGKGKDEMD

SEQ ID NO: 49578 - protein, 9 aa, synthetic construct
GGKGKDEMT

SEQ ID NO: 49579 - protein, 9 aa, synthetic construct
GGKGKDFFR

SEQ ID NO: 49580 - protein, 9 aa, synthetic construct
GGKGKDFFV

SEQ ID NO: 49581 - protein, 9 aa, synthetic construct
GGKGKDFIN

SEQ ID NO: 49582 - protein, 9 aa, synthetic construct
GGKGKDFLE

SEQ ID NO: 49583 - protein, 9 aa, synthetic construct
GGKGKDHIL

SEQ ID NO: 49584 - protein, 9 aa, synthetic construct
GGKGKDIFL

SEQ ID NO: 49585 - protein, 9 aa, synthetic construct
GGKGKDILR

SEQ ID NO: 49586 - protein, 9 aa, synthetic construct
GGKGKDILT

SEQ ID NO: 49587 - protein, 9 aa, synthetic construct
GGKGKDKIA

SEQ ID NO: 49588 - protein, 9 aa, synthetic construct
GGKGKDTMT

SEQ ID NO: 49589 - protein, 9 aa, synthetic construct
GGKGKDTMY

SEQ ID NO: 49590 - protein, 9 aa, synthetic construct
GGKGKDTVN

SEQ ID NO: 49591 - protein, 9 aa, synthetic construct
GGKGNDEIA

SEQ ID NO: 49592 - protein, 9 aa, synthetic construct
GGKGNDALN

SEQ ID NO: 49593 - protein, 9 aa, synthetic construct
GGKGNDAMS

SEQ ID NO: 49594 - protein, 9 aa, synthetic construct
GGKGNDAVS

SEQ ID NO: 49595 - protein, 9 aa, synthetic construct
GGKGNDAYD

SEQ ID NO: 49596 - protein, 9 aa, synthetic construct
GGKGNDAYS

SEQ ID NO: 49597 - protein, 9 aa, synthetic construct
GGKGNDCLD

SEQ ID NO: 49598 - protein, 9 aa, synthetic construct
GGKGNDDFV

SEQ ID NO: 49599 - protein, 9 aa, synthetic construct
GGKGNDDLF

SEQ ID NO: 49600 - protein, 9 aa, synthetic construct
GGKGNDDLI

SEQ ID NO: 49601 - protein, 9 aa, synthetic construct
GGKGNDDLS

SEQ ID NO: 49602 - protein, 9 aa, synthetic construct
GGKGNDDLT

SEQ ID NO: 49603 - protein, 9 aa, synthetic construct
GGKGNDDMS

SEQ ID NO: 49604 - protein, 9 aa, synthetic construct
GGKGNDDYG

SEQ ID NO: 49605 - protein, 9 aa, synthetic construct
GGKGNDEIF

SEQ ID NO: 49606 - protein, 9 aa, synthetic construct
GGKGNDALA

SEQ ID NO: 49607 - protein, 9 aa, synthetic construct
GGKGNDEIR

SEQ ID NO: 49608 - protein, 9 aa, synthetic construct
GGKGNDEIT

SEQ ID NO: 49609 - protein, 9 aa, synthetic construct
GGKGNDEIV

SEQ ID NO: 49610 - protein, 9 aa, synthetic construct
GGKGNDELA

SEQ ID NO: 49611 - protein, 9 aa, synthetic construct
GGKGNDELQ

SEQ ID NO: 49612 - protein, 9 aa, synthetic construct
GGKGNDEVQ

SEQ ID NO: 49613 - protein, 9 aa, synthetic construct
GGKGNDEYA

SEQ ID NO: 49614 - protein, 9 aa, synthetic construct
GGKGNDFIN

SEQ ID NO: 49615 - protein, 9 aa, synthetic construct
GGKGNDFLG

SEQ ID NO: 49616 - protein, 9 aa, synthetic construct
GGKGNDFLM

SEQ ID NO: 49617 - protein, 9 aa, synthetic construct
GGKGNDFLQ

SEQ ID NO: 49618 - protein, 9 aa, synthetic construct
GGKGNDFYD

SEQ ID NO: 49619 - protein, 9 aa, synthetic construct
GGKGNDFYV

SEQ ID NO: 49620 - protein, 9 aa, synthetic construct
GGKGNDALK

SEQ ID NO: 49621 - protein, 9 aa, synthetic construct
GGKGNDAIR

SEQ ID NO: 49622 - protein, 9 aa, synthetic construct
GGKGKDTVV

SEQ ID NO: 49623 - protein, 9 aa, synthetic construct
GGKGLDALD

SEQ ID NO: 49624 - protein, 9 aa, synthetic construct
GGKGKDTYV

SEQ ID NO: 49625 - protein, 9 aa, synthetic construct
GGKGKDVFG

SEQ ID NO: 49626 - protein, 9 aa, synthetic construct
GGKGKDVFK

SEQ ID NO: 49627 - protein, 9 aa, synthetic construct
GGKGKDVIA

SEQ ID NO: 49628 - protein, 9 aa, synthetic construct
GGKGKDVLD

SEQ ID NO: 49629 - protein, 9 aa, synthetic construct
GGKGKDVLK

SEQ ID NO: 49630 - protein, 9 aa, synthetic construct
GGKGKDVLT

SEQ ID NO: 49631 - protein, 9 aa, synthetic construct
GGKGKDVLV

SEQ ID NO: 49632 - protein, 9 aa, synthetic construct
GGKGKDVVT

SEQ ID NO: 49633 - protein, 9 aa, synthetic construct
GGKGKDWLN

SEQ ID NO: 49634 - protein, 9 aa, synthetic construct
GGKGKDWLS

SEQ ID NO: 49635 - protein, 9 aa, synthetic construct
GGKGKDYLD

SEQ ID NO: 49636 - protein, 9 aa, synthetic construct
GGKGKDYLN

SEQ ID NO: 49637 - protein, 9 aa, synthetic construct
GGKGLDDVH

SEQ ID NO: 49638 - protein, 9 aa, synthetic construct
GGKGMDLMS

SEQ ID NO: 49639 - protein, 9 aa, synthetic construct
GGKGLDFMN

SEQ ID NO: 49640 - protein, 9 aa, synthetic construct
GGKGLDFMR

SEQ ID NO: 49641 - protein, 9 aa, synthetic construct
GGKGLDMLK

SEQ ID NO: 49642 - protein, 9 aa, synthetic construct
GGKGLDRLE

SEQ ID NO: 49643 - protein, 9 aa, synthetic construct
GGKGLDRLF

SEQ ID NO: 49644 - protein, 9 aa, synthetic construct
GGKGLDRLN

SEQ ID NO: 49645 - protein, 9 aa, synthetic construct
GGKGLDSIE

SEQ ID NO: 49646 - protein, 9 aa, synthetic construct
GGKGLDVIE

SEQ ID NO: 49647 - protein, 9 aa, synthetic construct
GGKGLDVVI

SEQ ID NO: 49648 - protein, 9 aa, synthetic construct
GGKGLDVVS

SEQ ID NO: 49649 - protein, 9 aa, synthetic construct
GGKGLDYAD

SEQ ID NO: 49650 - protein, 9 aa, synthetic construct
GGKGMDELR

SEQ ID NO: 49651 - protein, 9 aa, synthetic construct
GGKGMDFIE

SEQ ID NO: 49652 - protein, 9 aa, synthetic construct
GGLGDDQMR

SEQ ID NO: 49653 - protein, 9 aa, synthetic construct
GGLGDDQMW

SEQ ID NO: 49654 - protein, 9 aa, synthetic construct
GGLGTDAMY

SEQ ID NO: 49655 - protein, 9 aa, synthetic construct
GGLGNDWLR

SEQ ID NO: 49656 - protein, 9 aa, synthetic construct
GGLGNDTFM

SEQ ID NO: 49657 - protein, 9 aa, synthetic construct
GGLGNDTFS

SEQ ID NO: 49658 - protein, 9 aa, synthetic construct
GGLGNDTIK

SEQ ID NO: 49659 - protein, 9 aa, synthetic construct
GGLGNDTIQ

SEQ ID NO: 49660 - protein, 9 aa, synthetic construct
GGLGNDTVA

SEQ ID NO: 49661 - protein, 9 aa, synthetic construct
GGLGNDTVG

SEQ ID NO: 49662 - protein, 9 aa, synthetic construct
GGLGNDTVK

SEQ ID NO: 49663 - protein, 9 aa, synthetic construct
GGLGNDTVV

SEQ ID NO: 49664 - protein, 9 aa, synthetic construct
GGLGNDTYN

SEQ ID NO: 49665 - protein, 9 aa, synthetic construct
GGLGNDTYQ

SEQ ID NO: 49666 - protein, 9 aa, synthetic construct
GGLGNDVFD

SEQ ID NO: 49667 - protein, 9 aa, synthetic construct
GGLGNDVFQ

SEQ ID NO: 49668 - protein, 9 aa, synthetic construct
GGLGNDVIT

SEQ ID NO: 49669 - protein, 9 aa, synthetic construct
GGLGNDVMA

SEQ ID NO: 49670 - protein, 9 aa, synthetic construct
GGLGNDVMF

SEQ ID NO: 49671 - protein, 9 aa, synthetic construct
GGLGNDVMV

SEQ ID NO: 49672 - protein, 9 aa, synthetic construct
GGLGNDVVD

SEQ ID NO: 49673 - protein, 9 aa, synthetic construct
GGLGNDVVM

SEQ ID NO: 49674 - protein, 9 aa, synthetic construct
GGLGNDVVY

SEQ ID NO: 49675 - protein, 9 aa, synthetic construct
GGLGNDVYD

SEQ ID NO: 49676 - protein, 9 aa, synthetic construct
GGLGNDVYE

SEQ ID NO: 49677 - protein, 9 aa, synthetic construct
GGLGNDVYH

SEQ ID NO: 49678 - protein, 9 aa, synthetic construct
GGLGNDVYM

SEQ ID NO: 49679 - protein, 9 aa, synthetic construct
GGLGNDWFN

SEQ ID NO: 49680 - protein, 9 aa, synthetic construct
GGLGNDWFV

SEQ ID NO: 49681 - protein, 9 aa, synthetic construct
GGLGNDWIE

SEQ ID NO: 49682 - protein, 9 aa, synthetic construct
GGLGNDWLA

SEQ ID NO: 49683 - protein, 9 aa, synthetic construct
GGLGNDWLE

SEQ ID NO: 49684 - protein, 9 aa, synthetic construct
GGLGNDWLF

SEQ ID NO: 49685 - protein, 9 aa, synthetic construct
GGLGNDTFL

SEQ ID NO: 49686 - protein, 9 aa, synthetic construct
GGLGNDTFA

SEQ ID NO: 49687 - protein, 9 aa, synthetic construct
GGLGNDTAE

SEQ ID NO: 49688 - protein, 9 aa, synthetic construct
GGLGNDRYI

SEQ ID NO: 49689 - protein, 9 aa, synthetic construct
GGLGNDRII

SEQ ID NO: 49690 - protein, 9 aa, synthetic construct
GGLGNDRIL

SEQ ID NO: 49691 - protein, 9 aa, synthetic construct
GGLGNDRLG

SEQ ID NO: 49692 - protein, 9 aa, synthetic construct
GGLGNDRLK

SEQ ID NO: 49693 - protein, 9 aa, synthetic construct
GGLGNDRLW

SEQ ID NO: 49694 - protein, 9 aa, synthetic construct
GGLGNDRME

SEQ ID NO: 49695 - protein, 9 aa, synthetic construct
GGLGNDRMF

SEQ ID NO: 49696 - protein, 9 aa, synthetic construct
GGLGNDRMI

SEQ ID NO: 49697 - protein, 9 aa, synthetic construct
GGLGNDRML

SEQ ID NO: 49698 - protein, 9 aa, synthetic construct
GGLGNDRVF

SEQ ID NO: 49699 - protein, 9 aa, synthetic construct
GGLGNDRVI

SEQ ID NO: 49700 - protein, 9 aa, synthetic construct
GGLGNDRVN

SEQ ID NO: 49701 - protein, 9 aa, synthetic construct
GGLGNDRYF

SEQ ID NO: 49702 - protein, 9 aa, synthetic construct
GGLGNDRYM

SEQ ID NO: 49703 - protein, 9 aa, synthetic construct
GGLGNDSYS

SEQ ID NO: 49704 - protein, 9 aa, synthetic construct
GGLGNDRYT

SEQ ID NO: 49705 - protein, 9 aa, synthetic construct
GGLGNDSFK

SEQ ID NO: 49706 - protein, 9 aa, synthetic construct
GGLGNDSFL

SEQ ID NO: 49707 - protein, 9 aa, synthetic construct
GGLGNDSFS

SEQ ID NO: 49708 - protein, 9 aa, synthetic construct
GGLGNDSFY

SEQ ID NO: 49709 - protein, 9 aa, synthetic construct
GGLGNDSIQ

SEQ ID NO: 49710 - protein, 9 aa, synthetic construct
GGLGNDSLR

SEQ ID NO: 49711 - protein, 9 aa, synthetic construct
GGLGNDSMS

SEQ ID NO: 49712 - protein, 9 aa, synthetic construct
GGLGNDSVA

SEQ ID NO: 49713 - protein, 9 aa, synthetic construct
GGLGNDSVF

SEQ ID NO: 49714 - protein, 9 aa, synthetic construct
GGLGNDSVH

SEQ ID NO: 49715 - protein, 9 aa, synthetic construct
GGLGNDSVT

SEQ ID NO: 49716 - protein, 9 aa, synthetic construct
GGLGNDSYA

SEQ ID NO: 49717 - protein, 9 aa, synthetic construct
GGLGNDWLN

SEQ ID NO: 49718 - protein, 9 aa, synthetic construct
GGLGNDWLY

SEQ ID NO: 49719 - protein, 9 aa, synthetic construct
GGLGQDTFA

SEQ ID NO: 49720 - protein, 9 aa, synthetic construct
GGLGNDWVN

SEQ ID NO: 49721 - protein, 9 aa, synthetic construct
GGLGQDEYR

SEQ ID NO: 49722 - protein, 9 aa, synthetic construct
GGLGQDFFY

SEQ ID NO: 49723 - protein, 9 aa, synthetic construct
GGLGQDFLF

SEQ ID NO: 49724 - protein, 9 aa, synthetic construct
GGLGQDFLY

SEQ ID NO: 49725 - protein, 9 aa, synthetic construct
GGLGQDHLI

SEQ ID NO: 49726 - protein, 9 aa, synthetic construct
GGLGQDHLL

SEQ ID NO: 49727 - protein, 9 aa, synthetic construct
GGLGQDIFV

SEQ ID NO: 49728 - protein, 9 aa, synthetic construct
GGLGQDILD

SEQ ID NO: 49729 - protein, 9 aa, synthetic construct
GGLGQDILN

SEQ ID NO: 49730 - protein, 9 aa, synthetic construct
GGLGQDKLL

SEQ ID NO: 49731 - protein, 9 aa, synthetic construct
GGLGQDLLA

SEQ ID NO: 49732 - protein, 9 aa, synthetic construct
GGLGQDLLH

SEQ ID NO: 49733 - protein, 9 aa, synthetic construct
GGLGQDLLK

SEQ ID NO: 49734 - protein, 9 aa, synthetic construct
GGLGQDMLI

SEQ ID NO: 49735 - protein, 9 aa, synthetic construct
GGLGQDNFV

SEQ ID NO: 49736 - protein, 9 aa, synthetic construct
GGLGQDNIS

SEQ ID NO: 49737 - protein, 9 aa, synthetic construct
GGLGQDNLT

SEQ ID NO: 49738 - protein, 9 aa, synthetic construct
GGLGQDQLC

SEQ ID NO: 49739 - protein, 9 aa, synthetic construct
GGLGQDQLT

SEQ ID NO: 49740 - protein, 9 aa, synthetic construct
GGLGQDQMS

SEQ ID NO: 49741 - protein, 9 aa, synthetic construct
GGLGQDRFL

SEQ ID NO: 49742 - protein, 9 aa, synthetic construct
GGLGQDRLI

SEQ ID NO: 49743 - protein, 9 aa, synthetic construct
GGLGQDRLM

SEQ ID NO: 49744 - protein, 9 aa, synthetic construct
GGLGQDRVF

SEQ ID NO: 49745 - protein, 9 aa, synthetic construct
GGLGQDRVI

SEQ ID NO: 49746 - protein, 9 aa, synthetic construct
GGLGQDSLE

SEQ ID NO: 49747 - protein, 9 aa, synthetic construct
GGLGQDSLH

SEQ ID NO: 49748 - protein, 9 aa, synthetic construct
GGLGQDSLL

SEQ ID NO: 49749 - protein, 9 aa, synthetic construct
GGLGQDSLV

SEQ ID NO: 49750 - protein, 9 aa, synthetic construct
GGLGQDELL

SEQ ID NO: 49751 - protein, 9 aa, synthetic construct
GGLGQDDMI

SEQ ID NO: 49752 - protein, 9 aa, synthetic construct
GGLGQDALS

SEQ ID NO: 49753 - protein, 9 aa, synthetic construct
GGLGPDIMD

SEQ ID NO: 49754 - protein, 9 aa, synthetic construct
GGLGNDWVV

SEQ ID NO: 49755 - protein, 9 aa, synthetic construct
GGLGNDYFD

SEQ ID NO: 49756 - protein, 9 aa, synthetic construct
GGLGNDYIE

SEQ ID NO: 49757 - protein, 9 aa, synthetic construct
GGLGNDYIN

SEQ ID NO: 49758 - protein, 9 aa, synthetic construct
GGLGNDYIQ

SEQ ID NO: 49759 - protein, 9 aa, synthetic construct
GGLGNDYIV

SEQ ID NO: 49760 - protein, 9 aa, synthetic construct
GGLGNDYLG

SEQ ID NO: 49761 - protein, 9 aa, synthetic construct
GGLGNDYLK

SEQ ID NO: 49762 - protein, 9 aa, synthetic construct
GGLGNDYMA

SEQ ID NO: 49763 - protein, 9 aa, synthetic construct
GGLGNDYME

SEQ ID NO: 49764 - protein, 9 aa, synthetic construct
GGLGNDYMY

SEQ ID NO: 49765 - protein, 9 aa, synthetic construct
GGLGNDYVN

SEQ ID NO: 49766 - protein, 9 aa, synthetic construct
GGLGPDALL

SEQ ID NO: 49767 - protein, 9 aa, synthetic construct
GGLGPDLID

SEQ ID NO: 49768 - protein, 9 aa, synthetic construct
GGLGPDWIE

SEQ ID NO: 49769 - protein, 9 aa, synthetic construct
GGLGPDNLF

SEQ ID NO: 49770 - protein, 9 aa, synthetic construct
GGLGPDQII

SEQ ID NO: 49771 - protein, 9 aa, synthetic construct
GGLGPDRFV

SEQ ID NO: 49772 - protein, 9 aa, synthetic construct
GGLGPDRMR

SEQ ID NO: 49773 - protein, 9 aa, synthetic construct
GGLGPDSLG

SEQ ID NO: 49774 - protein, 9 aa, synthetic construct
GGLGPDTFI

SEQ ID NO: 49775 - protein, 9 aa, synthetic construct
GGLGPDTIL

SEQ ID NO: 49776 - protein, 9 aa, synthetic construct
GGLGPDTLA

SEQ ID NO: 49777 - protein, 9 aa, synthetic construct
GGLGPDTLM

SEQ ID NO: 49778 - protein, 9 aa, synthetic construct
GGLGPDTLT

SEQ ID NO: 49779 - protein, 9 aa, synthetic construct
GGLGPDTLV

SEQ ID NO: 49780 - protein, 9 aa, synthetic construct
GGLGPDTMF

SEQ ID NO: 49781 - protein, 9 aa, synthetic construct
GGLGPDVFI

SEQ ID NO: 49782 - protein, 9 aa, synthetic construct
GGLGNDRIG

SEQ ID NO: 49783 - protein, 9 aa, synthetic construct
GGLGNDRFY

SEQ ID NO: 49784 - protein, 9 aa, synthetic construct
GGLGNDRFV

SEQ ID NO: 49785 - protein, 9 aa, synthetic construct
GGLGNDRFD

SEQ ID NO: 49786 - protein, 9 aa, synthetic construct
GGLGNDFFI

SEQ ID NO: 49787 - protein, 9 aa, synthetic construct
GGLGNDFIH

SEQ ID NO: 49788 - protein, 9 aa, synthetic construct
GGLGNDFIS

SEQ ID NO: 49789 - protein, 9 aa, synthetic construct
GGLGNDFLI

SEQ ID NO: 49790 - protein, 9 aa, synthetic construct
GGLGNDFLL

SEQ ID NO: 49791 - protein, 9 aa, synthetic construct
GGLGNDFLR

SEQ ID NO: 49792 - protein, 9 aa, synthetic construct
GGLGNDFMA

SEQ ID NO: 49793 - protein, 9 aa, synthetic construct
GGLGNDFML

SEQ ID NO: 49794 - protein, 9 aa, synthetic construct
GGLGNDFVI

SEQ ID NO: 49795 - protein, 9 aa, synthetic construct
GGLGNDFVL

SEQ ID NO: 49796 - protein, 9 aa, synthetic construct
GGLGNDFYI

SEQ ID NO: 49797 - protein, 9 aa, synthetic construct
GGLGNDFYS

SEQ ID NO: 49798 - protein, 9 aa, synthetic construct
GGLGNDFYV

SEQ ID NO: 49799 - protein, 9 aa, synthetic construct
GGLGNDGLF

SEQ ID NO: 49800 - protein, 9 aa, synthetic construct
GGLGNDGLL

SEQ ID NO: 49801 - protein, 9 aa, synthetic construct
GGLGNDGLW

SEQ ID NO: 49802 - protein, 9 aa, synthetic construct
GGLGNDHIM

SEQ ID NO: 49803 - protein, 9 aa, synthetic construct
GGLGNDHLD

SEQ ID NO: 49804 - protein, 9 aa, synthetic construct
GGLGNDHLG

SEQ ID NO: 49805 - protein, 9 aa, synthetic construct
GGLGNDHLT

SEQ ID NO: 49806 - protein, 9 aa, synthetic construct
GGLGNDHLV

SEQ ID NO: 49807 - protein, 9 aa, synthetic construct
GGLGNDHYI

SEQ ID NO: 49808 - protein, 9 aa, synthetic construct
GGLGNDHYL

SEQ ID NO: 49809 - protein, 9 aa, synthetic construct
GGLGNDHYQ

SEQ ID NO: 49810 - protein, 9 aa, synthetic construct
GGLGNDHYY

SEQ ID NO: 49811 - protein, 9 aa, synthetic construct
GGLGNDIAA

SEQ ID NO: 49812 - protein, 9 aa, synthetic construct
GGLGNDIAE

SEQ ID NO: 49813 - protein, 9 aa, synthetic construct
GGLGNDIAV

SEQ ID NO: 49814 - protein, 9 aa, synthetic construct
GGLGNDIFA

SEQ ID NO: 49815 - protein, 9 aa, synthetic construct
GGLGNDFAS

SEQ ID NO: 49816 - protein, 9 aa, synthetic construct
GGLGNDEMQ

SEQ ID NO: 49817 - protein, 9 aa, synthetic construct
GGLGNDELV

SEQ ID NO: 49818 - protein, 9 aa, synthetic construct
GGLGNDDIK

SEQ ID NO: 49819 - protein, 9 aa, synthetic construct
GGLGNDAIV

SEQ ID NO: 49820 - protein, 9 aa, synthetic construct
GGLGNDALL

SEQ ID NO: 49821 - protein, 9 aa, synthetic construct
GGLGNDALQ

SEQ ID NO: 49822 - protein, 9 aa, synthetic construct
GGLGNDAMR

SEQ ID NO: 49823 - protein, 9 aa, synthetic construct
GGLGNDAVH

SEQ ID NO: 49824 - protein, 9 aa, synthetic construct
GGLGNDAVL

SEQ ID NO: 49825 - protein, 9 aa, synthetic construct
GGLGNDAYI

SEQ ID NO: 49826 - protein, 9 aa, synthetic construct
GGLGNDAYY

SEQ ID NO: 49827 - protein, 9 aa, synthetic construct
GGLGNDDIA

SEQ ID NO: 49828 - protein, 9 aa, synthetic construct
GGLGNDDID

SEQ ID NO: 49829 - protein, 9 aa, synthetic construct
GGLGNDDIE

SEQ ID NO: 49830 - protein, 9 aa, synthetic construct
GGLGNDDIF

SEQ ID NO: 49831 - protein, 9 aa, synthetic construct
GGLGNDDIH

SEQ ID NO: 49832 - protein, 9 aa, synthetic construct
GGLGNDDIN

SEQ ID NO: 49833 - protein, 9 aa, synthetic construct
GGLGNDELL

SEQ ID NO: 49834 - protein, 9 aa, synthetic construct
GGLGNDDLF

SEQ ID NO: 49835 - protein, 9 aa, synthetic construct
GGLGNDDLI

SEQ ID NO: 49836 - protein, 9 aa, synthetic construct
GGLGNDDLK

SEQ ID NO: 49837 - protein, 9 aa, synthetic construct
GGLGNDDLL

SEQ ID NO: 49838 - protein, 9 aa, synthetic construct
GGLGNDDLW

SEQ ID NO: 49839 - protein, 9 aa, synthetic construct
GGLGNDDMH

SEQ ID NO: 49840 - protein, 9 aa, synthetic construct
GGLGNDDMN

SEQ ID NO: 49841 - protein, 9 aa, synthetic construct
GGLGNDEAH

SEQ ID NO: 49842 - protein, 9 aa, synthetic construct
GGLGNDEFH

SEQ ID NO: 49843 - protein, 9 aa, synthetic construct
GGLGNDEFL

SEQ ID NO: 49844 - protein, 9 aa, synthetic construct
GGLGNDEID

SEQ ID NO: 49845 - protein, 9 aa, synthetic construct
GGLGNDEIH

SEQ ID NO: 49846 - protein, 9 aa, synthetic construct
GGLGNDEIS

SEQ ID NO: 49847 - protein, 9 aa, synthetic construct
GGLGNDIFQ

SEQ ID NO: 49848 - protein, 9 aa, synthetic construct
GGLGNDIFR

SEQ ID NO: 49849 - protein, 9 aa, synthetic construct
GGLGNDIIA

SEQ ID NO: 49850 - protein, 9 aa, synthetic construct
GGLGNDNYI

SEQ ID NO: 49851 - protein, 9 aa, synthetic construct
GGLGNDMLK

SEQ ID NO: 49852 - protein, 9 aa, synthetic construct
GGLGNDMMH

SEQ ID NO: 49853 - protein, 9 aa, synthetic construct
GGLGNDMMI

SEQ ID NO: 49854 - protein, 9 aa, synthetic construct
GGLGNDMVF

SEQ ID NO: 49855 - protein, 9 aa, synthetic construct
GGLGNDMVK

SEQ ID NO: 49856 - protein, 9 aa, synthetic construct
GGLGNDMVN

SEQ ID NO: 49857 - protein, 9 aa, synthetic construct
GGLGNDNFV

SEQ ID NO: 49858 - protein, 9 aa, synthetic construct
GGLGNDNID

SEQ ID NO: 49859 - protein, 9 aa, synthetic construct
GGLGNDNIN

SEQ ID NO: 49860 - protein, 9 aa, synthetic construct
GGLGNDNIQ

SEQ ID NO: 49861 - protein, 9 aa, synthetic construct
GGLGNDNLN

SEQ ID NO: 49862 - protein, 9 aa, synthetic construct
GGLGNDNLR

SEQ ID NO: 49863 - protein, 9 aa, synthetic construct
GGLGNDNVS

SEQ ID NO: 49864 - protein, 9 aa, synthetic construct
GGLGNDNYR

SEQ ID NO: 49865 - protein, 9 aa, synthetic construct
GGLGNDLYY

SEQ ID NO: 49866 - protein, 9 aa, synthetic construct
GGLGNDQFT

SEQ ID NO: 49867 - protein, 9 aa, synthetic construct
GGLGNDQIG

SEQ ID NO: 49868 - protein, 9 aa, synthetic construct
GGLGNDQIW

SEQ ID NO: 49869 - protein, 9 aa, synthetic construct
GGLGNDQIY

SEQ ID NO: 49870 - protein, 9 aa, synthetic construct
GGLGNDQLA

SEQ ID NO: 49871 - protein, 9 aa, synthetic construct
GGLGNDQLK

SEQ ID NO: 49872 - protein, 9 aa, synthetic construct
GGLGNDQLV

SEQ ID NO: 49873 - protein, 9 aa, synthetic construct
GGLGNDQMS

SEQ ID NO: 49874 - protein, 9 aa, synthetic construct
GGLGNDQMT

SEQ ID NO: 49875 - protein, 9 aa, synthetic construct
GGLGNDQMV

SEQ ID NO: 49876 - protein, 9 aa, synthetic construct
GGLGNDQVL

SEQ ID NO: 49877 - protein, 9 aa, synthetic construct
GGLGNDQVR

SEQ ID NO: 49878 - protein, 9 aa, synthetic construct
GGLGNDQYR

SEQ ID NO: 49879 - protein, 9 aa, synthetic construct
GGLGNDMIK

SEQ ID NO: 49880 - protein, 9 aa, synthetic construct
GGLGNDLVS

SEQ ID NO: 49881 - protein, 9 aa, synthetic construct
GGLGNDIIG

SEQ ID NO: 49882 - protein, 9 aa, synthetic construct
GGLGNDKIR

SEQ ID NO: 49883 - protein, 9 aa, synthetic construct
GGLGNDIIL

SEQ ID NO: 49884 - protein, 9 aa, synthetic construct
GGLGNDIIM

SEQ ID NO: 49885 - protein, 9 aa, synthetic construct
GGLGNDIIQ

SEQ ID NO: 49886 - protein, 9 aa, synthetic construct
GGLGNDILW

SEQ ID NO: 49887 - protein, 9 aa, synthetic construct
GGLGNDIME

SEQ ID NO: 49888 - protein, 9 aa, synthetic construct
GGLGNDIVF

SEQ ID NO: 49889 - protein, 9 aa, synthetic construct
GGLGNDIVR

SEQ ID NO: 49890 - protein, 9 aa, synthetic construct
GGLGNDIVS

SEQ ID NO: 49891 - protein, 9 aa, synthetic construct
GGLGNDIYE

SEQ ID NO: 49892 - protein, 9 aa, synthetic construct
GGLGNDIYH

SEQ ID NO: 49893 - protein, 9 aa, synthetic construct
GGLGNDIYK

SEQ ID NO: 49894 - protein, 9 aa, synthetic construct
GGLGNDKIK

SEQ ID NO: 49895 - protein, 9 aa, synthetic construct
GGLGNDKIL

SEQ ID NO: 49896 - protein, 9 aa, synthetic construct
GGLGNDKLM

SEQ ID NO: 49897 - protein, 9 aa, synthetic construct
GGLGNDLVR

SEQ ID NO: 49898 - protein, 9 aa, synthetic construct
GGLGNDKMI

SEQ ID NO: 49899 - protein, 9 aa, synthetic construct
GGLGNDKMS

SEQ ID NO: 49900 - protein, 9 aa, synthetic construct
GGLGNDKMT

SEQ ID NO: 49901 - protein, 9 aa, synthetic construct
GGLGNDLAF

SEQ ID NO: 49902 - protein, 9 aa, synthetic construct
GGLGNDLAH

SEQ ID NO: 49903 - protein, 9 aa, synthetic construct
GGLGNDLAR

SEQ ID NO: 49904 - protein, 9 aa, synthetic construct
GGLGNDLAY

SEQ ID NO: 49905 - protein, 9 aa, synthetic construct
GGLGNDLIF

SEQ ID NO: 49906 - protein, 9 aa, synthetic construct
GGLGNDLIG

SEQ ID NO: 49907 - protein, 9 aa, synthetic construct
GGLGNDLLK

SEQ ID NO: 49908 - protein, 9 aa, synthetic construct
GGLGNDLMT

SEQ ID NO: 49909 - protein, 9 aa, synthetic construct
GGLGNDLMY

SEQ ID NO: 49910 - protein, 9 aa, synthetic construct
GGLGNDLVQ

SEQ ID NO: 49911 - protein, 9 aa, synthetic construct
GGLGQDSLW

SEQ ID NO: 49912 - protein, 9 aa, synthetic construct
GGLGQDTFT

SEQ ID NO: 49913 - protein, 9 aa, synthetic construct
GGLGDDQVF

SEQ ID NO: 49914 - protein, 9 aa, synthetic construct
GGLGSDQAN

SEQ ID NO: 49915 - protein, 9 aa, synthetic construct
GGLGSDLAR

SEQ ID NO: 49916 - protein, 9 aa, synthetic construct
GGLGSDLFL

SEQ ID NO: 49917 - protein, 9 aa, synthetic construct
GGLGSDLFV

SEQ ID NO: 49918 - protein, 9 aa, synthetic construct
GGLGSDLID

SEQ ID NO: 49919 - protein, 9 aa, synthetic construct
GGLGSDLIN

SEQ ID NO: 49920 - protein, 9 aa, synthetic construct
GGLGSDLLE

SEQ ID NO: 49921 - protein, 9 aa, synthetic construct
GGLGSDLLH

SEQ ID NO: 49922 - protein, 9 aa, synthetic construct
GGLGSDLLI

SEQ ID NO: 49923 - protein, 9 aa, synthetic construct
GGLGSDLLN

SEQ ID NO: 49924 - protein, 9 aa, synthetic construct
GGLGSDLLQ

SEQ ID NO: 49925 - protein, 9 aa, synthetic construct
GGLGSDLLR

SEQ ID NO: 49926 - protein, 9 aa, synthetic construct
GGLGSDLLV

SEQ ID NO: 49927 - protein, 9 aa, synthetic construct
GGLGSDLMF

SEQ ID NO: 49928 - protein, 9 aa, synthetic construct
GGLGSDLVA

SEQ ID NO: 49929 - protein, 9 aa, synthetic construct
GGLGSDLVN

SEQ ID NO: 49930 - protein, 9 aa, synthetic construct
GGLGSDLVS

SEQ ID NO: 49931 - protein, 9 aa, synthetic construct
GGLGSDLVY

SEQ ID NO: 49932 - protein, 9 aa, synthetic construct
GGLGSDMFQ

SEQ ID NO: 49933 - protein, 9 aa, synthetic construct
GGLGSDMLD

SEQ ID NO: 49934 - protein, 9 aa, synthetic construct
GGLGSDMLN

SEQ ID NO: 49935 - protein, 9 aa, synthetic construct
GGLGSDMLR

SEQ ID NO: 49936 - protein, 9 aa, synthetic construct
GGLGSDNIA

SEQ ID NO: 49937 - protein, 9 aa, synthetic construct
GGLGSDNIY

SEQ ID NO: 49938 - protein, 9 aa, synthetic construct
GGLGSDNLA

SEQ ID NO: 49939 - protein, 9 aa, synthetic construct
GGLGSDNLD

SEQ ID NO: 49940 - protein, 9 aa, synthetic construct
GGLGSDNLE

SEQ ID NO: 49941 - protein, 9 aa, synthetic construct
GGLGSDNLG

SEQ ID NO: 49942 - protein, 9 aa, synthetic construct
GGLGSDNLN

SEQ ID NO: 49943 - protein, 9 aa, synthetic construct
GGLGSDNLV

SEQ ID NO: 49944 - protein, 9 aa, synthetic construct
GGLGSDKLN

SEQ ID NO: 49945 - protein, 9 aa, synthetic construct
GGLGSDKLL

SEQ ID NO: 49946 - protein, 9 aa, synthetic construct
GGLGSDKLI

SEQ ID NO: 49947 - protein, 9 aa, synthetic construct
GGLGSDFLH

SEQ ID NO: 49948 - protein, 9 aa, synthetic construct
GGLGSDALS

SEQ ID NO: 49949 - protein, 9 aa, synthetic construct
GGLGSDDID

SEQ ID NO: 49950 - protein, 9 aa, synthetic construct
GGLGSDDIS

SEQ ID NO: 49951 - protein, 9 aa, synthetic construct
GGLGSDDLF

SEQ ID NO: 49952 - protein, 9 aa, synthetic construct
GGLGSDDLL

SEQ ID NO: 49953 - protein, 9 aa, synthetic construct
GGLGSDDLT

SEQ ID NO: 49954 - protein, 9 aa, synthetic construct
GGLGSDELA

SEQ ID NO: 49955 - protein, 9 aa, synthetic construct
GGLGSDELD

SEQ ID NO: 49956 - protein, 9 aa, synthetic construct
GGLGSDELF

SEQ ID NO: 49957 - protein, 9 aa, synthetic construct
GGLGSDELN

SEQ ID NO: 49958 - protein, 9 aa, synthetic construct
GGLGSDEMA

SEQ ID NO: 49959 - protein, 9 aa, synthetic construct
GGLGSDFAD

SEQ ID NO: 49960 - protein, 9 aa, synthetic construct
GGLGSDFLA

SEQ ID NO: 49961 - protein, 9 aa, synthetic construct
GGLGSDFVD

SEQ ID NO: 49962 - protein, 9 aa, synthetic construct
GGLGSDKLF

SEQ ID NO: 49963 - protein, 9 aa, synthetic construct
GGLGSDHIE

SEQ ID NO: 49964 - protein, 9 aa, synthetic construct
GGLGSDHIL

SEQ ID NO: 49965 - protein, 9 aa, synthetic construct
GGLGSDHLI

SEQ ID NO: 49966 - protein, 9 aa, synthetic construct
GGLGSDIAD

SEQ ID NO: 49967 - protein, 9 aa, synthetic construct
GGLGSDIFV

SEQ ID NO: 49968 - protein, 9 aa, synthetic construct
GGLGSDIIG

SEQ ID NO: 49969 - protein, 9 aa, synthetic construct
GGLGSDIIL

SEQ ID NO: 49970 - protein, 9 aa, synthetic construct
GGLGSDILY

SEQ ID NO: 49971 - protein, 9 aa, synthetic construct
GGLGSDIYL

SEQ ID NO: 49972 - protein, 9 aa, synthetic construct
GGLGSDIYM

SEQ ID NO: 49973 - protein, 9 aa, synthetic construct
GGLGSDIYQ

SEQ ID NO: 49974 - protein, 9 aa, synthetic construct
GGLGSDKIA

SEQ ID NO: 49975 - protein, 9 aa, synthetic construct
GGLGSDKLA

SEQ ID NO: 49976 - protein, 9 aa, synthetic construct
GGLGSDNME

SEQ ID NO: 49977 - protein, 9 aa, synthetic construct
GGLGSDQFH

SEQ ID NO: 49978 - protein, 9 aa, synthetic construct
GGLGQDTID

SEQ ID NO: 49979 - protein, 9 aa, synthetic construct
GGLGSDQFI

SEQ ID NO: 49980 - protein, 9 aa, synthetic construct
GGLGSDSYV

SEQ ID NO: 49981 - protein, 9 aa, synthetic construct
GGLGSDTAD

SEQ ID NO: 49982 - protein, 9 aa, synthetic construct
GGLGSDTAE

SEQ ID NO: 49983 - protein, 9 aa, synthetic construct
GGLGSDTAF

SEQ ID NO: 49984 - protein, 9 aa, synthetic construct
GGLGSDTAV

SEQ ID NO: 49985 - protein, 9 aa, synthetic construct
GGLGSDTFR

SEQ ID NO: 49986 - protein, 9 aa, synthetic construct
GGLGSDTIL

SEQ ID NO: 49987 - protein, 9 aa, synthetic construct
GGLGSDTIS

SEQ ID NO: 49988 - protein, 9 aa, synthetic construct
GGLGSDTMA

SEQ ID NO: 49989 - protein, 9 aa, synthetic construct
GGLGSDTMD

SEQ ID NO: 49990 - protein, 9 aa, synthetic construct
GGLGSDTMY

SEQ ID NO: 49991 - protein, 9 aa, synthetic construct
GGLGSDTVA

SEQ ID NO: 49992 - protein, 9 aa, synthetic construct
GGLGSDTYH

SEQ ID NO: 49993 - protein, 9 aa, synthetic construct
GGLGSDVFI

SEQ ID NO: 49994 - protein, 9 aa, synthetic construct
GGLGSDVID

SEQ ID NO: 49995 - protein, 9 aa, synthetic construct
GGLGSDVIS

SEQ ID NO: 49996 - protein, 9 aa, synthetic construct
GGLGSDVLH

SEQ ID NO: 49997 - protein, 9 aa, synthetic construct
GGLGSDVMK

SEQ ID NO: 49998 - protein, 9 aa, synthetic construct
GGLGSDVML

SEQ ID NO: 49999 - protein, 9 aa, synthetic construct
GGLGSDVMR

SEQ ID NO: 50000 - protein, 9 aa, synthetic construct
GGLGSDVMV

SEQ ID NO: 50001 - protein, 9 aa, synthetic construct
GGLGSDVYK

SEQ ID NO: 50002 - protein, 9 aa, synthetic construct
GGLGSDWFV

SEQ ID NO: 50003 - protein, 9 aa, synthetic construct
GGLGSDWIT

SEQ ID NO: 50004 - protein, 9 aa, synthetic construct
GGLGSDWLS

SEQ ID NO: 50005 - protein, 9 aa, synthetic construct
GGLGSDYIS

SEQ ID NO: 50006 - protein, 9 aa, synthetic construct
GGLGSDYLD

SEQ ID NO: 50007 - protein, 9 aa, synthetic construct
GGLGTDAAV

SEQ ID NO: 50008 - protein, 9 aa, synthetic construct
GGLGTDALY

SEQ ID NO: 50009 - protein, 9 aa, synthetic construct
GGLGSDSYI

SEQ ID NO: 50010 - protein, 9 aa, synthetic construct
GGLGSDSVG

SEQ ID NO: 50011 - protein, 9 aa, synthetic construct
GGLGSDSML

SEQ ID NO: 50012 - protein, 9 aa, synthetic construct
GGLGSDRLL

SEQ ID NO: 50013 - protein, 9 aa, synthetic construct
GGLGSDQFL

SEQ ID NO: 50014 - protein, 9 aa, synthetic construct
GGLGSDQFY

SEQ ID NO: 50015 - protein, 9 aa, synthetic construct
GGLGSDQIR

SEQ ID NO: 50016 - protein, 9 aa, synthetic construct
GGLGSDQLE

SEQ ID NO: 50017 - protein, 9 aa, synthetic construct
GGLGSDQLN

SEQ ID NO: 50018 - protein, 9 aa, synthetic construct
GGLGSDQLQ

SEQ ID NO: 50019 - protein, 9 aa, synthetic construct
GGLGSDQLT

SEQ ID NO: 50020 - protein, 9 aa, synthetic construct
GGLGSDQVW

SEQ ID NO: 50021 - protein, 9 aa, synthetic construct
GGLGSDRAS

SEQ ID NO: 50022 - protein, 9 aa, synthetic construct
GGLGSDRIF

SEQ ID NO: 50023 - protein, 9 aa, synthetic construct
GGLGSDRIN

SEQ ID NO: 50024 - protein, 9 aa, synthetic construct
GGLGSDRIS

SEQ ID NO: 50025 - protein, 9 aa, synthetic construct
GGLGSDRLH

SEQ ID NO: 50026 - protein, 9 aa, synthetic construct
GGLGSDRLN

SEQ ID NO: 50027 - protein, 9 aa, synthetic construct
GGLGSDSME

SEQ ID NO: 50028 - protein, 9 aa, synthetic construct
GGLGSDRLW

SEQ ID NO: 50029 - protein, 9 aa, synthetic construct
GGLGSDRME

SEQ ID NO: 50030 - protein, 9 aa, synthetic construct
GGLGSDSFD

SEQ ID NO: 50031 - protein, 9 aa, synthetic construct
GGLGSDSFY

SEQ ID NO: 50032 - protein, 9 aa, synthetic construct
GGLGSDSIF

SEQ ID NO: 50033 - protein, 9 aa, synthetic construct
GGLGSDSII

SEQ ID NO: 50034 - protein, 9 aa, synthetic construct
GGLGSDSIN

SEQ ID NO: 50035 - protein, 9 aa, synthetic construct
GGLGSDSIS

SEQ ID NO: 50036 - protein, 9 aa, synthetic construct
GGLGSDSLA

SEQ ID NO: 50037 - protein, 9 aa, synthetic construct
GGLGSDSLE

SEQ ID NO: 50038 - protein, 9 aa, synthetic construct
GGLGSDSLF

SEQ ID NO: 50039 - protein, 9 aa, synthetic construct
GGLGSDSLG

SEQ ID NO: 50040 - protein, 9 aa, synthetic construct
GGLGSDSLR

SEQ ID NO: 50041 - protein, 9 aa, synthetic construct
GGLGSDALR

SEQ ID NO: 50042 - protein, 9 aa, synthetic construct
GGLGSDALD

SEQ ID NO: 50043 - protein, 9 aa, synthetic construct
GGLGSDAIK

SEQ ID NO: 50044 - protein, 9 aa, synthetic construct
GGLGRDYVT

SEQ ID NO: 50045 - protein, 9 aa, synthetic construct
GGLGRDELV

SEQ ID NO: 50046 - protein, 9 aa, synthetic construct
GGLGRDELW

SEQ ID NO: 50047 - protein, 9 aa, synthetic construct
GGLGRDFLY

SEQ ID NO: 50048 - protein, 9 aa, synthetic construct
GGLGRDFVA

SEQ ID NO: 50049 - protein, 9 aa, synthetic construct
GGLGRDGFI

SEQ ID NO: 50050 - protein, 9 aa, synthetic construct
GGLGRDHIY

SEQ ID NO: 50051 - protein, 9 aa, synthetic construct
GGLGRDHLF

SEQ ID NO: 50052 - protein, 9 aa, synthetic construct
GGLGRDHLN

SEQ ID NO: 50053 - protein, 9 aa, synthetic construct
GGLGRDIIS

SEQ ID NO: 50054 - protein, 9 aa, synthetic construct
GGLGRDILA

SEQ ID NO: 50055 - protein, 9 aa, synthetic construct
GGLGRDILD

SEQ ID NO: 50056 - protein, 9 aa, synthetic construct
GGLGRDILF

SEQ ID NO: 50057 - protein, 9 aa, synthetic construct
GGLGRDILI

SEQ ID NO: 50058 - protein, 9 aa, synthetic construct
GGLGRDILV

SEQ ID NO: 50059 - protein, 9 aa, synthetic construct
GGLGRDIMT

SEQ ID NO: 50060 - protein, 9 aa, synthetic construct
GGLGRDKIA

SEQ ID NO: 50061 - protein, 9 aa, synthetic construct
GGLGRDKIR

SEQ ID NO: 50062 - protein, 9 aa, synthetic construct
GGLGRDKLH

SEQ ID NO: 50063 - protein, 9 aa, synthetic construct
GGLGRDKLI

SEQ ID NO: 50064 - protein, 9 aa, synthetic construct
GGLGRDKLL

SEQ ID NO: 50065 - protein, 9 aa, synthetic construct
GGLGRDKLM

SEQ ID NO: 50066 - protein, 9 aa, synthetic construct
GGLGRDKLY

SEQ ID NO: 50067 - protein, 9 aa, synthetic construct
GGLGRDKVN

SEQ ID NO: 50068 - protein, 9 aa, synthetic construct
GGLGRDLAS

SEQ ID NO: 50069 - protein, 9 aa, synthetic construct
GGLGRDLAY

SEQ ID NO: 50070 - protein, 9 aa, synthetic construct
GGLGRDLFC

SEQ ID NO: 50071 - protein, 9 aa, synthetic construct
GGLGRDLFW

SEQ ID NO: 50072 - protein, 9 aa, synthetic construct
GGLGRDLID

SEQ ID NO: 50073 - protein, 9 aa, synthetic construct
GGLGRDLIK

SEQ ID NO: 50074 - protein, 9 aa, synthetic construct
GGLGRDELT

SEQ ID NO: 50075 - protein, 9 aa, synthetic construct
GGLGRDELH

SEQ ID NO: 50076 - protein, 9 aa, synthetic construct
GGLGRDEIK

SEQ ID NO: 50077 - protein, 9 aa, synthetic construct
GGLGQDVVL

SEQ ID NO: 50078 - protein, 9 aa, synthetic construct
GGLGQDTIL

SEQ ID NO: 50079 - protein, 9 aa, synthetic construct
GGLGQDTIQ

SEQ ID NO: 50080 - protein, 9 aa, synthetic construct
GGLGQDTLD

SEQ ID NO: 50081 - protein, 9 aa, synthetic construct
GGLGQDTLW

SEQ ID NO: 50082 - protein, 9 aa, synthetic construct
GGLGQDTMD

SEQ ID NO: 50083 - protein, 9 aa, synthetic construct
GGLGQDTVE

SEQ ID NO: 50084 - protein, 9 aa, synthetic construct
GGLGQDTVR

SEQ ID NO: 50085 - protein, 9 aa, synthetic construct
GGLGQDVFG

SEQ ID NO: 50086 - protein, 9 aa, synthetic construct
GGLGQDVID

SEQ ID NO: 50087 - protein, 9 aa, synthetic construct
GGLGQDVLE

SEQ ID NO: 50088 - protein, 9 aa, synthetic construct
GGLGQDVLH

SEQ ID NO: 50089 - protein, 9 aa, synthetic construct
GGLGQDVLR

SEQ ID NO: 50090 - protein, 9 aa, synthetic construct
GGLGQDVLS

SEQ ID NO: 50091 - protein, 9 aa, synthetic construct
GGLGQDWIG

SEQ ID NO: 50092 - protein, 9 aa, synthetic construct
GGLGRDDLT

SEQ ID NO: 50093 - protein, 9 aa, synthetic construct
GGLGQDWLT

SEQ ID NO: 50094 - protein, 9 aa, synthetic construct
GGLGQDYLD

SEQ ID NO: 50095 - protein, 9 aa, synthetic construct
GGLGQDYLS

SEQ ID NO: 50096 - protein, 9 aa, synthetic construct
GGLGRDAFR

SEQ ID NO: 50097 - protein, 9 aa, synthetic construct
GGLGRDAFV

SEQ ID NO: 50098 - protein, 9 aa, synthetic construct
GGLGRDALR

SEQ ID NO: 50099 - protein, 9 aa, synthetic construct
GGLGRDAME

SEQ ID NO: 50100 - protein, 9 aa, synthetic construct
GGLGRDAVS

SEQ ID NO: 50101 - protein, 9 aa, synthetic construct
GGLGRDAVT

SEQ ID NO: 50102 - protein, 9 aa, synthetic construct
GGLGRDCLT

SEQ ID NO: 50103 - protein, 9 aa, synthetic construct
GGLGRDDIH

SEQ ID NO: 50104 - protein, 9 aa, synthetic construct
GGLGRDDLI

SEQ ID NO: 50105 - protein, 9 aa, synthetic construct
GGLGRDDLR

SEQ ID NO: 50106 - protein, 9 aa, synthetic construct
GGLGRDLIV

SEQ ID NO: 50107 - protein, 9 aa, synthetic construct
GGLGRDLIW

SEQ ID NO: 50108 - protein, 9 aa, synthetic construct
GGLGRDLLD

SEQ ID NO: 50109 - protein, 9 aa, synthetic construct
GGLGRDTVV

SEQ ID NO: 50110 - protein, 9 aa, synthetic construct
GGLGRDTIL

SEQ ID NO: 50111 - protein, 9 aa, synthetic construct
GGLGRDTIN

SEQ ID NO: 50112 - protein, 9 aa, synthetic construct
GGLGRDTIT

SEQ ID NO: 50113 - protein, 9 aa, synthetic construct
GGLGRDTIY

SEQ ID NO: 50114 - protein, 9 aa, synthetic construct
GGLGRDTLK

SEQ ID NO: 50115 - protein, 9 aa, synthetic construct
GGLGRDTLQ

SEQ ID NO: 50116 - protein, 9 aa, synthetic construct
GGLGRDTLW

SEQ ID NO: 50117 - protein, 9 aa, synthetic construct
GGLGRDTLY

SEQ ID NO: 50118 - protein, 9 aa, synthetic construct
GGLGRDTMD

SEQ ID NO: 50119 - protein, 9 aa, synthetic construct
GGLGRDTMR

SEQ ID NO: 50120 - protein, 9 aa, synthetic construct
GGLGRDTMT

SEQ ID NO: 50121 - protein, 9 aa, synthetic construct
GGLGRDTMY

SEQ ID NO: 50122 - protein, 9 aa, synthetic construct
GGLGRDTVL

SEQ ID NO: 50123 - protein, 9 aa, synthetic construct
GGLGRDTYE

SEQ ID NO: 50124 - protein, 9 aa, synthetic construct
GGLGRDSYY

SEQ ID NO: 50125 - protein, 9 aa, synthetic construct
GGLGRDVFH

SEQ ID NO: 50126 - protein, 9 aa, synthetic construct
GGLGRDVFL

SEQ ID NO: 50127 - protein, 9 aa, synthetic construct
GGLGRDVFV

SEQ ID NO: 50128 - protein, 9 aa, synthetic construct
GGLGRDVIS

SEQ ID NO: 50129 - protein, 9 aa, synthetic construct
GGLGRDVIT

SEQ ID NO: 50130 - protein, 9 aa, synthetic construct
GGLGRDVLG

SEQ ID NO: 50131 - protein, 9 aa, synthetic construct
GGLGRDVME

SEQ ID NO: 50132 - protein, 9 aa, synthetic construct
GGLGRDWLS

SEQ ID NO: 50133 - protein, 9 aa, synthetic construct
GGLGRDWLT

SEQ ID NO: 50134 - protein, 9 aa, synthetic construct
GGLGRDWLW

SEQ ID NO: 50135 - protein, 9 aa, synthetic construct
GGLGRDYLV

SEQ ID NO: 50136 - protein, 9 aa, synthetic construct
GGLGRDYMD

SEQ ID NO: 50137 - protein, 9 aa, synthetic construct
GGLGRDYMT

SEQ ID NO: 50138 - protein, 9 aa, synthetic construct
GGLGRDTAL

SEQ ID NO: 50139 - protein, 9 aa, synthetic construct
GGLGRDSLY

SEQ ID NO: 50140 - protein, 9 aa, synthetic construct
GGLGRDLLE

SEQ ID NO: 50141 - protein, 9 aa, synthetic construct
GGLGRDQMR

SEQ ID NO: 50142 - protein, 9 aa, synthetic construct
GGLGRDLLL

SEQ ID NO: 50143 - protein, 9 aa, synthetic construct
GGLGRDLLS

SEQ ID NO: 50144 - protein, 9 aa, synthetic construct
GGLGRDLLY

SEQ ID NO: 50145 - protein, 9 aa, synthetic construct
GGLGRDLMS

SEQ ID NO: 50146 - protein, 9 aa, synthetic construct
GGLGRDLVS

SEQ ID NO: 50147 - protein, 9 aa, synthetic construct
GGLGRDMLD

SEQ ID NO: 50148 - protein, 9 aa, synthetic construct
GGLGRDMLN

SEQ ID NO: 50149 - protein, 9 aa, synthetic construct
GGLGRDQFH

SEQ ID NO: 50150 - protein, 9 aa, synthetic construct
GGLGRDQLA

SEQ ID NO: 50151 - protein, 9 aa, synthetic construct
GGLGRDQLD

SEQ ID NO: 50152 - protein, 9 aa, synthetic construct
GGLGRDQLI

SEQ ID NO: 50153 - protein, 9 aa, synthetic construct
GGLGRDQLV

SEQ ID NO: 50154 - protein, 9 aa, synthetic construct
GGLGRDQLY

SEQ ID NO: 50155 - protein, 9 aa, synthetic construct
GGLGRDRAI

SEQ ID NO: 50156 - protein, 9 aa, synthetic construct
GGLGRDSLT

SEQ ID NO: 50157 - protein, 9 aa, synthetic construct
GGLGRDRFA

SEQ ID NO: 50158 - protein, 9 aa, synthetic construct
GGLGRDRIA

SEQ ID NO: 50159 - protein, 9 aa, synthetic construct
GGLGRDRID

SEQ ID NO: 50160 - protein, 9 aa, synthetic construct
GGLGRDRLN

SEQ ID NO: 50161 - protein, 9 aa, synthetic construct
GGLGRDRLR

SEQ ID NO: 50162 - protein, 9 aa, synthetic construct
GGLGRDRLW

SEQ ID NO: 50163 - protein, 9 aa, synthetic construct
GGLGRDRVD

SEQ ID NO: 50164 - protein, 9 aa, synthetic construct
GGLGRDRVL

SEQ ID NO: 50165 - protein, 9 aa, synthetic construct
GGLGRDSIL

SEQ ID NO: 50166 - protein, 9 aa, synthetic construct
GGLGRDSLA

SEQ ID NO: 50167 - protein, 9 aa, synthetic construct
GGLGRDSLD

SEQ ID NO: 50168 - protein, 9 aa, synthetic construct
GGLGRDSLF

SEQ ID NO: 50169 - protein, 9 aa, synthetic construct
GGLGRDSLI

SEQ ID NO: 50170 - protein, 9 aa, synthetic construct
GGLGNDAIS

SEQ ID NO: 50171 - protein, 9 aa, synthetic construct
GGLGNDAIH

SEQ ID NO: 50172 - protein, 9 aa, synthetic construct
GGLGNDAFI

SEQ ID NO: 50173 - protein, 9 aa, synthetic construct
GGLGFDVIL

SEQ ID NO: 50174 - protein, 9 aa, synthetic construct
GGLGFDIAA

SEQ ID NO: 50175 - protein, 9 aa, synthetic construct
GGLGFDILN

SEQ ID NO: 50176 - protein, 9 aa, synthetic construct
GGLGFDILS

SEQ ID NO: 50177 - protein, 9 aa, synthetic construct
GGLGFDKMG

SEQ ID NO: 50178 - protein, 9 aa, synthetic construct
GGLGFDLAD

SEQ ID NO: 50179 - protein, 9 aa, synthetic construct
GGLGFDLLL

SEQ ID NO: 50180 - protein, 9 aa, synthetic construct
GGLGFDLLN

SEQ ID NO: 50181 - protein, 9 aa, synthetic construct
GGLGFDLMT

SEQ ID NO: 50182 - protein, 9 aa, synthetic construct
GGLGFDMAS

SEQ ID NO: 50183 - protein, 9 aa, synthetic construct
GGLGFDRIN

SEQ ID NO: 50184 - protein, 9 aa, synthetic construct
GGLGFDRLA

SEQ ID NO: 50185 - protein, 9 aa, synthetic construct
GGLGFDRLG

SEQ ID NO: 50186 - protein, 9 aa, synthetic construct
GGLGFDRLN

SEQ ID NO: 50187 - protein, 9 aa, synthetic construct
GGLGFDRVS

SEQ ID NO: 50188 - protein, 9 aa, synthetic construct
GGLGFDSLD

SEQ ID NO: 50189 - protein, 9 aa, synthetic construct
GGLGFDSLE

SEQ ID NO: 50190 - protein, 9 aa, synthetic construct
GGLGFDSMS

SEQ ID NO: 50191 - protein, 9 aa, synthetic construct
GGLGFDTAS

SEQ ID NO: 50192 - protein, 9 aa, synthetic construct
GGLGFDTFA

SEQ ID NO: 50193 - protein, 9 aa, synthetic construct
GGLGFDTID

SEQ ID NO: 50194 - protein, 9 aa, synthetic construct
GGLGFDTIS

SEQ ID NO: 50195 - protein, 9 aa, synthetic construct
GGLGFDTIY

SEQ ID NO: 50196 - protein, 9 aa, synthetic construct
GGLGFDTLH

SEQ ID NO: 50197 - protein, 9 aa, synthetic construct
GGLGFDTLL

SEQ ID NO: 50198 - protein, 9 aa, synthetic construct
GGLGFDTLV

SEQ ID NO: 50199 - protein, 9 aa, synthetic construct
GGLGFDTYQ

SEQ ID NO: 50200 - protein, 9 aa, synthetic construct
GGLGFDVAE

SEQ ID NO: 50201 - protein, 9 aa, synthetic construct
GGLGFDVAT

SEQ ID NO: 50202 - protein, 9 aa, synthetic construct
GGLGFDVFV

SEQ ID NO: 50203 - protein, 9 aa, synthetic construct
GGLGFDFLS

SEQ ID NO: 50204 - protein, 9 aa, synthetic construct
GGLGFDFAS

SEQ ID NO: 50205 - protein, 9 aa, synthetic construct
GGLGFDEMD

SEQ ID NO: 50206 - protein, 9 aa, synthetic construct
GGLGEDVFV

SEQ ID NO: 50207 - protein, 9 aa, synthetic construct
GGLGEDSLQ

SEQ ID NO: 50208 - protein, 9 aa, synthetic construct
GGLGEDSLR

SEQ ID NO: 50209 - protein, 9 aa, synthetic construct
GGLGEDSLS

SEQ ID NO: 50210 - protein, 9 aa, synthetic construct
GGLGEDTAD

SEQ ID NO: 50211 - protein, 9 aa, synthetic construct
GGLGEDTFH

SEQ ID NO: 50212 - protein, 9 aa, synthetic construct
GGLGEDTFN

SEQ ID NO: 50213 - protein, 9 aa, synthetic construct
GGLGEDTIY

SEQ ID NO: 50214 - protein, 9 aa, synthetic construct
GGLGEDTLA

SEQ ID NO: 50215 - protein, 9 aa, synthetic construct
GGLGEDTLD

SEQ ID NO: 50216 - protein, 9 aa, synthetic construct
GGLGEDTLK

SEQ ID NO: 50217 - protein, 9 aa, synthetic construct
GGLGEDTLL

SEQ ID NO: 50218 - protein, 9 aa, synthetic construct
GGLGEDTML

SEQ ID NO: 50219 - protein, 9 aa, synthetic construct
GGLGEDTYF

SEQ ID NO: 50220 - protein, 9 aa, synthetic construct
GGLGEDVID

SEQ ID NO: 50221 - protein, 9 aa, synthetic construct
GGLGFDEIN

SEQ ID NO: 50222 - protein, 9 aa, synthetic construct
GGLGEDVIF

SEQ ID NO: 50223 - protein, 9 aa, synthetic construct
GGLGEDVIY

SEQ ID NO: 50224 - protein, 9 aa, synthetic construct
GGLGEDVLA

SEQ ID NO: 50225 - protein, 9 aa, synthetic construct
GGLGEDVLS

SEQ ID NO: 50226 - protein, 9 aa, synthetic construct
GGLGEDVLV

SEQ ID NO: 50227 - protein, 9 aa, synthetic construct
GGLGEDVLY

SEQ ID NO: 50228 - protein, 9 aa, synthetic construct
GGLGEDWLD

SEQ ID NO: 50229 - protein, 9 aa, synthetic construct
GGLGEDWLI

SEQ ID NO: 50230 - protein, 9 aa, synthetic construct
GGLGEDWLL

SEQ ID NO: 50231 - protein, 9 aa, synthetic construct
GGLGFDAID

SEQ ID NO: 50232 - protein, 9 aa, synthetic construct
GGLGFDDLH

SEQ ID NO: 50233 - protein, 9 aa, synthetic construct
GGLGFDDLI

SEQ ID NO: 50234 - protein, 9 aa, synthetic construct
GGLGFDDMY

SEQ ID NO: 50235 - protein, 9 aa, synthetic construct
GGLGFDVIE

SEQ ID NO: 50236 - protein, 9 aa, synthetic construct
GGLGFDVIT

SEQ ID NO: 50237 - protein, 9 aa, synthetic construct
GGLGNDAAY

SEQ ID NO: 50238 - protein, 9 aa, synthetic construct
GGLGFDVLD

SEQ ID NO: 50239 - protein, 9 aa, synthetic construct
GGLGGDMLS

SEQ ID NO: 50240 - protein, 9 aa, synthetic construct
GGLGGDNLL

SEQ ID NO: 50241 - protein, 9 aa, synthetic construct
GGLGGDQLT

SEQ ID NO: 50242 - protein, 9 aa, synthetic construct
GGLGGDRIL

SEQ ID NO: 50243 - protein, 9 aa, synthetic construct
GGLGGDRLH

SEQ ID NO: 50244 - protein, 9 aa, synthetic construct
GGLGGDRLI

SEQ ID NO: 50245 - protein, 9 aa, synthetic construct
GGLGGDRLK

SEQ ID NO: 50246 - protein, 9 aa, synthetic construct
GGLGGDRME

SEQ ID NO: 50247 - protein, 9 aa, synthetic construct
GGLGGDRYV

SEQ ID NO: 50248 - protein, 9 aa, synthetic construct
GGLGGDSLE

SEQ ID NO: 50249 - protein, 9 aa, synthetic construct
GGLGGDSLR

SEQ ID NO: 50250 - protein, 9 aa, synthetic construct
GGLGGDSLS

SEQ ID NO: 50251 - protein, 9 aa, synthetic construct
GGLGGDTFA

SEQ ID NO: 50252 - protein, 9 aa, synthetic construct
GGLGGDTFH

SEQ ID NO: 50253 - protein, 9 aa, synthetic construct
GGLGGDTFL

SEQ ID NO: 50254 - protein, 9 aa, synthetic construct
GGLGGDTIA

SEQ ID NO: 50255 - protein, 9 aa, synthetic construct
GGLGGDTIH

SEQ ID NO: 50256 - protein, 9 aa, synthetic construct
GGLGGDTIK

SEQ ID NO: 50257 - protein, 9 aa, synthetic construct
GGLGGDTLA

SEQ ID NO: 50258 - protein, 9 aa, synthetic construct
GGLGGDTLF

SEQ ID NO: 50259 - protein, 9 aa, synthetic construct
GGLGGDTLG

SEQ ID NO: 50260 - protein, 9 aa, synthetic construct
GGLGGDTLN

SEQ ID NO: 50261 - protein, 9 aa, synthetic construct
GGLGGDTLQ

SEQ ID NO: 50262 - protein, 9 aa, synthetic construct
GGLGGDTMA

SEQ ID NO: 50263 - protein, 9 aa, synthetic construct
GGLGGDTMF

SEQ ID NO: 50264 - protein, 9 aa, synthetic construct
GGLGGDTMS

SEQ ID NO: 50265 - protein, 9 aa, synthetic construct
GGLGGDTMY

SEQ ID NO: 50266 - protein, 9 aa, synthetic construct
GGLGGDTYH

SEQ ID NO: 50267 - protein, 9 aa, synthetic construct
GGLGGDTYL

SEQ ID NO: 50268 - protein, 9 aa, synthetic construct
GGLGGDLMT

SEQ ID NO: 50269 - protein, 9 aa, synthetic construct
GGLGGDLMS

SEQ ID NO: 50270 - protein, 9 aa, synthetic construct
GGLGGDLLY

SEQ ID NO: 50271 - protein, 9 aa, synthetic construct
GGLGGDELF

SEQ ID NO: 50272 - protein, 9 aa, synthetic construct
GGLGFDVLR

SEQ ID NO: 50273 - protein, 9 aa, synthetic construct
GGLGFDVLS

SEQ ID NO: 50274 - protein, 9 aa, synthetic construct
GGLGFDWLD

SEQ ID NO: 50275 - protein, 9 aa, synthetic construct
GGLGFDYAY

SEQ ID NO: 50276 - protein, 9 aa, synthetic construct
GGLGGDALD

SEQ ID NO: 50277 - protein, 9 aa, synthetic construct
GGLGGDALK

SEQ ID NO: 50278 - protein, 9 aa, synthetic construct
GGLGGDALL

SEQ ID NO: 50279 - protein, 9 aa, synthetic construct
GGLGGDALN

SEQ ID NO: 50280 - protein, 9 aa, synthetic construct
GGLGGDALR

SEQ ID NO: 50281 - protein, 9 aa, synthetic construct
GGLGGDALY

SEQ ID NO: 50282 - protein, 9 aa, synthetic construct
GGLGGDAMA

SEQ ID NO: 50283 - protein, 9 aa, synthetic construct
GGLGGDDLT

SEQ ID NO: 50284 - protein, 9 aa, synthetic construct
GGLGGDDLY

SEQ ID NO: 50285 - protein, 9 aa, synthetic construct
GGLGGDEMS

SEQ ID NO: 50286 - protein, 9 aa, synthetic construct
GGLGGDLLR

SEQ ID NO: 50287 - protein, 9 aa, synthetic construct
GGLGGDFIY

SEQ ID NO: 50288 - protein, 9 aa, synthetic construct
GGLGGDFLF

SEQ ID NO: 50289 - protein, 9 aa, synthetic construct
GGLGGDFLL

SEQ ID NO: 50290 - protein, 9 aa, synthetic construct
GGLGGDFLR

SEQ ID NO: 50291 - protein, 9 aa, synthetic construct
GGLGGDIIS

SEQ ID NO: 50292 - protein, 9 aa, synthetic construct
GGLGGDILF

SEQ ID NO: 50293 - protein, 9 aa, synthetic construct
GGLGGDILW

SEQ ID NO: 50294 - protein, 9 aa, synthetic construct
GGLGGDILY

SEQ ID NO: 50295 - protein, 9 aa, synthetic construct
GGLGGDIMD

SEQ ID NO: 50296 - protein, 9 aa, synthetic construct
GGLGGDKLI

SEQ ID NO: 50297 - protein, 9 aa, synthetic construct
GGLGGDKLW

SEQ ID NO: 50298 - protein, 9 aa, synthetic construct
GGLGGDKLY

SEQ ID NO: 50299 - protein, 9 aa, synthetic construct
GGLGGDLLK

SEQ ID NO: 50300 - protein, 9 aa, synthetic construct
GGLGEDSLL

SEQ ID NO: 50301 - protein, 9 aa, synthetic construct
GGLGEDSLF

SEQ ID NO: 50302 - protein, 9 aa, synthetic construct
GGLGEDSIV

SEQ ID NO: 50303 - protein, 9 aa, synthetic construct
GGLGEDRMT

SEQ ID NO: 50304 - protein, 9 aa, synthetic construct
GGLGDDSVR

SEQ ID NO: 50305 - protein, 9 aa, synthetic construct
GGLGDDSVS

SEQ ID NO: 50306 - protein, 9 aa, synthetic construct
GGLGDDSVW

SEQ ID NO: 50307 - protein, 9 aa, synthetic construct
GGLGDDSYL

SEQ ID NO: 50308 - protein, 9 aa, synthetic construct
GGLGDDSYT

SEQ ID NO: 50309 - protein, 9 aa, synthetic construct
GGLGDDTAS

SEQ ID NO: 50310 - protein, 9 aa, synthetic construct
GGLGDDTAV

SEQ ID NO: 50311 - protein, 9 aa, synthetic construct
GGLGDDTFD

SEQ ID NO: 50312 - protein, 9 aa, synthetic construct
GGLGDDTFE

SEQ ID NO: 50313 - protein, 9 aa, synthetic construct
GGLGDDTFF

SEQ ID NO: 50314 - protein, 9 aa, synthetic construct
GGLGDDTFG

SEQ ID NO: 50315 - protein, 9 aa, synthetic construct
GGLGDDTFH

SEQ ID NO: 50316 - protein, 9 aa, synthetic construct
GGLGDDTFR

SEQ ID NO: 50317 - protein, 9 aa, synthetic construct
GGLGDDTIK

SEQ ID NO: 50318 - protein, 9 aa, synthetic construct
GGLGDDTLM

SEQ ID NO: 50319 - protein, 9 aa, synthetic construct
GGLGDDTME

SEQ ID NO: 50320 - protein, 9 aa, synthetic construct
GGLGDDTMH

SEQ ID NO: 50321 - protein, 9 aa, synthetic construct
GGLGDDTMR

SEQ ID NO: 50322 - protein, 9 aa, synthetic construct
GGLGDDTMS

SEQ ID NO: 50323 - protein, 9 aa, synthetic construct
GGLGDDTMV

SEQ ID NO: 50324 - protein, 9 aa, synthetic construct
GGLGDDTYA

SEQ ID NO: 50325 - protein, 9 aa, synthetic construct
GGLGDDTYE

SEQ ID NO: 50326 - protein, 9 aa, synthetic construct
GGLGDDTYN

SEQ ID NO: 50327 - protein, 9 aa, synthetic construct
GGLGDDTYS

SEQ ID NO: 50328 - protein, 9 aa, synthetic construct
GGLGDDVAA

SEQ ID NO: 50329 - protein, 9 aa, synthetic construct
GGLGDDVAL

SEQ ID NO: 50330 - protein, 9 aa, synthetic construct
GGLGDDVFI

SEQ ID NO: 50331 - protein, 9 aa, synthetic construct
GGLGDDVFM

SEQ ID NO: 50332 - protein, 9 aa, synthetic construct
GGLGDDVFS

SEQ ID NO: 50333 - protein, 9 aa, synthetic construct
GGLGDDSVN

SEQ ID NO: 50334 - protein, 9 aa, synthetic construct
GGLGDDSVL

SEQ ID NO: 50335 - protein, 9 aa, synthetic construct
GGLGDDSVH

SEQ ID NO: 50336 - protein, 9 aa, synthetic construct
GGLGDDSAD

SEQ ID NO: 50337 - protein, 9 aa, synthetic construct
GGLGDDQVS

SEQ ID NO: 50338 - protein, 9 aa, synthetic construct
GGLGDDRFE

SEQ ID NO: 50339 - protein, 9 aa, synthetic construct
GGLGDDRFI

SEQ ID NO: 50340 - protein, 9 aa, synthetic construct
GGLGDDRFY

SEQ ID NO: 50341 - protein, 9 aa, synthetic construct
GGLGDDRII

SEQ ID NO: 50342 - protein, 9 aa, synthetic construct
GGLGDDRIL

SEQ ID NO: 50343 - protein, 9 aa, synthetic construct
GGLGDDRIQ

SEQ ID NO: 50344 - protein, 9 aa, synthetic construct
GGLGDDRLG

SEQ ID NO: 50345 - protein, 9 aa, synthetic construct
GGLGDDRLH

SEQ ID NO: 50346 - protein, 9 aa, synthetic construct
GGLGDDRLK

SEQ ID NO: 50347 - protein, 9 aa, synthetic construct
GGLGDDRMA

SEQ ID NO: 50348 - protein, 9 aa, synthetic construct
GGLGDDRVE

SEQ ID NO: 50349 - protein, 9 aa, synthetic construct
GGLGDDRVF

SEQ ID NO: 50350 - protein, 9 aa, synthetic construct
GGLGDDSAG

SEQ ID NO: 50351 - protein, 9 aa, synthetic construct
GGLGDDSVD

SEQ ID NO: 50352 - protein, 9 aa, synthetic construct
GGLGDDSFD

SEQ ID NO: 50353 - protein, 9 aa, synthetic construct
GGLGDDSFI

SEQ ID NO: 50354 - protein, 9 aa, synthetic construct
GGLGDDSFT

SEQ ID NO: 50355 - protein, 9 aa, synthetic construct
GGLGDDSFV

SEQ ID NO: 50356 - protein, 9 aa, synthetic construct
GGLGDDSFY

SEQ ID NO: 50357 - protein, 9 aa, synthetic construct
GGLGDDSIA

SEQ ID NO: 50358 - protein, 9 aa, synthetic construct
GGLGDDSIG

SEQ ID NO: 50359 - protein, 9 aa, synthetic construct
GGLGDDSLW

SEQ ID NO: 50360 - protein, 9 aa, synthetic construct
GGLGDDSLY

SEQ ID NO: 50361 - protein, 9 aa, synthetic construct
GGLGDDSMI

SEQ ID NO: 50362 - protein, 9 aa, synthetic construct
GGLGDDSMM

SEQ ID NO: 50363 - protein, 9 aa, synthetic construct
GGLGDDSMQ

SEQ ID NO: 50364 - protein, 9 aa, synthetic construct
GGLGDDSMS

SEQ ID NO: 50365 - protein, 9 aa, synthetic construct
GGLGDDVIT

SEQ ID NO: 50366 - protein, 9 aa, synthetic construct
GGLGDDVIW

SEQ ID NO: 50367 - protein, 9 aa, synthetic construct
GGLGDDVLM

SEQ ID NO: 50368 - protein, 9 aa, synthetic construct
GGLGEDIVD

SEQ ID NO: 50369 - protein, 9 aa, synthetic construct
GGLGEDAAI

SEQ ID NO: 50370 - protein, 9 aa, synthetic construct
GGLGEDALY

SEQ ID NO: 50371 - protein, 9 aa, synthetic construct
GGLGEDDID

SEQ ID NO: 50372 - protein, 9 aa, synthetic construct
GGLGEDDLR

SEQ ID NO: 50373 - protein, 9 aa, synthetic construct
GGLGEDEIL

SEQ ID NO: 50374 - protein, 9 aa, synthetic construct
GGLGEDEML

SEQ ID NO: 50375 - protein, 9 aa, synthetic construct
GGLGEDFLF

SEQ ID NO: 50376 - protein, 9 aa, synthetic construct
GGLGEDIIL

SEQ ID NO: 50377 - protein, 9 aa, synthetic construct
GGLGEDILK

SEQ ID NO: 50378 - protein, 9 aa, synthetic construct
GGLGEDILN

SEQ ID NO: 50379 - protein, 9 aa, synthetic construct
GGLGEDILV

SEQ ID NO: 50380 - protein, 9 aa, synthetic construct
GGLGEDILY

SEQ ID NO: 50381 - protein, 9 aa, synthetic construct
GGLGEDIMT

SEQ ID NO: 50382 - protein, 9 aa, synthetic construct
GGLGEDIYY

SEQ ID NO: 50383 - protein, 9 aa, synthetic construct
GGLGDDYVH

SEQ ID NO: 50384 - protein, 9 aa, synthetic construct
GGLGEDKIT

SEQ ID NO: 50385 - protein, 9 aa, synthetic construct
GGLGEDKLS

SEQ ID NO: 50386 - protein, 9 aa, synthetic construct
GGLGEDKMI

SEQ ID NO: 50387 - protein, 9 aa, synthetic construct
GGLGEDLFS

SEQ ID NO: 50388 - protein, 9 aa, synthetic construct
GGLGEDLLL

SEQ ID NO: 50389 - protein, 9 aa, synthetic construct
GGLGEDLVY

SEQ ID NO: 50390 - protein, 9 aa, synthetic construct
GGLGEDNLT

SEQ ID NO: 50391 - protein, 9 aa, synthetic construct
GGLGEDRFF

SEQ ID NO: 50392 - protein, 9 aa, synthetic construct
GGLGEDRIV

SEQ ID NO: 50393 - protein, 9 aa, synthetic construct
GGLGEDRLA

SEQ ID NO: 50394 - protein, 9 aa, synthetic construct
GGLGEDRLD

SEQ ID NO: 50395 - protein, 9 aa, synthetic construct
GGLGEDRLH

SEQ ID NO: 50396 - protein, 9 aa, synthetic construct
GGLGEDRMD

SEQ ID NO: 50397 - protein, 9 aa, synthetic construct
GGLGDDYYF

SEQ ID NO: 50398 - protein, 9 aa, synthetic construct
GGLGDDYMA

SEQ ID NO: 50399 - protein, 9 aa, synthetic construct
GGLGDDVMH

SEQ ID NO: 50400 - protein, 9 aa, synthetic construct
GGLGDDWLG

SEQ ID NO: 50401 - protein, 9 aa, synthetic construct
GGLGDDVVE

SEQ ID NO: 50402 - protein, 9 aa, synthetic construct
GGLGDDVVF

SEQ ID NO: 50403 - protein, 9 aa, synthetic construct
GGLGDDVVK

SEQ ID NO: 50404 - protein, 9 aa, synthetic construct
GGLGDDVVT

SEQ ID NO: 50405 - protein, 9 aa, synthetic construct
GGLGDDVVV

SEQ ID NO: 50406 - protein, 9 aa, synthetic construct
GGLGDDVYC

SEQ ID NO: 50407 - protein, 9 aa, synthetic construct
GGLGDDVYD

SEQ ID NO: 50408 - protein, 9 aa, synthetic construct
GGLGDDVYF

SEQ ID NO: 50409 - protein, 9 aa, synthetic construct
GGLGDDVYW

SEQ ID NO: 50410 - protein, 9 aa, synthetic construct
GGLGDDWFR

SEQ ID NO: 50411 - protein, 9 aa, synthetic construct
GGLGDDWIE

SEQ ID NO: 50412 - protein, 9 aa, synthetic construct
GGLGDDWIN

SEQ ID NO: 50413 - protein, 9 aa, synthetic construct
GGLGDDWLE

SEQ ID NO: 50414 - protein, 9 aa, synthetic construct
GGLGDDWLH

SEQ ID NO: 50415 - protein, 9 aa, synthetic construct
GGLGDDYLY

SEQ ID NO: 50416 - protein, 9 aa, synthetic construct
GGLGDDWLI

SEQ ID NO: 50417 - protein, 9 aa, synthetic construct
GGLGDDWLQ

SEQ ID NO: 50418 - protein, 9 aa, synthetic construct
GGLGDDWLT

SEQ ID NO: 50419 - protein, 9 aa, synthetic construct
GGLGDDWVE

SEQ ID NO: 50420 - protein, 9 aa, synthetic construct
GGLGDDXLI

SEQ ID NO: 50421 - protein, 9 aa, synthetic construct
GGLGDDYAD

SEQ ID NO: 50422 - protein, 9 aa, synthetic construct
GGLGDDYFE

SEQ ID NO: 50423 - protein, 9 aa, synthetic construct
GGLGDDYFV

SEQ ID NO: 50424 - protein, 9 aa, synthetic construct
GGLGDDYIA

SEQ ID NO: 50425 - protein, 9 aa, synthetic construct
GGLGDDYIE

SEQ ID NO: 50426 - protein, 9 aa, synthetic construct
GGLGDDYLI

SEQ ID NO: 50427 - protein, 9 aa, synthetic construct
GGLGDDYLR

SEQ ID NO: 50428 - protein, 9 aa, synthetic construct
GGLGDDYLT

SEQ ID NO: 50429 - protein, 9 aa, synthetic construct
GGLGGDVID

SEQ ID NO: 50430 - protein, 9 aa, synthetic construct
GGLGGDVIF

SEQ ID NO: 50431 - protein, 9 aa, synthetic construct
GGLGGDVIH

SEQ ID NO: 50432 - protein, 9 aa, synthetic construct
GGLGIDVLQ

SEQ ID NO: 50433 - protein, 9 aa, synthetic construct
GGLGKDRLI

SEQ ID NO: 50434 - protein, 9 aa, synthetic construct
GGLGKDRLK

SEQ ID NO: 50435 - protein, 9 aa, synthetic construct
GGLGKDRMT

SEQ ID NO: 50436 - protein, 9 aa, synthetic construct
GGLGKDSFV

SEQ ID NO: 50437 - protein, 9 aa, synthetic construct
GGLGKDSID

SEQ ID NO: 50438 - protein, 9 aa, synthetic construct
GGLGKDSYN

SEQ ID NO: 50439 - protein, 9 aa, synthetic construct
GGLGKDTFL

SEQ ID NO: 50440 - protein, 9 aa, synthetic construct
GGLGKDTID

SEQ ID NO: 50441 - protein, 9 aa, synthetic construct
GGLGKDTIS

SEQ ID NO: 50442 - protein, 9 aa, synthetic construct
GGLGKDTIT

SEQ ID NO: 50443 - protein, 9 aa, synthetic construct
GGLGKDTLA

SEQ ID NO: 50444 - protein, 9 aa, synthetic construct
GGLGKDTLF

SEQ ID NO: 50445 - protein, 9 aa, synthetic construct
GGLGKDTLR

SEQ ID NO: 50446 - protein, 9 aa, synthetic construct
GGLGKDTMD

SEQ ID NO: 50447 - protein, 9 aa, synthetic construct
GGLGKDTMI

SEQ ID NO: 50448 - protein, 9 aa, synthetic construct
GGLGKDTMK

SEQ ID NO: 50449 - protein, 9 aa, synthetic construct
GGLGKDTVD

SEQ ID NO: 50450 - protein, 9 aa, synthetic construct
GGLGKDTYD

SEQ ID NO: 50451 - protein, 9 aa, synthetic construct
GGLGKDVAA

SEQ ID NO: 50452 - protein, 9 aa, synthetic construct
GGLGKDVIT

SEQ ID NO: 50453 - protein, 9 aa, synthetic construct
GGLGKDVLY

SEQ ID NO: 50454 - protein, 9 aa, synthetic construct
GGLGKDVMM

SEQ ID NO: 50455 - protein, 9 aa, synthetic construct
GGLGKDVVA

SEQ ID NO: 50456 - protein, 9 aa, synthetic construct
GGLGKDWAE

SEQ ID NO: 50457 - protein, 9 aa, synthetic construct
GGLGKDYLD

SEQ ID NO: 50458 - protein, 9 aa, synthetic construct
GGLGLDAIT

SEQ ID NO: 50459 - protein, 9 aa, synthetic construct
GGLGLDALF

SEQ ID NO: 50460 - protein, 9 aa, synthetic construct
GGLGLDALH

SEQ ID NO: 50461 - protein, 9 aa, synthetic construct
GGLGLDALI

SEQ ID NO: 50462 - protein, 9 aa, synthetic construct
GGLGKDRLE

SEQ ID NO: 50463 - protein, 9 aa, synthetic construct
GGLGKDRID

SEQ ID NO: 50464 - protein, 9 aa, synthetic construct
GGLGKDQLK

SEQ ID NO: 50465 - protein, 9 aa, synthetic construct
GGLGKDIMK

SEQ ID NO: 50466 - protein, 9 aa, synthetic construct
GGLGIDVMT

SEQ ID NO: 50467 - protein, 9 aa, synthetic construct
GGLGIDVVN

SEQ ID NO: 50468 - protein, 9 aa, synthetic construct
GGLGIDWIY

SEQ ID NO: 50469 - protein, 9 aa, synthetic construct
GGLGIDWVT

SEQ ID NO: 50470 - protein, 9 aa, synthetic construct
GGLGKDEID

SEQ ID NO: 50471 - protein, 9 aa, synthetic construct
GGLGKDEIQ

SEQ ID NO: 50472 - protein, 9 aa, synthetic construct
GGLGKDELQ

SEQ ID NO: 50473 - protein, 9 aa, synthetic construct
GGLGKDFLV

SEQ ID NO: 50474 - protein, 9 aa, synthetic construct
GGLGKDFMH

SEQ ID NO: 50475 - protein, 9 aa, synthetic construct
GGLGKDHLT

SEQ ID NO: 50476 - protein, 9 aa, synthetic construct
GGLGKDHLY

SEQ ID NO: 50477 - protein, 9 aa, synthetic construct
GGLGKDILK

SEQ ID NO: 50478 - protein, 9 aa, synthetic construct
GGLGKDILV

SEQ ID NO: 50479 - protein, 9 aa, synthetic construct
GGLGKDKLF

SEQ ID NO: 50480 - protein, 9 aa, synthetic construct
GGLGKDQLH

SEQ ID NO: 50481 - protein, 9 aa, synthetic construct
GGLGKDKLV

SEQ ID NO: 50482 - protein, 9 aa, synthetic construct
GGLGKDKMT

SEQ ID NO: 50483 - protein, 9 aa, synthetic construct
GGLGKDKVA

SEQ ID NO: 50484 - protein, 9 aa, synthetic construct
GGLGKDLLD

SEQ ID NO: 50485 - protein, 9 aa, synthetic construct
GGLGKDLLK

SEQ ID NO: 50486 - protein, 9 aa, synthetic construct
GGLGKDLLL

SEQ ID NO: 50487 - protein, 9 aa, synthetic construct
GGLGKDLLN

SEQ ID NO: 50488 - protein, 9 aa, synthetic construct
GGLGKDLLY

SEQ ID NO: 50489 - protein, 9 aa, synthetic construct
GGLGKDMLS

SEQ ID NO: 50490 - protein, 9 aa, synthetic construct
GGLGKDNIN

SEQ ID NO: 50491 - protein, 9 aa, synthetic construct
GGLGKDNLR

SEQ ID NO: 50492 - protein, 9 aa, synthetic construct
GGLGKDNLS

SEQ ID NO: 50493 - protein, 9 aa, synthetic construct
GGLGKDQLF

SEQ ID NO: 50494 - protein, 9 aa, synthetic construct
GGLGLDEIF

SEQ ID NO: 50495 - protein, 9 aa, synthetic construct
GGLGLDELS

SEQ ID NO: 50496 - protein, 9 aa, synthetic construct
GGLGLDELT

SEQ ID NO: 50497 - protein, 9 aa, synthetic construct
GGLGLDVVD

SEQ ID NO: 50498 - protein, 9 aa, synthetic construct
GGLGLDTLH

SEQ ID NO: 50499 - protein, 9 aa, synthetic construct
GGLGLDTLL

SEQ ID NO: 50500 - protein, 9 aa, synthetic construct
GGLGLDTMI

SEQ ID NO: 50501 - protein, 9 aa, synthetic construct
GGLGLDTMT

SEQ ID NO: 50502 - protein, 9 aa, synthetic construct
GGLGLDTVR

SEQ ID NO: 50503 - protein, 9 aa, synthetic construct
GGLGLDTVS

SEQ ID NO: 50504 - protein, 9 aa, synthetic construct
GGLGLDTVY

SEQ ID NO: 50505 - protein, 9 aa, synthetic construct
GGLGLDTYI

SEQ ID NO: 50506 - protein, 9 aa, synthetic construct
GGLGLDTYK

SEQ ID NO: 50507 - protein, 9 aa, synthetic construct
GGLGLDVAS

SEQ ID NO: 50508 - protein, 9 aa, synthetic construct
GGLGLDVFV

SEQ ID NO: 50509 - protein, 9 aa, synthetic construct
GGLGLDVLE

SEQ ID NO: 50510 - protein, 9 aa, synthetic construct
GGLGLDVLY

SEQ ID NO: 50511 - protein, 9 aa, synthetic construct
GGLGLDYLT

SEQ ID NO: 50512 - protein, 9 aa, synthetic construct
GGLGLDTLA

SEQ ID NO: 50513 - protein, 9 aa, synthetic construct
GGLGMDELF

SEQ ID NO: 50514 - protein, 9 aa, synthetic construct
GGLGMDELT

SEQ ID NO: 50515 - protein, 9 aa, synthetic construct
GGLGMDILD

SEQ ID NO: 50516 - protein, 9 aa, synthetic construct
GGLGMDMLT

SEQ ID NO: 50517 - protein, 9 aa, synthetic construct
GGLGMDQLT

SEQ ID NO: 50518 - protein, 9 aa, synthetic construct
GGLGMDRLY

SEQ ID NO: 50519 - protein, 9 aa, synthetic construct
GGLGMDTLE

SEQ ID NO: 50520 - protein, 9 aa, synthetic construct
GGLGMDTLN

SEQ ID NO: 50521 - protein, 9 aa, synthetic construct
GGLGMDTLS

SEQ ID NO: 50522 - protein, 9 aa, synthetic construct
GGLGMDTLY

SEQ ID NO: 50523 - protein, 9 aa, synthetic construct
GGLGMDTVT

SEQ ID NO: 50524 - protein, 9 aa, synthetic construct
GGLGMDVAG

SEQ ID NO: 50525 - protein, 9 aa, synthetic construct
GGLGMDVLT

SEQ ID NO: 50526 - protein, 9 aa, synthetic construct
GGLGLDTLE

SEQ ID NO: 50527 - protein, 9 aa, synthetic construct
GGLGLDTIQ

SEQ ID NO: 50528 - protein, 9 aa, synthetic construct
GGLGLDIID

SEQ ID NO: 50529 - protein, 9 aa, synthetic construct
GGLGLDQLR

SEQ ID NO: 50530 - protein, 9 aa, synthetic construct
GGLGLDIIL

SEQ ID NO: 50531 - protein, 9 aa, synthetic construct
GGLGLDILI

SEQ ID NO: 50532 - protein, 9 aa, synthetic construct
GGLGLDILL

SEQ ID NO: 50533 - protein, 9 aa, synthetic construct
GGLGLDKLV

SEQ ID NO: 50534 - protein, 9 aa, synthetic construct
GGLGLDKLY

SEQ ID NO: 50535 - protein, 9 aa, synthetic construct
GGLGLDLID

SEQ ID NO: 50536 - protein, 9 aa, synthetic construct
GGLGLDLIR

SEQ ID NO: 50537 - protein, 9 aa, synthetic construct
GGLGLDLLG

SEQ ID NO: 50538 - protein, 9 aa, synthetic construct
GGLGLDLLV

SEQ ID NO: 50539 - protein, 9 aa, synthetic construct
GGLGLDMAS

SEQ ID NO: 50540 - protein, 9 aa, synthetic construct
GGLGLDNLI

SEQ ID NO: 50541 - protein, 9 aa, synthetic construct
GGLGLDNLT

SEQ ID NO: 50542 - protein, 9 aa, synthetic construct
GGLGLDQLD

SEQ ID NO: 50543 - protein, 9 aa, synthetic construct
GGLGLDQLS

SEQ ID NO: 50544 - protein, 9 aa, synthetic construct
GGLGLDTIL

SEQ ID NO: 50545 - protein, 9 aa, synthetic construct
GGLGLDRAV

SEQ ID NO: 50546 - protein, 9 aa, synthetic construct
GGLGLDRIE

SEQ ID NO: 50547 - protein, 9 aa, synthetic construct
GGLGLDRLE

SEQ ID NO: 50548 - protein, 9 aa, synthetic construct
GGLGLDRLS

SEQ ID NO: 50549 - protein, 9 aa, synthetic construct
GGLGLDRLW

SEQ ID NO: 50550 - protein, 9 aa, synthetic construct
GGLGLDRVK

SEQ ID NO: 50551 - protein, 9 aa, synthetic construct
GGLGLDRVW

SEQ ID NO: 50552 - protein, 9 aa, synthetic construct
GGLGLDSAS

SEQ ID NO: 50553 - protein, 9 aa, synthetic construct
GGLGLDSLA

SEQ ID NO: 50554 - protein, 9 aa, synthetic construct
GGLGLDSLD

SEQ ID NO: 50555 - protein, 9 aa, synthetic construct
GGLGLDSLY

SEQ ID NO: 50556 - protein, 9 aa, synthetic construct
GGLGLDTAE

SEQ ID NO: 50557 - protein, 9 aa, synthetic construct
GGLGLDTFK

SEQ ID NO: 50558 - protein, 9 aa, synthetic construct
GGLGIDVLS

SEQ ID NO: 50559 - protein, 9 aa, synthetic construct
GGLGIDVLI

SEQ ID NO: 50560 - protein, 9 aa, synthetic construct
GGLGGDVLF

SEQ ID NO: 50561 - protein, 9 aa, synthetic construct
GGLGIDVLD

SEQ ID NO: 50562 - protein, 9 aa, synthetic construct
GGLGHDKLF

SEQ ID NO: 50563 - protein, 9 aa, synthetic construct
GGLGHDKLY

SEQ ID NO: 50564 - protein, 9 aa, synthetic construct
GGLGHDLLD

SEQ ID NO: 50565 - protein, 9 aa, synthetic construct
GGLGHDLLE

SEQ ID NO: 50566 - protein, 9 aa, synthetic construct
GGLGHDLLI

SEQ ID NO: 50567 - protein, 9 aa, synthetic construct
GGLGHDLLL

SEQ ID NO: 50568 - protein, 9 aa, synthetic construct
GGLGHDLLT

SEQ ID NO: 50569 - protein, 9 aa, synthetic construct
GGLGHDLLV

SEQ ID NO: 50570 - protein, 9 aa, synthetic construct
GGLGHDLMI

SEQ ID NO: 50571 - protein, 9 aa, synthetic construct
GGLGHDLMV

SEQ ID NO: 50572 - protein, 9 aa, synthetic construct
GGLGHDLYH

SEQ ID NO: 50573 - protein, 9 aa, synthetic construct
GGLGHDQLE

SEQ ID NO: 50574 - protein, 9 aa, synthetic construct
GGLGHDQLW

SEQ ID NO: 50575 - protein, 9 aa, synthetic construct
GGLGHDRLF

SEQ ID NO: 50576 - protein, 9 aa, synthetic construct
GGLGHDRLG

SEQ ID NO: 50577 - protein, 9 aa, synthetic construct
GGLGHDRLS

SEQ ID NO: 50578 - protein, 9 aa, synthetic construct
GGLGHDRLT

SEQ ID NO: 50579 - protein, 9 aa, synthetic construct
GGLGHDSIY

SEQ ID NO: 50580 - protein, 9 aa, synthetic construct
GGLGHDSLD

SEQ ID NO: 50581 - protein, 9 aa, synthetic construct
GGLGHDSMQ

SEQ ID NO: 50582 - protein, 9 aa, synthetic construct
GGLGHDSYT

SEQ ID NO: 50583 - protein, 9 aa, synthetic construct
GGLGHDTAD

SEQ ID NO: 50584 - protein, 9 aa, synthetic construct
GGLGHDTFV

SEQ ID NO: 50585 - protein, 9 aa, synthetic construct
GGLGHDTIE

SEQ ID NO: 50586 - protein, 9 aa, synthetic construct
GGLGHDTIS

SEQ ID NO: 50587 - protein, 9 aa, synthetic construct
GGLGHDTLD

SEQ ID NO: 50588 - protein, 9 aa, synthetic construct
GGLGHDTLG

SEQ ID NO: 50589 - protein, 9 aa, synthetic construct
GGLGHDTLK

SEQ ID NO: 50590 - protein, 9 aa, synthetic construct
GGLGHDTLM

SEQ ID NO: 50591 - protein, 9 aa, synthetic construct
GGLGHDIMT

SEQ ID NO: 50592 - protein, 9 aa, synthetic construct
GGLGHDILY

SEQ ID NO: 50593 - protein, 9 aa, synthetic construct
GGLGHDILW

SEQ ID NO: 50594 - protein, 9 aa, synthetic construct
GGLGHDELF

SEQ ID NO: 50595 - protein, 9 aa, synthetic construct
GGLGGDVLL

SEQ ID NO: 50596 - protein, 9 aa, synthetic construct
GGLGGDVMD

SEQ ID NO: 50597 - protein, 9 aa, synthetic construct
GGLGGDVMI

SEQ ID NO: 50598 - protein, 9 aa, synthetic construct
GGLGGDVMT

SEQ ID NO: 50599 - protein, 9 aa, synthetic construct
GGLGGDWLE

SEQ ID NO: 50600 - protein, 9 aa, synthetic construct
GGLGGDWLF

SEQ ID NO: 50601 - protein, 9 aa, synthetic construct
GGLGGDWLY

SEQ ID NO: 50602 - protein, 9 aa, synthetic construct
GGLGGDYLA

SEQ ID NO: 50603 - protein, 9 aa, synthetic construct
GGLGGDYLE

SEQ ID NO: 50604 - protein, 9 aa, synthetic construct
GGLGHDALF

SEQ ID NO: 50605 - protein, 9 aa, synthetic construct
GGLGHDALM

SEQ ID NO: 50606 - protein, 9 aa, synthetic construct
GGLGHDALT

SEQ ID NO: 50607 - protein, 9 aa, synthetic construct
GGLGHDDLT

SEQ ID NO: 50608 - protein, 9 aa, synthetic construct
GGLGHDELL

SEQ ID NO: 50609 - protein, 9 aa, synthetic construct
GGLGHDILS

SEQ ID NO: 50610 - protein, 9 aa, synthetic construct
GGLGHDEMH

SEQ ID NO: 50611 - protein, 9 aa, synthetic construct
GGLGHDFIS

SEQ ID NO: 50612 - protein, 9 aa, synthetic construct
GGLGHDFLL

SEQ ID NO: 50613 - protein, 9 aa, synthetic construct
GGLGHDFLS

SEQ ID NO: 50614 - protein, 9 aa, synthetic construct
GGLGHDFYI

SEQ ID NO: 50615 - protein, 9 aa, synthetic construct
GGLGHDGLF

SEQ ID NO: 50616 - protein, 9 aa, synthetic construct
GGLGHDGVE

SEQ ID NO: 50617 - protein, 9 aa, synthetic construct
GGLGHDHIS

SEQ ID NO: 50618 - protein, 9 aa, synthetic construct
GGLGHDHLT

SEQ ID NO: 50619 - protein, 9 aa, synthetic construct
GGLGHDIFY

SEQ ID NO: 50620 - protein, 9 aa, synthetic construct
GGLGHDIIA

SEQ ID NO: 50621 - protein, 9 aa, synthetic construct
GGLGHDILA

SEQ ID NO: 50622 - protein, 9 aa, synthetic construct
GGLGHDILI

SEQ ID NO: 50623 - protein, 9 aa, synthetic construct
GGLGHDTLN

SEQ ID NO: 50624 - protein, 9 aa, synthetic construct
GGLGHDTLW

SEQ ID NO: 50625 - protein, 9 aa, synthetic construct
GGLGHDTMR

SEQ ID NO: 50626 - protein, 9 aa, synthetic construct
GGLGIDTAR

SEQ ID NO: 50627 - protein, 9 aa, synthetic construct
GGLGIDNMI

SEQ ID NO: 50628 - protein, 9 aa, synthetic construct
GGLGIDQFR

SEQ ID NO: 50629 - protein, 9 aa, synthetic construct
GGLGIDRIY

SEQ ID NO: 50630 - protein, 9 aa, synthetic construct
GGLGIDRLA

SEQ ID NO: 50631 - protein, 9 aa, synthetic construct
GGLGIDRLM

SEQ ID NO: 50632 - protein, 9 aa, synthetic construct
GGLGIDRLN

SEQ ID NO: 50633 - protein, 9 aa, synthetic construct
GGLGIDRLS

SEQ ID NO: 50634 - protein, 9 aa, synthetic construct
GGLGIDRLY

SEQ ID NO: 50635 - protein, 9 aa, synthetic construct
GGLGIDRML

SEQ ID NO: 50636 - protein, 9 aa, synthetic construct
GGLGIDSLY

SEQ ID NO: 50637 - protein, 9 aa, synthetic construct
GGLGIDSME

SEQ ID NO: 50638 - protein, 9 aa, synthetic construct
GGLGIDTAD

SEQ ID NO: 50639 - protein, 9 aa, synthetic construct
GGLGIDTAK

SEQ ID NO: 50640 - protein, 9 aa, synthetic construct
GGLGIDTAV

SEQ ID NO: 50641 - protein, 9 aa, synthetic construct
GGLGIDLLY

SEQ ID NO: 50642 - protein, 9 aa, synthetic construct
GGLGIDTFM

SEQ ID NO: 50643 - protein, 9 aa, synthetic construct
GGLGIDTFT

SEQ ID NO: 50644 - protein, 9 aa, synthetic construct
GGLGIDTIE

SEQ ID NO: 50645 - protein, 9 aa, synthetic construct
GGLGIDTII

SEQ ID NO: 50646 - protein, 9 aa, synthetic construct
GGLGIDTLF

SEQ ID NO: 50647 - protein, 9 aa, synthetic construct
GGLGIDTME

SEQ ID NO: 50648 - protein, 9 aa, synthetic construct
GGLGIDTMF

SEQ ID NO: 50649 - protein, 9 aa, synthetic construct
GGLGIDTML

SEQ ID NO: 50650 - protein, 9 aa, synthetic construct
GGLGIDTMN

SEQ ID NO: 50651 - protein, 9 aa, synthetic construct
GGLGIDTMR

SEQ ID NO: 50652 - protein, 9 aa, synthetic construct
GGLGIDTYQ

SEQ ID NO: 50653 - protein, 9 aa, synthetic construct
GGLGIDVFA

SEQ ID NO: 50654 - protein, 9 aa, synthetic construct
GGLGIDVIY

SEQ ID NO: 50655 - protein, 9 aa, synthetic construct
GGLGIDNLS

SEQ ID NO: 50656 - protein, 9 aa, synthetic construct
GGLGIDLLT

SEQ ID NO: 50657 - protein, 9 aa, synthetic construct
GGLGHDTVH

SEQ ID NO: 50658 - protein, 9 aa, synthetic construct
GGLGHDWMA

SEQ ID NO: 50659 - protein, 9 aa, synthetic construct
GGLGHDTVL

SEQ ID NO: 50660 - protein, 9 aa, synthetic construct
GGLGHDTYI

SEQ ID NO: 50661 - protein, 9 aa, synthetic construct
GGLGHDTYY

SEQ ID NO: 50662 - protein, 9 aa, synthetic construct
GGLGHDVFQ

SEQ ID NO: 50663 - protein, 9 aa, synthetic construct
GGLGHDVIR

SEQ ID NO: 50664 - protein, 9 aa, synthetic construct
GGLGHDVIT

SEQ ID NO: 50665 - protein, 9 aa, synthetic construct
GGLGHDVLK

SEQ ID NO: 50666 - protein, 9 aa, synthetic construct
GGLGHDVLR

SEQ ID NO: 50667 - protein, 9 aa, synthetic construct
GGLGHDVLW

SEQ ID NO: 50668 - protein, 9 aa, synthetic construct
GGLGHDVMD

SEQ ID NO: 50669 - protein, 9 aa, synthetic construct
GGLGHDVML

SEQ ID NO: 50670 - protein, 9 aa, synthetic construct
GGLGHDVYT

SEQ ID NO: 50671 - protein, 9 aa, synthetic construct
GGLGHDWLH

SEQ ID NO: 50672 - protein, 9 aa, synthetic construct
GGLGHDYID

SEQ ID NO: 50673 - protein, 9 aa, synthetic construct
GGLGIDLLD

SEQ ID NO: 50674 - protein, 9 aa, synthetic construct
GGLGHDYLE

SEQ ID NO: 50675 - protein, 9 aa, synthetic construct
GGLGHDYLR

SEQ ID NO: 50676 - protein, 9 aa, synthetic construct
GGLGHDYLS

SEQ ID NO: 50677 - protein, 9 aa, synthetic construct
GGLGIDALD

SEQ ID NO: 50678 - protein, 9 aa, synthetic construct
GGLGIDDIH

SEQ ID NO: 50679 - protein, 9 aa, synthetic construct
GGLGIDDMT

SEQ ID NO: 50680 - protein, 9 aa, synthetic construct
GGLGIDHMK

SEQ ID NO: 50681 - protein, 9 aa, synthetic construct
GGLGIDIAD

SEQ ID NO: 50682 - protein, 9 aa, synthetic construct
GGLGIDIMA

SEQ ID NO: 50683 - protein, 9 aa, synthetic construct
GGLGIDIMD

SEQ ID NO: 50684 - protein, 9 aa, synthetic construct
GGLGIDKAL

SEQ ID NO: 50685 - protein, 9 aa, synthetic construct
GGLGIDKIY

SEQ ID NO: 50686 - protein, 9 aa, synthetic construct
GGLGIDLLA

SEQ ID NO: 50687 - protein, 9 aa, synthetic construct
GGAGADAAG

SEQ ID NO: 50688 - protein, 10 aa, synthetic construct
GNSLAKNVLF

SEQ ID NO: 50689 - protein, 118 aa, synthetic construct
YLSGYGHHIIDDDGGKEDKLSLADIDFRDVAFKREGNDLIMYKAEGNVLSIGHKNGITFRNWFEKESGDISNHQIEQIFDKSGRIITPDSLKKALEYQQRNNKASYVYGNDALAYGSQ

SEQ ID NO: 50690 - protein, 218 aa, synthetic construct
GNSLAKNVLFGGKGNDKLYGSEGADLLDGGEGDDLLKGGYGNDIYRYLSGYGHHIIDDDGGKEDKLSLADIDFRDVAFKREGNDLIMYKAEGNVLSIGHKNGITFRNWFEKESGDISNHQIEQIFDKSGRIITPDSLKKALEYQQRNNKASYVYGNDALAYGSQGDLNPLINEISKIISAAGSFDVKEERTAASLLQLSGNASDFSYGRNSITLTTSA

SEQ ID NO: 50691 - protein, 128 aa, synthetic construct
GNSLAKNVLFYLSGYGHHIIDDDGGKEDKLSLADIDFRDVAFKREGNDLIMYKAEGNVLSIGHKNGITFRNWFEKESGDISNHQIEQIFDKSGRIITPDSLKKALEYQQRNNKASYVYGNDALAYGSQ

SEQ ID NO: 50692 - protein, 9 aa, synthetic construct
GGAGNATLV

SEQ ID NO: 50693 - protein, 5 aa, synthetic construct
GGGGS

SEQ ID NO: 50694 - protein, 7 aa, synthetic construct
ENLYFQX

SEQ ID NO: 50695 - protein, 36 aa, synthetic construct
GGKGNDKLYGSEGADLLDGGEGDDLLKGGYGNDIYR

SEQ ID NO: 50696 - protein, 53 aa, Homo sapiens
NSDSECPLSHDGYCLHDGVCMYIEALDKYACNCVVGYIGERCQYRDLKWWELR
